European Patent Specification EP 3 802 789 B1, published April 8, 2026. Title: ENGINEERING ANTIMICROBIAL PEPTIDES. Applicant: Syngulon SA Gabant, Philippe. The sequence listing filed with the application follows.

SEQUENCE LISTING (750 sequences)

SEQ ID NO: 1 - protein, 40 aa, Enterococcus faecalis
WLPPAGLLGRCGRWFRPWLLWLQSGAQYKWLGNLFGLGPK

SEQ ID NO: 2 - protein, 5 aa, Artificial Sequence
  N-terminal motif of class terminal IIa
  VARIANT 3: Xaa = any amino acid
YGXGV

SEQ ID NO: 3 - protein, 135 aa, Artificial Sequence
  Hybrid bacteriocin Ent35-MccV
GKYYGNGVSCNKKGCSVDWGRAIGIIGNNSAANLATGGAAGWKSGGGASGRDIAMAIGTLSGQFVAGGIGAAAGGVAGGAIYDYASTHKPNPAMSPSGLGGTIKQKPEGIPSEAWNYAAGRLCNWSPNNLSDVCL

SEQ ID NO: 4 - protein, 46 aa, Lactobacillus acidophilus
MISSHQKTLTDKELALISGGKTHYPTNAWKSLWKGFWESLRYTDGF

SEQ ID NO: 5 - DNA, 141 bp, Lactobacillus acidophilus
atgatttcatctcatcaaaaaacgttaactgataaagaattagcattaatttctggggggaaaacgcactacccgactaatgcatggaaaagtctttggaaaggtttctgggaaagccttcgttatactgacggtttttag

SEQ ID NO: 6 - protein, 81 aa, Lactobacillus acidophilus
MISMISSHQKTLTDKELALISGGKTYYGTNGVHCTKKSLWGKVRLKNVIPGTLCRKQSLPIKQDLKILLGWATGAFGKTFH

SEQ ID NO: 7 - DNA, 246 bp, Lactobacillus acidophilus
atgatttcaatgatttcatctcatcaaaaaacgttaactgataaagaattagcattaatttctggggggaaaacgtactatggtactaatggtgtgcattgtactaaaaagagtctttggggtaaagtacgcttaaaaaacgtgattcctggaactctttgtcgtaagcaatcgttgccgatcaaacaggatttaaaaattttactgggctgggctacaggtgcttttggcaagacatttcattaa

SEQ ID NO: 8 - protein, 60 aa, Lactobacillus acidophilus
MDKKTKILFEVLYIICIIGPQFILFVTAKNNMYQLVGSFVGIVWFSYIFWYIFFKQHKKM

SEQ ID NO: 9 - DNA, 183 bp, Lactobacillus acidophilus
atggataagaaaacaaaaatattatttgaagtattatacatcatctgtataataggccctcaatttatattatttgtgactgcaaaaaacaatatgtatcagttggtgggttcgtttgttggaatagtatggttttcgtatattttttggtatatttttttcaaacaacataaaaaaatgtag

SEQ ID NO: 10 - protein, 65 aa, Lactobacillus gasseri
MALKTLEKHELRNVMGGNKWGNAVIGAATGATRGVSWCRGFGPWGMTACALGGAAIGGYLGYKSN

SEQ ID NO: 11 - DNA, 198 bp, Lactobacillus gasseri
atggctttaaaaacattagaaaaacatgaattaagaaatgtaatgggtggaaacaagtgggggaatgctgtaataggagctgctacgggagctactcgcggagtaagttggtgcagaggattcggaccatggggaatgactgcctgtgcgttaggaggtgctgcaattggaggatatctgggatataagagtaattaa

SEQ ID NO: 12 - protein, 51 aa, Staphylococcus aureus [sequence omitted]

SEQ ID NO: 13 - DNA, 156 bp, Staphylococcus aureus
atgagttggttaaattttttaaaatacatcgctaaatatggcaaaaaagcggtatctgctgcttggaagtacaaaggtaaagtattagaatggcttaatgttggtcctactcttgaatgggtatggcaaaaattaaagaaaattgctggattataa

SEQ ID NO: 14 - protein, 61 aa, Enterococcus avium
MTRSKKLNLREMKNVVGGTYYGNGVSCNKKGCSVDWGKAISIIGNNSAANLATGGAAGWKS

SEQ ID NO: 15 - DNA, 186 bp, Enterococcus avium
atgacaagatcaaaaaaattaaatttacgcgaaatgaagaatgttgttggtggtacctactatggaaatggtgtatcttgtaacaagaaaggctgttcagttgactggggcaaagccatcagtattataggaaataattccgcagcaaacttagcaactggtggtgctgctggttggaagtcataa

SEQ ID NO: 16 - protein, 67 aa, Enterococcus faecalis
MKKKLVICGIIGIGFTALGTNVEAATYYGNGLYCNKQKCWVDWNKASREIGKIIVNGWVQHGPWAPR

SEQ ID NO: 17 - DNA, 204 bp, Enterococcus faecalis
atgaaaaagaaattagttatttgtggcattattgggattggttttacagcattaggaacaaatgtagaagctgctacgtattacggaaatggtttatattgtaataagcaaaaatgttgggtagactggaataaagcttcaagggaaattggaaaaattattgttaatggttgggtacaacatggcccttgggctcctagatag

SEQ ID NO: 18 - protein, 51 aa, Lactococcus lactis
MKEQNSFNLLQEVTESELDLILGAKGGSGVIHTISHEVIYNSWNFVFTCCS

SEQ ID NO: 19 - DNA, 156 bp, Lactococcus lactis
atgaaagaacaaaactcttttaatcttcttcaagaagtgacagaaagtgaattggaccttattttaggtgcaaaaggcggcagtggagttattcatacaatttctcatgaagtaatatataatagctggaactttgtatttacttgctgctcttaa

SEQ ID NO: 20 - protein, 74 aa, Enterococcus faecium
MKKKVLKHCVILGILGTCLAGIGTGIKVDAATYYGNGLYCNKEKCWVDWNQAKGEIGKIIVNGWVNHGPWAPRR

SEQ ID NO: 21 - DNA, 225 bp, Enterococcus faecium
atgaaaaagaaagtattaaaacattgtgttattctaggaatattaggaacttgtctagctggcatcggtacaggaataaaagttgatgcagctacttactatggaaatggtctttattgtaacaaagaaaaatgttgggtagattggaatcaagctaaaggagaaattggaaaaattattgttaatggttgggttaatcatggtccatgggcacctagaaggtag

SEQ ID NO: 22 - protein, 50 aa, Clostridium botulinum
MQKPEIISADLGLCAVNEFVALAAIPGGAATFAVCQMPNLDEIVSNAAYV

SEQ ID NO: 23 - DNA, 153 bp, Clostridium botulinum
atgcaaaaaccagaaattattagtgctgatttagggctttgtgcagttaatgaatttgtagctcttgctgccattcctggtggtgctgctacatttgcagtatgccaaatgccaaacttggatgagattgttagtaatgcagcatatgtttaa

SEQ ID NO: 24 - protein, 58 aa, Streptococcus equinus
MMNATENQIFVETVSDQELEMLIGGADRGWIKTLTKDCPNVISSICAGTIITACKNCA

SEQ ID NO: 25 - DNA, 177 bp, Streptococcus equinus
atgatgaatgctactgaaaaccaaatttttgttgagactgtgagtgaccaagaattagaaatgttaattggtggtgcagatcgtggatggattaagactttaacaaaagattgtccaaatgtaatttcttcaatttgtgcaggtacaattattacagcttgtaaaaattgtgcttaa

SEQ ID NO: 26 - protein, 77 aa, Brochothrix campestris
MHKVKKLNNQELQQIVGGYSSKDCLKDIGKGIGAGTVAGAAGGGLAAGLGAIPGAFVGAHFGVIGGSAACIGGLLGN

SEQ ID NO: 27 - DNA, 234 bp, Brochothrix campestris
atgcacaaggtaaaaaaattaaacaatcaagagttacaacagatcgtgggaggttacagttcaaaagattgtctaaaagatattggtaaaggaattggtgctggtacagtagctggggcagccggcggtggcctagctgcaggattaggtgctatcccaggagcattcgttggagcacattttggagtaatcggcggatctgccgcatgcattggtggattattaggtaactag

SEQ ID NO: 28 - protein, 80 aa, Butyrivibrio fibrisolvens
MSKKQIMSNCISIALLIALIPNIYFIADKMGIQLAPAWYQDIVNWVSAGGTLTTGFAIIVGVTVPAWIAEAAAAFGIASA

SEQ ID NO: 29 - DNA, 243 bp, Butyrivibrio fibrisolvens
atgagtaaaaaacaaattatgagtaactgtatatcaattgcattattaatagcactaattcctaatatctattttattgcagataaaatgggaattcagttagcacctgcttggtatcaagatattgtgaattgggtatctgctggtggaacacttactactggttttgcgattattgtaggagttacagtaccggcatggatagcagaagcagctgcagcttttggtatagcttcagcatga

SEQ ID NO: 30 - protein, 48 aa, Butyrivibrio fibrisolvens
MNKELNALTNPIDEKELEQILGGGNGVIKTISHECHMNTWQFIFTCCS

SEQ ID NO: 31 - DNA, 147 bp, Butyrivibrio fibrisolvens
atgaacaaagaacttaatgcacttacaaatcctattgacgagaaggagcttgagcagatcctcggtggtggcaatggtgtcatcaagacaatcagccacgagtgccacatgaacacatggcagttcattttcacatgttgctcttaa

SEQ ID NO: 32 - protein, 66 aa, Carnobacterium maltaromaticum
MNSVKELNVKEMKQLHGGVNYGNGVSCSKTKCSVNWGQAFQERYTAGINSFVSGVASGAGSIGRRP

SEQ ID NO: 33 - DNA, 201 bp, Carnobacterium maltaromaticum
atgaatagcgtaaaagaattaaacgtgaaagaaatgaaacaattacacggtggagtaaattatggtaatggtgtttcttgcagtaaaacaaaatgttcagttaactggggacaagcctttcaagaaagatacacagctggaattaactcatttgtaagtggagtcgcttctggggcaggatccattggtaggagaccgtaa

SEQ ID NO: 34 - protein, 61 aa, Carnobacterium maltaromaticum
MKSVKELNKKEMQQINGGAISYGNGVYCNKEKCWVNKAENKQAITGIVIGGWASSLAGMGH

SEQ ID NO: 35 - DNA, 186 bp, Carnobacterium maltaromaticum
atgaaaagcgttaaagaactaaataaaaaagaaatgcaacaaattaatggtggagctatctcttatggcaatggtgtttattgtaacaaagagaaatgttgggtaaacaaggcagaaaacaaacaagctattactggaatagttatcggtggatgggcttctagtttagcaggaatgggacattaa

SEQ ID NO: 36 - protein, 71 aa, Carnobacterium maltaromaticum
MNNVKELSIKEMQQVTGGDQMSDGVNYGKGSSLSKGGAKCGLGIVGGLATIPSGPLGWLAGAAGVINSCMK

SEQ ID NO: 37 - DNA, 216 bp, Carnobacterium maltaromaticum
atgaataatgtaaaagagttaagtattaaagaaatgcaacaagttactggtggagaccaaatgtcagatggtgtaaattatggaaaaggctctagcttatcaaaaggtggtgccaaatgtggtttagggatcgtcggcggattagctactatcccttcaggtcctttaggctggttagccggagcagcaggtgtaattaatagctgtatgaaataa

SEQ ID NO: 38 - protein, 64 aa, Carnobacterium maltaromaticum
MLYELVAYGIAQGTAEKVVSLINAGLTVGSIISILGGVTVGLSGVFTAVKAAIAKQGIKKAIQL

SEQ ID NO: 39 - DNA, 195 bp, Carnobacterium maltaromaticum
atgttatatgaattagttgcatatggtatcgcacaaggtacagctgaaaaggttgtaagtctaattaacgcaggtttaacagtagggtctattatttcaattttgggtggggtcacagtcggtttatcaggtgtcttcacagcagttaaagcagcaattgctaaacaaggaataaaaaaagcaattcaattataa

SEQ ID NO: 40 - protein, 836 aa, Pectobacterium carotovorum subsp. carotovorum
MIKYRLYAPNDGDTMTVSGGGGWVSNDDRKGGNDRDNGKGGSAVDFSKNPEKQAIVNPYLAIAIPMPVYPLYGKLGFTINTTAIETELANVRAAINTKLATLSAVIGRSLPVVGRVFGVTAAGMWPSSTAPSSLDSIYNQAHQQALAQLAAQQGVLNKGYNVTAMPAGFVSSLPVSEIKSLPTAPASLLAQSVINTELSQRQLALTQPTTNAPVANIPVVKAEKTAMPGVYSAKIIAGEPAFQIKVDNTKPALAQNPPKVKDDIQVSSFLSSPVADTHHAFIDFGSDHEPVYVSLSKIVTAEEEKKQVEEAKRREQEWLLRHPITAAERKLTEIRQVISFAQQLKESSVATISEKTKTVAVYQEQVNTAAKNRDNFYNQNRGLLSAGITGGPGYPIYLALWQTMNNFHQAYFRANNALEQESHVLNLARSDLAKAEQLLAENNRLQVETERTLAEEKEIKRNRVNVSTFGTVQTQLSKLLSDFYAVTSLSQSVPSGALASFSYNPQGMIGSGKIVGKDVDVLFSIPVKDIPGYKSPINLDDLAKKNGSLDLPIRLAFSDENGERVLRAFKADSLRIPSSVRGVAGSYDKNTGIFSAEIDGVSSRLVLENPAFPPTGNVGNTGNTAPDYKALLNTGVDVKPVDKITVTVTPVADPVDIDDYIIWLPTASGSGVEPIYVVFNSNPYGGTEKGKYSKRYYNPDKAGGPILELDWKNVKIDHAGVDNVKLHTGRFKASVENKVMIERLENILNGQITATDTDKRFYTHELRELNRYRNLGIKDGEVPSSIQEESAVWNDTHTATLEDYKINEKEQPLYTDAALQAAYEQELKDALGGKHG

SEQ ID NO: 41 - DNA, 2511 bp, Pectobacterium carotovorum subsp. carotovorum
atgattaaataccgtttatatgctccaaatgatggagacaccatgacagtgagtggtggtggtggttgggtttcaaacgatgatcgcaaaggtggtaatgacagggacaatggcaaaggtggttctgccgttgattttagtaaaaatccagaaaagcaggctatcgttaatccctatttggcaatcgcgataccgatgccggtctaccctctttatggaaagctagggttcacaataaatacgacggcaattgagactgaactcgcaaatgtcagagcagcaattaacactaaacttgcaacactcagtgcagtgattggcagatcacttccggtcgttgggcgggtatttggtgttactgccgccggaatgtggccttctagtaccgctcccagtagtctcgattctatatacaatcaagcacatcagcaggctttagcccagttagctgctcaacagggagtattaaataaagggtataacgttacagcaatgcctgcaggtttcgtcagcagtttgcctgttagtgaaatcaaatcattgccaacagctcccgccagtttactggcacaaagtgtgattaataccgaactttcccagcgtcaactggctcttactcagcccacgacgaatgcaccagtcgcgaatattcccgtagttaaagcagagaaaacagcaatgccaggtgtgtattcagcgaaaattattgctggtgagcctgcattccaaatcaaggtcgataataccaaacctgctttggcacagaatccgccgaaagtaaaagatgatattcaggtatcttctttcctttcctcgccagtagctgatacgcaccatgcatttattgattttggcagcgatcatgaaccggtatacgtgtctctttcaaagatcgtgacagccgaggaggagaaaaaacaggttgaagaggccaagcgccgtgagcaggagtggttgttgcgtcatccaattacagctgcggagcgaaaattaactgaaatccgccaagtgatctcttttgctcaacagctaaaagaaagctctgtcgcaaccatttcagaaaaaactaaaactgttgcggtttaccaagaacaggtgaataccgctgcaaaaaatcgcgacaatttttataatcaaaatagaggtctgttaagtgcgggtataactgggggaccgggatatcctatttatcttgctttatggcaaacgatgaataactttcatcaggcttatttcagagcaaataatgcattggaacaagagagtcatgttctgaacctggctcgttctgatctggctaaggctgagcaattgcttgctgagaataatcgacttcaggttgaaacggagcgaacgcttgccgaagaaaaagagataaaacgcaacagggttaatgtatcaacatttggcacagtgcaaactcaacttagtaaattgctgtcagatttttatgctgttacatcactttcccaaagtgttccttcgggggcattagcctctttttcatataatccacaagggatgattggcagcggtaagattgttgggaaggatgtcgatgttttattttccatcccagtaaaagatattccgggatataaatctcctattaacttggacgatttagccaagaaaaatggaagtctggatcttcccattcgtctggcattttctgatgagaatggagaaagggttcttcgggcattcaaagcggatagtctgcgaatcccttcgagtgtcagaggtgtagcgggcagttatgacaaaaatacgggtatttttagtgcagaaattgatggtgtttcatctcgccttgtactggaaaacccagcgtttcctccgaccggaaatgtcggtaatacgggtaatactgcacctgactataaagcattactgaatactggtgttgatgttaaacctgttgataaaatcacagttacggtaacaccagttgctgatccagtggatattgatgactatataatctggttgccaactgcgtctggttctggcgtggaacccatttatgtcgtgtttaacagtaatccgtatggtgggacggaaaaaggaaaatatagcaaacgttattataatccagataaggcaggcggtccgatcttggagctggattggaaaaacgttaagattgaccatgcaggtgtggacaatgttaaattacacacagggcgtttcaaagcgtcggttgaaaacaaagtgatgattgaacgtttggaaaacatactgaatggtcaaatcacggccacggatactgacaagcgattctatacgcatgaattaagagagttaaaccgctacagaaatttaggcatcaaagacggtgaagtgcctagtagcattcaagaagaaagcgctgtttggaacgacacacacacagcgacgcttgaagactacaaaattaatgagaaagagcaaccgttgtacactgatgctgctttgcaggcagcctacgaacaggaactcaaagacgcattaggagggaaacatggctaa

SEQ ID NO: 42 - protein, 74 aa, Bacillus cereus
MENLQMLTEEELMEIEGGGWWNSWGKCVAGTIGGAGTGGLGGAAAGSAVPVIGTGIGGAIGGVSGGLTGAATFC

SEQ ID NO: 43 - DNA, 225 bp, Bacillus cereus
atggaaaacttacaaatgttaactgaagaagaattaatggaaattgaaggtggaggctggtggaatagctggggtaaatgtgttgctggaactatcggtggagctggaactggtggtttaggtggagctgctgcaggttcagctgttccggttattggtactggtattggtggcgctattggtggagttagcggtggccttacaggtgcagctactttttgctaa

SEQ ID NO: 44 - protein, 78 aa, Streptoverticillium griseoverticillatum
MTASILQQSVVDADFRAALLENPAAFGASAAALPTPVEAQDQASLDFWTKDIAATEAFACRQSCSFGPFTFVCDGNTK

SEQ ID NO: 45 - DNA, 237 bp, Streptoverticillium griseoverticillatum
atgaccgcttccattcttcagcagtccgtcgtggacgccgacttccgcgcggcgctgcttgagaaccccgccgccttcggcgcttccgccgcggccctgcccacgcccgtcgaggcccaggaccaggcgtcccttgacttctggaccaaggacatcgccgccacggaagccttcgcctgccgccagagctgcagcttcggcccgttcaccttcgtgtgcgacggcaacaccaagtaa

SEQ ID NO: 46 - protein, 76 aa, Geobacillus kaustophilus
MSLLALVAGTLGVSQSIATTVVSIVLTGSTLISIILGITAILSGGVDAILEIGWSAFVATVKKIVAERGKAAAIAW

SEQ ID NO: 47 - DNA, 231 bp, Geobacillus kaustophilus
atgagtttgctggcgcttgttgccgggacgctcggcgtgtcacagtcaatcgcgacgacggttgtttcgattgtgttgaccggctccactctcatttctattattcttgggatcaccgctattttgtcaggtggagtcgacgccattttggaaattgggtggtcagcttttgtcgcgacggtgaaaaaaatagtggcggaacgaggaaaagcggcagcgattgcatggtaa

SEQ ID NO: 48 - protein, 309 aa, Clostridium tyrobutyricum
MRKVFLRSIISTLVMCAFVSSSFSVNADESKPNDEKIINNIENVTTTKDIVKSNKNNIVYLDEGVMSIPLSGRKPIAIKDDNNKEDLTVTLPIKNTGDISKISSNGTILYKNNSSNSSNIALQPKNDGFKALININDKLANKEYEFTFNLPKNSKLISAATYLGKEYDTKEVFVVDKNNIITSIISPAWAKDANGHNVSTYYKIVSNNKLVQVVEFTENTAFPVVADPNWTKIGKCAGSIAWAIGSGLFGGAKLIKIKKYIAELGGLQKAAKLLVGATTWEEKLHAGGYALINLAAELTGVAGIQANCF

SEQ ID NO: 49 - DNA, 930 bp, Clostridium tyrobutyricum
ttgagaaaagtatttttaagatcaataatttcaacattagttatgtgtgcatttgtttcaagcagcttttcagtaaatgcggatgaaagcaaaccaaatgatgaaaaaataattaataacatagaaaacgttactactactaaagatattgtaaaaagtaataaaaataatattgtatatttagatgaaggtgtaatgagtattccattgtctgggagaaaacccattgctattaaagatgataataataaagaagatttaactgttacattacctattaagaatactggagatatatctaaaattagtagtaatggtactattctgtataaaaataatagtagtaattcatctaatatagctttacaacctaaaaatgatggatttaaggctttaataaatattaatgataagttagctaataaagaatatgaatttacatttaatttacccaaaaacagtaaattaattagtgctgccacatatttgggtaaagaatatgatacaaaagaagtatttgtagtagacaaaaataatataattacgagtattattagtccagcttgggctaaagatgcaaatggacataatgtttctacttattataagatagtatcgaataataaattagtacaagttgttgaattcacagaaaatactgcattcccggtggtagctgatcctaattggactaaaattgggaaatgcgctgggtcaatagcatgggctataggttctggcctttttggtggagcaaagctaattaaaataaaaaaatatatagcagagcttggaggacttcaaaaagcagctaaattattagttggtgcaaccacttgggaagaaaaattacacgcaggcggttatgcattaattaacttagctgctgagctaacaggtgtagcaggtatacaagcaaattgtttttaa

SEQ ID NO: 50 - protein, 62 aa, Bacillus coagulans
MKKIEKLTEKEMANIIGGKYYGNGVTCGKHSCSVDWGKATTCIINNGAMAWATGGHQGTHKC

SEQ ID NO: 51 - DNA, 189 bp, Bacillus coagulans
atgaaaaaaattgaaaaattaactgaaaaagaaatggccaatatcattggtggtaaatactacggtaatggggttacttgtggcaaacattcctgctctgttgactggggtaaggctaccacctgcataatcaataatggagctatggcatgggctactggtggacatcaaggtactcataaatgctag

SEQ ID NO: 52 - protein, 490 aa, Escherichia coli
MDKVTDNSPDVESTESTEGSFPTVGVDTGDTITATLATGTENVGGGGGAFGGASESSAAIHATAKWSTAQLKKHQAEQAARAAAAEAALAKAKSQRDALTQRLKDIVNDALRANAARSPSVTDLAHANNMAMQAEAERLRLAKAEQKAREEAEAAEKALREAERQRDEIARQQAETAHLLAMAEAAEAEKNRQDSLDEEHRAVEVAEKKLAEAKAELAKAESDVQSKQAIVSRVAGELENAQKSVDVKVTGFPGWRDVQKKLERQLQDKKNEYSSVTNALNSAVSIRDAKKTEVQNAEIKLKEAKDALEKSQVKDSVDTMVGFYQYITEQYGEKYSRIAQDLAEKAKGSKFNSVDEALAAFEKYKNVLDKKFSKVDRDDIFNALESITYDEWAKHLEKISRALKVTGYLSFGYDVWDGTLKGLKTGDWKPLFVTLEKSAVDFGVAKIVALMFSFIVGAPLGFWGIAIITGIVSSYIGDDELNKLNELLGI

SEQ ID NO: 53 - DNA, 1473 bp, Escherichia coli
atggataaagtcactgataattctccagatgtggagagcacagaatctactgaggggtcattcccaactgttggggttgatactggcgatacgattacagcgacgcttgcaactggaactgaaaatgttggtggaggcggtggagcatttggtggggccagtgaaagttctgctgcgatacatgcaaccgctaaatggtctaccgcgcagttgaaaaaacatcaggctgaacaggctgcccgtgctgctgcggctgaggcagcattggcaaaagcgaaatctcagcgtgatgccctgactcaacgtctcaaggatattgttaatgacgctttacgtgctaatgccgctcgtagtccatcagtaactgaccttgctcatgccaataatatggcaatgcaggcagaggctgagcgtttgcgccttgcgaaggcagagcaaaaagcccgtgaagaagctgaagcagcagaaaaagcgctccgggaagcagaacgccaacgtgatgagattgcccgccaacaggctgaaaccgcgcatttgttagcaatggcggaggcagcagaggctgagaaaaatcgacaggattctcttgatgaagagcatcgggctgtggaagtggcagagaagaagctggctgaggctaaagctgaactggcgaaggccgaaagcgatgtacagagtaagcaagcgattgtttccagagttgcaggggagcttgaaaacgctcaaaaaagtgttgatgtgaaggttaccggatttcctggatggcgtgatgttcagaaaaaactggagagacaattgcaggataagaagaatgaatattcgtcagtgacgaatgctcttaattctgctgttagcattagagatgctaaaaaaacagaagttcagaatgctgagataaaattaaaagaagctaaggatgctcttgagaagagtcaggtaaaagactctgttgatactatggttgggttttatcaatatataaccgaacaatatggggaaaaatattccagaatagctcaggatttagctgaaaaggcgaagggtagtaaatttaatagtgttgatgaagcacttgctgcatttgaaaagtataaaaatgtactggataagaaattcagtaaggttgatagggatgatatttttaatgctttagagtctattacttatgatgagtgggccaagcatctagaaaagatctctagggctcttaaggttactggatatttgtctttcgggtatgatgtatgggatggtaccctaaagggattaaaaacaggagactggaagcctttatttgtcactctggagaagagcgcggtagatttcggcgtggcaaaaattgtggcattaatgtttagttttattgttggtgcgcctcttggcttctggggaattgcaattatcacaggtattgtttcttcttacataggggatgatgagttgaacaagcttaatgaattactaggtatttaa

SEQ ID NO: 54 - protein, 522 aa, Escherichia coli
METAVAYYKDGVPYDDKGQVIITLLNGTPDGSGSGGGGGKGGSKSESSAAIHATAKWSTAQLKKTQAEQAARAKAAAEAQAKAKANRDALTQRLKDIVNEALRHNASRTPSATELAHANNAAMQAEDERLRLAKAEEKARKEAEAAEKAFQEAEQRRKEIEREKAETERQLKLAEAEEKRLAALSEEAKAVEIAQKKLSAAQSEVVKMDGEIKTLNSRLSSSIHARDAEMKTLAGKRNELAQASAKYKELDELVKKLSPRANDPLQNRPFFEATRRRVGAGKIREEKQKQVTASETRINRINADITQIQKAISQVSNNRNAGIARVHEAEENLKKAQNNLLNSQIKDAVDATVSFYQTLTEKYGEKYSKMAQELADKSKGKKIGNVNEALAAFEKYKDVLNKKFSKADRDAIFNALASVKYDDWAKHLDQFAKYLKITGHVSFGYDVVSDILKIKDTGDWKPLFLTLEKKAADAGVSYVVALLFSLLAGTTLGIWGIAIVTGILCSYIDKNKLNTINEVLGI

SEQ ID NO: 55 - DNA, 1569 bp, Escherichia coli
atggaaaccgcggtagcgtactataaagatggtgttccttatgatgataagggacaggtaattattactcttttgaatggtactcctgacgggagtggctctggcggcggaggtggaaaaggaggcagtaaaagtgaaagttctgcagctattcatgcaactgctaaatggtctactgctcaattaaagaaaacacaggcagagcaggctgcccgggcaaaagctgcagcggaagcacaggcgaaagcaaaggcaaacagggatgcgctgactcagcgcctgaaggatatcgtgaatgaggctcttcgtcacaatgcctcacgtacgccttcagcaacagagcttgctcatgctaataatgcagctatgcaggcggaagacgagcgtttgcgccttgcgaaagcagaagaaaaagcccgtaaagaagcggaagcagcagaaaaggcttttcaggaagcagaacaacgacgtaaagagattgaacgggagaaggctgaaacagaacgccagttgaaactggctgaagctgaagagaaacgactggctgcattgagtgaagaagctaaagctgttgagatcgcccaaaaaaaactttctgctgcacaatctgaagtggtgaaaatggatggagagattaagactctcaattctcgtttaagctccagtatccatgcccgtgatgcagaaatgaaaacgctcgctggaaaacgaaatgaactggctcaggcatccgctaaatataaagaactggatgagctggtcaaaaaactatcaccaagagccaatgatccgcttcagaaccgtcctttttttgaagcaaccagacgacgggttggggccggtaagattagagaagaaaaacaaaaacaggtaacagcatcagaaacacgtattaaccggataaatgctgatataactcagatccagaaggctatttctcaggtcagtaataatcgtaatgccggtatcgctcgtgttcatgaagctgaagaaaatttgaaaaaagcacagaataatctccttaattcacagattaaggatgctgttgatgcaacagttagcttttatcaaacgctgactgaaaaatatggtgaaaaatattcgaaaatggcacaggaacttgctgataagtctaaaggtaagaaaatcggcaatgtgaatgaagctctcgctgcttttgaaaaatacaaggatgttttaaataagaaattcagcaaagccgatcgtgatgctatttttaatgcgttggcatcggtgaagtatgatgactgggctaaacatttagatcagtttgccaagtacttgaagattacggggcatgtttcttttggatatgatgtggtatctgatatcctaaaaattaaggatacaggtgactggaagccactatttcttacattagagaagaaagctgcagatgcaggggtgagttatgttgttgctttactttttagcttgcttgctggaactacattaggtatttggggtattgctattgttacaggaattctatgctcctatattgataagaataaacttaatactataaatgaggtgttagggatttaa

SEQ ID NO: 56 - protein, 626 aa, Escherichia coli
MSDPVRITNPGAESLGYDSDGHEIMAVDIYVNPPRVDVFHGTPPAWSSFGNKTIWGGNEWVDDSPTRSDIEKRDKEITAYKNTLSAQQKENENKRTEAGKRLSAAIAAREKDENTLKTLRAGNADAADITRQEFRLLQAELREYGFRTEIAGYDALRLHTESRMLFADADSLRISPREARSLIEQAEKRQKDAQNADKKAADMLAEYERRKGILDTRLSELEKNGGAALAVLDAQQARLLGQQTRNDRAISEARNKLSSVTESLNTARNALTRAEQQLTQQKNTPDGKTIVSPEKFPGRSSTNHSIVVSGDPRFAGTIKITTSAVIDNRANLNYLLSHSGLDYKRNILNDRNPVVTEDVEGDKKIYNAEVAEWDKLRQRLLDARNKITSAESAVNSARNNLSARTNEQKHANDALNALLKEKENIRNQLSGINQKIAEEKRKQDELKATKDAINFTTEFLKSVSEKYGAKAEQLAREMAGQAKGKKIRNVEEALKTYEKYRADINKKINAKDRAAIAAALESVKLSDISSNLNRFSRGLGYAGKFTSLADWITEFGKAVRTENWRPLFVKTETIIAGNAATALVALVFSILTGSALGIIGYGLLMAVTGALIDESLVEKANKFWGI

SEQ ID NO: 57 - DNA, 1881 bp, Escherichia coli
atgtctgaccctgtacgtattacaaatcccggtgcagaatcgctggggtatgattcagatggccatgaaattatggccgttgatatttatgtaaaccctccacgtgtcgatgtctttcatggtaccccgcctgcatggagttccttcgggaacaaaaccatctggggcggaaacgagtgggttgatgattccccaacccgaagtgatatcgaaaaaagggacaaggaaatcacagcgtacaaaaacacgctcagcgcgcagcagaaagagaatgagaataagcgtactgaagccggaaaacgcctctctgcggcgattgctgcaagggaaaaagatgaaaacacactgaaaacactccgtgccggaaacgcagatgccgctgatattacacgacaggagttcagactcctgcaggcagagctgagagaatacggattccgtactgaaatcgccggatatgacgccctccggctgcatacagagagccggatgctgtttgctgatgctgattctcttcgtatatctccccgggaggccaggtcgttaatcgaacaggctgaaaaacggcagaaggatgcgcagaacgcagacaagaaggccgctgatatgcttgctgaatacgagcgcagaaaaggtattctggacacccggttgtcagagctggaaaaaaatggcggggcagcccttgccgttcttgatgcacaacaggcccgtctgctcgggcagcagacacggaatgacagggccatttcagaggcccggaataaactcagttcagtgacggaatcgcttaacacggcccgtaatgcattaaccagagctgaacaacagctgacgcaacagaaaaacacgcctgacggcaaaacgatagtttcccctgaaaaattcccggggcgttcatcaacaaatgattctattgttgtgagcggtgatccgagatttgccggtacgataaaaatcacaaccagcgcagtcatcgataaccgtgcaaacctgaattatcttctgagccattccggtctggactataaacgcaatattctgaatgaccggaatccggtggtgacagaggatgtggaaggtgacaagaaaatttataatgctgaagttgctgaatgggataagttacggcaaagattgcttgatgccagaaataaaatcacctctgctgaatctgcggtaaattcggcgagaaataacctcagtgccagaacaaatgagcaaaagcatgcaaatgacgctcttaatgccctgttgaaggaaaaagagaatatccgtaaccagctttccggcatcaatcagaagatagcggaagagaaaagaaaacaggatgaactgaaggcaacgaaagacgcaattaatttcacaacagagttcctgaaatcagtttcagaaaaatatggtgcaaaagctgagcagttagccagagagatggccgggcaggctaaagggaagaaaatacgtaatgttgaagaggcattaaaaacgtatgaaaagtaccgggctgacattaacaaaaaaattaatgcaaaagatcgtgcagcgattgccgcagcccttgagtctgtgaagctgtctgatatatcgtctaatctgaacagattcagtcggggactgggatatgcaggaaaatttacaagtcttgctgactggatcactgagtttggtaaggctgtccggacagagaactggcgtcctctttttgttaaaacagaaaccatcatagcaggcaatgccgcaacggctcttgtggcactggtcttcagtattcttaccggaagcgctttaggcattatcgggtatggtttactgatggctgtcaccggtgcgctgattgatgaatcgcttgtggaaaaagcgaataagttctggggtatttaa

SEQ ID NO: 58 - protein, 626 aa, Escherichia coli
MSDPVRITNPGAESLGYDSDGHEIMAVDIYVNPPRVDVFHGTPPAWSSFGNKTIWGGNEWVDDSPTRSDIEKRDKEITAYKNTLSAQQKENENKRTEAGKRLSAAIAAREKDENTLKTLRAGNADAADITRQEFRLLQAELREYGFRTEIAGYDALRLHTESRMLFADADSLRISPREARSLIEQAEKRQKDAQNADKKAADMLAEYERRKGILDTRLSELEKNGGAALAVLDAQQARLLGQQTRNDRAISEARNKLSSVTESLKTARNALTRAEQQLTQQKNTPDGKTIVSPEKFPGRSSTNHSIVVSGDPRFAGTIKITTSAVIDNRANLNYLLTHSGLDYKRNILNDRNPVVTEDVEGDKKIYNAEVAEWDKLRQRLLDARNKITSAESAINSARNNVSARTNEQKHANDALNALLKEKENIRSQLADINQKIAEEKRKRDEINMVKDAIKLTSDFYRTIYDEFGKQASELAKELASVSQGKQIKSVDDALNAFDKFRNNLNKKYNIQDRMAISKALEAINQVHMAENFKLFSKAFGFTGKVIERYDVAVELQKAVKTDNWRPFFVKLESLAAGRAASAVTAWAFSVMLGTPVGILGFAIIMAAVSALVNDKFIEQVNKLIGI

SEQ ID NO: 59 - DNA, 1881 bp, Escherichia coli
atgtctgaccctgtacgtattacaaatcccggtgcagaatcgctgggatatgattcagatggccatgaaattatggccgttgatatttatgtaaaccctccacgtgtcgatgtctttcatggtaccccgcctgcatggagttccttcgggaacaaaaccatctggggtggaaacgagtgggtcgatgattccccaacccgaagtgatatcgaaaaaagggacaaggaaatcacagcgtacaaaaacacgctcagcgcgcagcagaaagagaatgagaataagcgtactgaagctggaaaacgcctttctgcggcaattgctgcaagggaaaaagatgaaaacacactgaaaacactccgtgccggaaacgcagatgccgctgatattacacgacaggagttcagactcctgcaggcagagctgagagaatacggattccgtactgaaatcgccggatatgatgccctccggctgcatacagagagccggatgctgtttgctgatgctgattctcttcgtatatctccccgcgaggccaggtcgttaatcgaacaggctgaaaaacggcagaaggatgcgcagaacgcagacaagaaggccgctgatatgcttgctgaatacgagcgcagaaaaggtattctggacacgcggttgtcagagctggaaaaaaatggcggggcagcccttgccgttcttgatgcacaacaggcccgtctgctcgggcagcagacacggaatgacagggccatttcagaggcccggaataaactcagttcggtgacggaatcgcttaagacggcccgtaatgcattaaccagagctgaacaacagctgacgcaacagaaaaacacgcctgacggcaaaacgatagtttcccctgaaaaattcccggggcgttcatcaacaaatcattctattgttgtgagtggtgatccgaggtttgccggtacgataaaaatcacaaccagcgcggtcatcgataaccgtgcaaacctgaattatcttctgacccattccggtctggactataaacgcaatattctgaatgaccggaatccggtggtgacagaggatgtggaaggtgacaagaaaatttataatgctgaagttgctgaatgggataagttacggcaacgattgcttgatgccagaaataaaatcacctctgctgaatctgcgataaattcggcgagaaataacgtcagtgccagaacaaatgaacaaaagcatgcaaatgacgctcttaatgccctgttgaaggaaaaagagaatatccgtagccagcttgctgacatcaatcagaaaatagctgaagagaaaagaaaaagggatgaaataaatatggtaaaggatgccataaaactcacctctgatttctacagaacgatatatgatgagttcggtaaacaagcatccgaacttgctaaggagctggcttctgtatctcaagggaaacagattaagagtgtggatgatgcactgaacgcttttgataaattccgtaataatctgaacaagaaatataacatacaagatcgcatggccatttctaaagccctggaagctattaatcaggtccatatggcggagaattttaagctgttcagtaaggcatttggttttaccggaaaagttattgaacgttatgatgttgctgtggagttacaaaaggctgtaaaaacggacaactggcgtccattttttgtaaaacttgaatcactggcagcaggaagagctgcttcagcagttacagcatgggcgttttccgtcatgctgggaacccctgtaggtattctgggttttgcaattattatggcggctgtgagtgcgcttgttaatgataagtttattgagcaggtcaataaacttattggtatctga

SEQ ID NO: 60 - protein, 271 aa, Escherichia coli
METLTVHAPSPSTNLPSYGNGAFSLSAPHVPGAGPLLVQVVYSFFQSPNMCLQALTQLEDYIKKHGASNPLTLQIISTNIGYFCNADRNLVLHPGISVYDAYHFAKPAPSQYDYRSMNMKQMSGNVTTPIVALAHYLWGNGAERSVNIANIGLKISPMKINQIKDIIKSGVVGTFPVSTKFTHATGDYNVITGAYLGNITLKTEGTLTISANGSWTYNGVVRSYDDKYDFNASTHRGIIGESLTRLGAMFSGKEYQILLPGEIHIKESGKR

SEQ ID NO: 61 - DNA, 816 bp, Escherichia coli
atggaaaccttaactgttcatgcaccatcaccatcaactaacttaccaagttatggcaatggtgcattttctctttcagcaccacatgtgcctggtgctggccctcttttagtccaggttgtttatagttttttccagagtccaaacatgtgtcttcaggctttaactcaacttgaggattacatcaaaaaacatggggccagcaaccctctcacattgcagatcatatcgacaaatattggttacttctgtaacgccgaccgaaatctggttcttcaccctggaataagcgtttatgacgcttaccacttcgcaaaaccagcgccaagtcaatatgactatcgctcaatgaatatgaaacaaatgagcggtaatgtcactacaccaattgtggcgcttgctcactatttatggggtaatggcgctgaaaggagcgttaatatcgccaacattggtcttaaaatttcccctatgaaaattaatcagataaaagacattataaaatctggtgtagtaggcacattccctgtttctacaaagttcacacatgccactggtgattataatgttattaccggtgcatatcttggtaatatcacactgaaaacagaaggtactttaactatctctgccaatggctcctggacttacaatggcgttgttcgttcatatgatgataaatacgattttaacgccagcactcaccgtggcattatcggagagtcgctcacaaggctcggggcgatgttttctggtaaagagtaccagatactgcttcctggtgaaattcacattaaagaaagtggtaagcgataa

SEQ ID NO: 62 - protein, 387 aa, Escherichia coli
MGSNGADNAHNNAFGGGKNPGIGNTSGAGSNGSASSNRGNSNGWSWSNKPHKNDGFHSDGSYHITFHGDNNSKPKPGGNSGNRGNNGDGASAKVGEITITPDNSKPGRYISSNPEYSLLAKLIDAESIKGTEVYTFHTRKGQYVKVTVPDSNIDKMRVDYVNWKGPKYNNKLVKRFVSQFLLFRKEEKEKNEKEALLKASELVSGMGDKLGEYLGVKYKNVAKEVANDIKNFHGRNIRSYNEAMASLNKVLANPKMKVNKSDKDAIVNAWKQVNAKDMANKIGNLGKAFKVADLAIKVEKIREKSIEGYNTGNWGPLLLEVESWIIGGVVAGVAISLFGAVLSFLPISGLAVTALGVIGIMTISYLSSFIDANRVSNINNIISSVIR

SEQ ID NO: 63 - DNA, 51 bp, Escherichia coli
gcaaatcgagtttcgaatataaataacattatatctagtgttattcgatga

SEQ ID NO: 64 - protein, 103 aa, Escherichia coli
MRTLTLNELDSVSGGASGRDIAMAIGTLSGQFVAGGIGAAAGGVAGGAIYDYASTHKPNPAMSPSGLGGTIKQKPEGIPSEAWNYAAGRLCNWSPNNLSDVCL

SEQ ID NO: 65 - DNA, 312 bp, Escherichia coli
atgagaactctgactctaaatgaattagattctgtttctggtggtgcttcagggcgtgatattgcgatggctataggaacactatccggacaatttgttgcaggaggaattggagcagctgctgggggtgtggctggaggtgcaatatatgactatgcatccactcacaaacctaatcctgcaatgtctccatccggtttaggaggaacaattaagcaaaaacccgaagggataccttcagaagcatggaactatgctgcgggaagattgtgtaattggagtccaaataatcttagtgatgtttgtttataa

SEQ ID NO: 66 - protein, 58 aa, Enterococcus columbae
MMNATENQIFVETVSDQELEMLIGGAGRGWIKTLTKDCPNVISSICAGTIITACKNCA

SEQ ID NO: 67 - DNA, 177 bp, Enterococcus columbae
atgatgaatgctactgaaaaccaaatttttgttgagactgtgagtgaccaagaattagaaatgttaattggtggtgcaggtcgtggatggattaagactttaacaaaagattgtccaaatgtgatttcttcaatttgtgcaggtacaattattacagcttgtaaaaattgtgcttaa

SEQ ID NO: 68 - protein, 59 aa, Lactobacillus curvatus
MNNVKELSMTELQTITGGARSYGNGVYCNNKKCWVNRGEATQSIIGGMISGWASGLAGM

SEQ ID NO: 69 - DNA, 180 bp, Lactobacillus curvatus
atgaataatgtaaaagaattaagtatgacagaattacaaacaattaccggcggtgctagatcatatggcaacggtgtttactgtaataataaaaaatgttgggtaaatcggggtgaagcaacgcaaagtattattggtggtatgattagcggctgggctagtggtttagctggaatgtaa

SEQ ID NO: 70 - protein, 64 aa, Streptomyces sp.
MRSEMTLTSTNSAEALAAQDFANTVLSAAAPGFHADCETPAMATPATPTVAQFVIQGSTICLVC

SEQ ID NO: 71 - DNA, 195 bp, Streptomyces sp.
gtgcgatctgagatgactcttacgagcacgaattccgctgaggctctggcggcgcaggactttgcgaacaccgttctcagcgcggcggccccgggcttccacgcggactgcgagacgccggccatggccaccccggccacgccgaccgtcgcccagttcgtgatccagggcagcacgatctgcctggtctgctga

SEQ ID NO: 72 - protein, 65 aa, Bacillus halodurans
MVNSKDLRNPEFRKAQGLQFVDEVNEKELSSLAGSGDVHAQTTWPCATVGVSVALCPTTKCTSQC

SEQ ID NO: 73 - DNA, 198 bp, Bacillus halodurans
atggtaaattcaaaagatttgcgtaatcctgaattccgcaaagcccaaggtctacaattcgttgacgaggtgaacgagaaggaactttcgtctctagctggttcaggagatgtgcatgcacaaacaacttggccttgcgctacagttggtgtctccgtagccttgtgcccaactacaaagtgtacaagccagtgctaa

SEQ ID NO: 74 - protein, 66 aa, Carnobacterium divergens
MKNLKEGSYTAVNTDELKSINGGTKYYGNGVYCNSKKCWVDWGQASGCIGQTVVGGWLGGAIPGKC

SEQ ID NO: 75 - DNA, 201 bp, Carnobacterium divergens
atgaaaaacttaaaagaaggttcatacactgctgttaatactgatgaattaaaaagtatcaatggtggaacaaaatattatgggaatggcgtttattgcaattctaaaaaatgttgggtagattggggacaagcttcaggttgtatcggtcaaactgttgttggcggatggctaggcggagctataccaggtaaatgctaa

SEQ ID NO: 76 - protein, 63 aa, Carnobacterium divergens
MIKREKNRTISSLGYEEISNHKLQEIQGGKGILGKLGVVQAGVDFVSGVWAGIKQSAKDHPNA

SEQ ID NO: 77 - DNA, 192 bp, Carnobacterium divergens
atgattaaaagagaaaagaacagaacaatttcttcccttggttatgaagaaatttctaatcataaattgcaagaaatacaaggtggaaaaggaattcttggtaaactaggagtagtacaggcaggagtggattttgtatcaggagtgtgggctggaataaaacagtctgccaaagatcatcctaatgcgtaa

SEQ ID NO: 78 - protein, 75 aa, Carnobacterium divergens
MKKQILKGLVIVVCLSGATFFSTPQQASAAAPKITQKQKNCVNGQLGGMLAGALGGPGGVVLGGIGGAIAGGCFN

SEQ ID NO: 79 - DNA, 228 bp, Carnobacterium divergens
atgaaaaaacaaattttaaaagggttggttatagttgtttgtttatctggggcaacatttttctcaacaccacaacaagcttctgctgctgcaccgaaaattactcaaaaacaaaaaaattgtgttaatggacaattaggtggaatgcttgctggagctttgggtggacctggcggagttgtgttaggtggtataggtggtgcaatagcaggaggttgttttaattaa

SEQ ID NO: 80 - protein, 72 aa, Enterococcus durans
MQTIKELNTMELQEIIGGENDHRMPYELNRPNNLSKGGAKCAAGILGAGLGAVGGGPGGFISAGISAVLGCM

SEQ ID NO: 81 - DNA, 219 bp, Enterococcus durans
atgcaaacgatcaaagaattgaacacgatggaattacaagaaataattggaggtgaaaatgaccatcggatgccttacgaattgaaccgtccaaataatttatccaaaggtggggctaagtgtgctgctggaatacttggcgctggactaggcgcagtaggcggtggacctggcggatttattagtgccggaatcagtgctgttcttggttgtatgtaa

SEQ ID NO: 82 - protein, 72 aa, Enterococcus durans
MQTIKELNTMELQKIIGGENDHRMPYELNRPNNLSKGGAKCAAGILGAGLGAVGGGPGGFISAGISAVLGCM

SEQ ID NO: 83 - DNA, 219 bp, Enterococcus durans
atgcaaacgatcaaagaattgaacacgatggaattacaaaaaataattggaggtgaaaatgaccatcggatgccttacgaattgaaccgtccaaataatttatccaaaggtggagctaagtgcgctgccggaatacttggtgctggattaggcgcagtaggcggtggacctggcggatttattagtgccggaatcagtgctgttcttggttgtatgtaa

SEQ ID NO: 84 - protein, 220 aa, Streptococcus dysgalactiae subsp. equisimilis
MKKLKRLVISLVTSLLVISSTVPALVYANETNNFAETQKEITTNSEATLTNEDYTKLTSEVKTIYTNLIQYDQTKNKFYVDEDKTEQYYNYDDESIKGVYLMKDSLNDELNNNNSSNYSEIINQKISEIDYVLQGNDINNLIPSNTRVKRSADFSWIQRCLEEAWGYAISLVTLKGIINLFKAGKFEAAAAKLASATAGRIAGMAALFAFVATCGATTVS

SEQ ID NO: 85 - DNA, 663 bp, Streptococcus dysgalactiae subsp. equisimilis
atgaaaaaattaaaacgtcttgttatctctcttgttacttcattactagtaatttcaagtacagttccagcacttgtttacgctaatgaaacaaataactttgcagaaactcaaaaagaaattacaacaaattcagaagcaacattaaccaatgaagactacactaaattaacttccgaagtaaaaacaatttatacaaatctgattcaatacgaccaaacaaaaaacaaattttacgtcgatgaagacaaaactgaacaatattataactacgatgatgaaagtataaaaggggtttatctcatgaaagatagtttgaacgatgagttaaacaataataactcttcaaactattctgaaataattaatcaaaaaatctctgaaattgactatgtccttcaaggaaacgatataaataatttaattcctagcaataccagagtaaaaagatcagcagatttttcttggattcaaagatgtctagaagaagcatggggatatgctattagtctagttactctaaaaggaataatcaatctatttaaagcaggaaaatttgaagctgctgctgctaaattagcttctgctacagcaggtagaatcgctggaatggctgccttatttgctttcgtagcaacttgcggtgcgacaactgtatcataa

SEQ ID NO: 86 - protein, 57 aa, Enterococcus faecalis
MKQYKVLNEKEMKKPIGGESVFSKIGNAVGPAAYWILKGLGNMSDVNQADRINRKKH

SEQ ID NO: 87 - DNA, 174 bp, Enterococcus faecalis
atgaagcaatataaagtattgaatgaaaaagaaatgaaaaaacctattgggggagagtcggtttttagtaaaataggtaatgctgtaggtccagctgcttattggattttaaaaggattaggtaatatgagtgatgtaaaccaagctgatagaattaatagaaagaaacattaa

SEQ ID NO: 88 - protein, 44 aa, Enterococcus faecalis
MGAIAKLVAKFGWPIVKKYYKQIMQFIGEGWAINKIIDWIKKHI

SEQ ID NO: 89 - DNA, 135 bp, Enterococcus faecalis
atgggagcaatcgcaaaattagtagcaaagtttggatggccaattgttaaaaagtattacaaacaaattatgcaatttattggagaaggatgggcaattaacaaaattattgattggatcaaaaaacatatttaa

SEQ ID NO: 90 - protein, 43 aa, Enterococcus faecalis
MGAIAKLVAKFGWPFIKKFYKQIMQFIGQGWTIDQIEKWLKRH

SEQ ID NO: 91 - DNA, 132 bp, Enterococcus faecalis
atgggagcaatcgcaaaattagtagcaaagtttggatggccatttattaaaaaattctacaaacaaattatgcagtttatcggacaaggatggacaatagatcaaattgaaaaatggttaaaaagacattga

SEQ ID NO: 92 - protein, 74 aa, Enterococcus faecalis
MLNKKLLENGVVNAVTIDELDAQFGGMSKRDCNLMKACCAGQAVTYAIHSLLNRLGGDSSDPAGCNDIVRKYCK

SEQ ID NO: 93 - DNA, 225 bp, Enterococcus faecalis
atgttaaataaaaaattattagaaaatggtgtagtaaatgctgtaacaattgatgaacttgatgctcaatttggtggaatgagcaaacgtgattgtaacttgatgaaggcgtgttgtgctggacaagcagtaacatatgctattcatagtcttttaaatcgattaggtggagactctagtgatccagctggttgtaatgatattgtaagaaaatattgtaaataa

SEQ ID NO: 94 - protein, 65 aa, Enterococcus faecium
MKHLKILSIKETQLIYGGTTHSGKYYGNGVYCTKNKCTVDWAKATTCIAGMSIGGFLGGAIPGKC

SEQ ID NO: 95 - DNA, 195 bp, Enterococcus faecium
atgaaacatttaaaaattttgtctattaaagagacacaacttatctatgggggtaccactcatagtggaaaatattatggaaatggagtgtattgcactaaaaataaatgtacggtcgattgggccaaggcaactacttgtattgcaggaatgtctataggtggttttttaggtggagcaattccagggaagtgc

SEQ ID NO: 96 - protein, 105 aa, Enterococcus faecalis
MVKENKFSKIFILMALSFLGLALFSASLQFLPIAHMAKEFGIPAAVAGTVLNVVEAGGWVTTIVSILTAVGSGGLSLLAAAGRESIKAYLKKEIKKKGKRAVIAW

SEQ ID NO: 97 - DNA, 318 bp, Enterococcus faecalis
atggttaaagaaaataaattttctaagatttttattttaatggctttgagttttttggggttagccttgtttagtgcaagtcttcagtttttgcccattgcacatatggctaaagagttcggtataccagcagcagttgcaggaactgtgcttaatgtagttgaagctggtggatgggtcactactattgtatcaattcttactgctgtaggtagcggaggtctttctttactcgctgcagcaggaagagagtcaattaaagcataccttaagaaagaaattaagaaaaaaggaaaaagagcagttattgcttggtaa

SEQ ID NO: 98 - protein, 71 aa, Enterococcus faecium
MQNVKELSTKEMKQIIGGENDHRMPNELNRPNNLSKGGAKCGAAIAGGLFGIPKGPLAWAAGLANVYSKCN

SEQ ID NO: 99 - DNA, 216 bp, Enterococcus faecium
atgcaaaatgtaaaagaattaagtacgaaagagatgaaacaaattatcggtggagaaaatgatcacagaatgcctaatgagttaaatagacctaacaacttatctaaaggtggagcaaaatgtggtgctgcaattgctgggggattatttggaatcccaaaaggaccactagcatgggctgctgggttagcaaatgtatactctaaatgcaactaa

SEQ ID NO: 100 - protein, 58 aa, Enterococcus mundtii
MKKLTSKEMAQVVGGKYYGNGVSCNKKGCSVDWGKAIGIIGNNSAANLATGGAAGWKS

SEQ ID NO: 101 - DNA, 177 bp, Enterococcus mundtii
ttgaagaaattaacatcaaaagaaatggcacaagtagtaggtggaaaatactacggtaatggagtctcatgtaataaaaaagggtgcagtgttgattggggaaaagctattggcattattggaaataattctgctgcgaatttagctactggtggagcagctggttggaaaagttaa

SEQ ID NO: 102 - protein, 44 aa, Enterococcus faecalis
MLAKIKAMIKKFPNPYTLAAKLTTYEINWYKQQYGRYPWERPVA

SEQ ID NO: 103 - DNA, 135 bp, Enterococcus faecalis
atgttagcaaaaattaaagcgatgattaagaagtttccgaacccttatactttagcagctaagctaacgacttacgaaattaattggtataaacaacaatacggtcgttatccttgggagcgccctgtagcataa

SEQ ID NO: 104 - protein, 71 aa, Enterococcus faecium
MRKKLFSLALIGIFGLVVTNFGTKVDAATRSYGNGVYCNNSKCWVNWGEAKENIAGIVISGWASGLAGMGH

SEQ ID NO: 105 - DNA, 216 bp, Enterococcus faecium
atgagaaaaaaattatttagtttagctcttattggaatatttgggttagttgtgacaaattttggtacaaaagttgatgcagctacgcgttcatatggtaatggtgtttattgtaataatagtaaatgctgggttaactggggagaagctaaagagaatattgcaggaatcgttattagtggctgggcttctggtttggcaggtatgggacattaa

SEQ ID NO: 106 - protein, 34 aa, Enterococcus faecium
MNFLKNGIAKWMTGAELQAYKKKYGCLPWEKISC

SEQ ID NO: 107 - DNA, 105 bp, Enterococcus faecium
atgaattttcttaaaaatggtatcgcaaaatggatgaccggtgctgaattgcaagcgtataaaaagaaatatggatgcttgccatgggaaaaaatttcttgttaa

SEQ ID NO: 108 - protein, 76 aa, Enterococcus faecalis
MKKKLVKGLVICGMIGIGFTALGTNVEAATYYGNGVYCNKQKCWVDWSRARSEIIDRGVKAYVNGFTKVLGGIGGR

SEQ ID NO: 109 - DNA, 231 bp, Enterococcus faecalis
atgaaaaagaaattagttaaaggcttagttatttgtggcatgattgggattggttttacagcattaggaacaaatgtagaagccgccacgtattacggaaatggtgtctattgcaataagcaaaaatgttgggtagattggagtagagcacgttctgaaattatagacagaggcgtaaaagcatacgtcaatggatttacgaaagtgttaggtggtataggtggaagataa

SEQ ID NO: 110 - protein, 60 aa, Enterococcus faecalis
MKKEELVGMAKEDFLNVICENDNKLENSGAKCPWWNLSCHLGNDGKICTYSHECTAGCNA

SEQ ID NO: 111 - DNA, 183 bp, Enterococcus faecalis
atgaaaaaagaagaattagtaggaatggctaaggaagactttttaaatgttatttgtgaaaatgacaacaaactagaaaatagtggagcaaaatgtccttggtggaatctttcttgtcatttaggcaatgatggtaaaatttgcacttattcacatgaatgtaccgcaggttgtaatgcataa

SEQ ID NO: 112 - protein, 61 aa, Enterococcus faecalis
MTELNKRLQLKRDVSTENSLKKISNTDETHGGVTTSIPCTVMVSAAVCPTLVCSNKCGGRG

SEQ ID NO: 113 - DNA, 186 bp, Enterococcus faecalis
atgactgaacttaacaaaagattacaattaaaaagagatgtttcaacagaaaatagtttgaaaaaaatttctaatactgatgaaacacatgggggagttactacatcaattccatgtacagtaatggttagtgcggcagtatgtcctacccttgtttgctcgaataaatgtggcggtagaggctag

SEQ ID NO: 114 - protein, 58 aa, Enterococcus faecium
MQNVKEVSVKEMKQIIGGSNDSLWYGVGQFMGKQANCITNHPVKHMIIPGYCLSKILG

SEQ ID NO: 115 - DNA, 177 bp, Enterococcus faecium
atgcaaaatgtaaaagaagtttctgtaaaagagatgaaacaaattatcggtggttctaatgatagtctttggtatggtgtaggacaatttatgggtaaacaagcaaactgtataacaaaccatcctgttaaacacatgataattcctggatattgtttatcgaaaattttagggtaa

SEQ ID NO: 116 - protein, 55 aa, Enterococcus faecium
MKKYNELSKKELLQIQGGIAPIIVAGLGYLVKDAWDHSDQIISGFKKGWNGGRRK

SEQ ID NO: 117 - DNA, 168 bp, Enterococcus faecium
atgaaaaaatataatgagttatctaaaaaagaacttctacagattcaaggaggaatagcacctattatagttgctggccttggctatttagtaaaagatgcatgggatcactcagatcaaataatctcaggatttaaaaaaggttggaatggtggacgtagaaaataa

SEQ ID NO: 118 - protein, 343 aa, Enterococcus faecalis
MKNILLSILGVLSIVVSLAFSSYSVNAASNEWSWPLGKPYAGRYEEGQQFGNTAFNRGGTYFHDGFDFGSAIYGNGSVYAVHDGKILYAGWDPVGGGSLGAFIVLQAGNTNVIYQEFSRNVGDIKVSTGQTVKKGQLIGKFTSSHLHLGMTKKEWRSAHSSWNKDDGTWFNPIPILQGGSTPTPPNPGPKNFTTNVRYGLRVLGGSWLPEVTNFNNTNDGFAGYPNRQHDMLYIKVDKGQMKYRVHTAQSGWLPWVSKGDKSDTVNGAAGMPGQAIDGVQLNYITPKGEKLSQAYYRSQTTKRSGWLKVSADNGSIPGLDSYAGIFGEPLDRLQIGISQSNPF

SEQ ID NO: 119 - DNA, 1032 bp, Enterococcus faecalis
atgaaaaatattttactttctattctaggggtattatctatcgttgtttctttggcgttttcttcttattctgtcaacgcagcttctaatgagtggtcgtggccactgggcaaaccatatgcgggaagatatgaagaaggacaacaattcgggaacactgcatttaaccgaggaggtacttatttccatgatgggtttgactttggttctgctatttatggaaatggcagtgtgtatgctgtgcatgatggtaaaattttatatgctggttgggatcctgtaggtggaggctcattaggtgcatttattgtactacaagcgggaaacacaaatgtgatttatcaagaatttagccgaaatgttggagatattaaagttagcactggacaaactgttaaaaaaggacagctgataggaaagtttacttctagtcatttacatttaggaatgacaaaaaaagaatggcgttctgctcattcttcttggaataaagatgatggcacttggtttaacccaattcctatacttcaaggaggatctacgcctacgcctccaaatccaggaccaaaaaatttcacaacaaatgttcgttacggattgcgggtcctcggaggttcatggttaccagaagtaaccaactttaacaataccaatgatggtttcgcaggttaccctaatcgtcaacatgatatgctttatataaaggtagataaagggcaaatgaaatatcgtgttcacacggctcaaagtggatggttgccttgggtaagtaaaggggataagagcgatacagtaaatggagcggcaggtatgcctggacaagcaattgatggtgttcagctaaactatataactcctaagggagaaaaattatcacaggcttactatcgttcacaaactacgaaacgatcaggctggttaaaagtaagtgcagataatggttctattcctggactagacagttatgcaggaatctttggagaaccgttggatcgcttgcaaataggtatttcacagtcaaatccattttaa

SEQ ID NO: 120 - protein, 56 aa, Staphylococcus epidermidis
MENKKDLFDLEIKKDNMENNNELEAQSLGPAIKATRQVCPKATRFVTVSCKKSDCQ

SEQ ID NO: 121 - DNA, 171 bp, Staphylococcus epidermidis
atggaaaacaaaaaagatttatttgatttagaaatcaaaaaagataatatggaaaataataatgaattagaagctcaatctcttggtcctgcaattaaggcaactagacaggtatgtcctaaagcaacacgttttgttacagtttcttgtaaaaaaagtgattgtcaatag

SEQ ID NO: 122 - protein, 51 aa, Staphylococcus epidermidis
MAAFMKLIQFLATKGQKYVSLAWKHKGTILKWINAGQSFEWIYKQIKKLWA

SEQ ID NO: 123 - DNA, 156 bp, Staphylococcus epidermidis
atggcagcatttatgaagttaattcagttcttagcaactaaaggtcaaaagtatgtttcacttgcatggaaacataaaggtactattttaaaatggattaacgccggtcaaagttttgaatggatttataaacaaatcaaaaaattatgggcataa

SEQ ID NO: 124 - protein, 52 aa, Staphylococcus epidermidis
MEAVKEKNDLFNLDVKVNAKESNDSGAEPRIASKFICTPGCAKTGSFNSYCC

SEQ ID NO: 125 - DNA, 159 bp, Staphylococcus epidermidis
atggaagcagtaaaagaaaaaaatgatctttttaatcttgatgttaaagttaatgcaaaagaatctaacgattcaggagctgaaccaagaattgctagtaaatttatatgtactcctggatgtgcaaaaacaggtagttttaacagttattgttgttaa

SEQ ID NO: 126 - protein, 55 aa, Staphylococcus epidermidis
MNNSLFDLNLNKGVETQKSDLSPQSASVLKTSIKVSKKYCKGVTLTCGCNITGGK

SEQ ID NO: 127 - DNA, 168 bp, Staphylococcus epidermidis
atgaataactcattattcgatttaaacctaaacaaaggtgtagaaactcaaaagagtgatttaagtccgcaatctgctagtgtcttgaagacttctattaaagtatctaaaaaatattgtaaaggtgttactttaacatgcggttgcaatattactggtggtaaataa

SEQ ID NO: 128 - protein, 52 aa, Staphylococcus gallinarum
MEAVKEKNELFDLDVKVNAKESNDSGAEPRIASKFLCTPGCAKTGSFNSYCC

SEQ ID NO: 129 - DNA, 159 bp, Staphylococcus gallinarum
atggaagcagtaaaagagaaaaatgaactttttgatcttgacgttaaagtaaatgcaaaagagtctaatgattcaggcgcagaaccacgaattgctagtaaatttttatgtactcctggatgtgccaaaacaggtagcttcaatagctactgttgttaa

SEQ ID NO: 130 - protein, 63 aa, Lactococcus garvieae
MENNNYTVLSDEELQKIDGGIGGALGNALNGLGTWANMMNGGGFVNQWQVYANKGKINQYRPY

SEQ ID NO: 131 - DNA, 192 bp, Lactococcus garvieae
atggaaaacaacaattacacagtactttcagatgaagaactacaaaaaattgatggtggaatcggcggggctcttggtaatgctctcaacggattaggtacctgggcaaacatgatgaacggtggaggatttgttaatcagtggcaagtttatgctaataaaggaaaaataaatcaataccgtccgtattaa

SEQ ID NO: 132 - protein, 63 aa, Lactococcus garvieae
MFDLVATGMAAGVAKTIVNAVSAGMDIATALSLFSGAFTAAGGIMALIKKYAQKKLWKQLIAA

SEQ ID NO: 133 - DNA, 192 bp, Lactococcus garvieae
atgtttgatttagtcgcgactggaatggctgcaggtgtagcaaaaactattgttaatgccgttagtgctggtatggatattgccactgctttatcattgttctcaggagcttttactgcagctgggggaattatggcactcattaaaaaatatgctcaaaagaaattatggaaacagcttattgctgcataa

SEQ ID NO: 134 - protein, 91 aa, Lactobacillus gasseri
MVTKYGRNLGLNKVELFAIWAVLVVALLLTTANIYWIADQFGIHLATGTARKLLDAMASGASLGTAFAAILGVTLPAWALAAAGALGATAA

SEQ ID NO: 135 - DNA, 276 bp, Lactobacillus gasseri
atggttactaagtacggacgtaatttaggtttgaacaaggtagagttgtttgcaatttgggcggttttagtagttgctcttttattgaccacagcgaacatttattggattgctgatcaattcgggattcatttagcgactggaacagcccgtaagttattagatgcaatggcttctggtgcctcattgggaactgcctttgctgctattttgggcgtgacattacctgcatgggctttggcagctgcaggagcattgggagcgactgcagcctag

SEQ ID NO: 136 - protein, 75 aa, Lactobacillus gasseri
MKNFNTLSFETLANIVGGRNNWAANIGGVGGATVAGWALGNAVCGPACGFVGAHYVPIAWAGVTAATGGFGKIRK

SEQ ID NO: 137 - DNA, 228 bp, Lactobacillus gasseri
atgaaaaattttaatacattatcatttgaaacattggctaacatagttggtgggagaaataattgggctgctaatataggtggagtaggtggagcgacagtcgctggatgggctcttggaaatgcagtttgcggtcctgcttgtggctttgttggagcacactatgttccaatagcatgggctggcgtaacggcagctactggtggattcggaaagataagaaagtag

SEQ ID NO: 138 - protein, 64 aa, Lactobacillus plantarum
MSKLVKTLTISEISKAQNNGGKPAWCWYTLAMCGAGYDSGTCDYMYSHCFGIKHHSSGSSSYHC

SEQ ID NO: 139 - DNA, 195 bp, Lactobacillus plantarum
atgagtaaattggttaagacacttactataagtgaaatttctaaggctcaaaacaacggtggaaaacctgcatggtgttggtatactttagcaatgtgtggtgctggttatgattcgggaacctgtgattatatgtattcgcattgttttggtataaagcatcatagtagtggtagtagcagttatcattgttag

SEQ ID NO: 140 - protein, 359 aa, Haloferax mediterranei
MSKDRDGRRTSRRGTLKKIGGFSLGALSFGAVGRTQAATGSSVTTADIAPPGPNGDPKSVQIDDKYTGAEMYGEGDFRVGLGTDLTMYPPVYRESLGNGSGGWEFDFTVCGSTACRFVDSNGDVKEDDKAKEMWWQEINFNDINQDLYSRNDSDWVGSTPADTQPEFDYTEFALARDGVTLALTALNPAMGSLALGATYFLSDMVNWIASQHEDDSSLKRKWDYDGLSGPLYADSSTYLLARDEMTSNSYESFTIDNIAVAFPEFPVRTKYYVTFTAPDDPSTQSISTLEEEGIYRVPATEVAAARPPGSRRSKSAADEMVYVADPKKFIEVEPVKNPSIPDRIYEEIEQKKKQRSRKQ

SEQ ID NO: 141 - DNA, 1080 bp, Haloferax mediterranei
atgtcgaaagacagagatgggagaaggacaagtcggcgaggcacgttaaagaaaatcggcggtttcagtctcggagcgcttagtttcggggcagtcggacgaactcaagcggcgaccggctcatcggttacgaccgctgatatcgcacctcccggaccgaacggagacccgaagagtgttcagatagatgataaatacaccggagccgagatgtacggcgagggtgacttcagagtcggtctcggaactgacctgacgatgtatccgcccgtgtaccgtgagagtcttggaaatggaagcgggggttgggaattcgacttcaccgtttgtgggtccactgcctgtcgatttgtggacagtaacggtgacgtcaaagaggacgacaaggcgaaagaaatgtggtggcaggaaattaacttcaacgacataaatcaggatttatacagtcggaacgattccgactgggtcgggtcgacccctgccgatacccaaccggagttcgattacaccgactttgcgctcgctcgggacggagtgacgctcgctctcacggcactcaaccccgcaatggggagtcttgcactcggtgccacgtacttcctcagcgacatggtgaactggattgcgagccagcacgaagacgacagttcgctcaagagaaaatgggattacgacgggctaagtgggccgttgtacgccgattcgtcgacgtacctactggcacgcgacgagatgacttcgaactcgtacgaatcattcacgatcgataacatcgccgttgccttcccagagttccccgtccggaccaagtactacgtcacattcactgcgccggatgacccgtcaacgcagtcgatatctacgctcgaagaggagggaatctaccgagtgcccgctacggaagtggctgcggccagaccaccggggtcccgacgttccaaatcggcagccgacgagatggtgtacgttgccgatccgaagaagttcatagaggtcgagccggtgaagaacccaagtatcccggaccgaatctacgaggagatagagcaaaaaaagaaacaacggagtaggaaacagtag

SEQ ID NO: 142 - protein, 311 aa, Haloarchaeon S8a
MSDKDSINRRNVLRKIGGIGVASAVGFSGLASGESLSDDEKQDVIDTIYKSQRVEQIKKKFGGVNIEPKKVQSVTTNQSGDLVTAKLSVSDGDLVYSSVKDTTVIVQFDRSASEIGESWPKNTEAFIKSTSSGVDLLRTATDEEIKDVTEGVNTSEIESADAVNIFIDPESQTYYMEKYDFNNKVLEMFELATGGTSSGKISPTREDQNHEYNVREHKVFNSEKQNIQLQSDCNINSNTAADVILCFNQVGSCALCSPTLVGGPVPTVACLLVVCFGTPNAVSAILEEVDNSCFNLIKDVISCWDEWTSFW

SEQ ID NO: 143 - DNA, 936 bp, Haloarchaeon S8a
atgtcggataaagacagcattaacagaagaaatgtattaagaaaaattggcggtatcggtgtggcttcagctgtcggattttctggtttggcaagcggggaaagtcttagcgatgatgagaaacaagatgttattgacacaatttacaaatcacaaagagttgaacagataaagaaaaagttcggaggagtgaatattgagccgaaaaaggttcaatctgtaacgaccaatcagagcggagatcttgttacggcgaagctgtcggttagtgatggggatttggtatattcgagtgtcaaagatacaactgtaatagttcagttcgatagatcggcttctgaaattggtgaaagttggcccaagaatactgaggcattcatcaaatcgacgtcctctggggtcgatcttctacgtacagcaactgatgaagaaataaaggacgttactgagggagtcaacacatctgaaattgaatctgcggatgctgttaacatatttattgatcctgaatcacagacatactatatggagaaatatgactttaataataaggtacttgagatgtttgaattagcgacaggtgggacaagtagtggtaaaatctcccccacacgtgaagaccagaatcacgaatataatgttagggaacataaagtatttaactcagaaaaacagaatatacaacttcagagtgactgtaatataaacagtaacaccgctgctgatgttattctatgcttcaaccaggttggttcttgtgcactctgctccccgactttagtcggaggtccagtccctacagttgcatgtctcttagtcgtctgtttcggcactccaaatgctgtgtccgcgatacttgaagaagtcgataattcttgctttaacttgatcaaggatgtaatttcgtgttgggatgaatggactagcttctggtga

SEQ ID NO: 144 - protein, 333 aa, Lactobacillus helveticus
MKHLNETTNVRILSQFDMDTGYQAVVQKGNVGSKYVYGLQLRKGATTILRGYRGSKINNPILELSGQAGGHTQTWEFAGDRKDINGEERAGQWFIGVKPSKIEGSKIIWAKQIARVDLRNQMGPHYSNTDFPRLSYLNRAGSNPFAGNKMTHAEAAVSPDYTKFLIATVENNCIGHFTIYNLDTINEKLDEKGNSEDVNLETVKYEDSFIIDNLYGDDNNSIVNSIQGYDLDNDGNIYISSQKAPDFDGSYYAHHKQIVKIPYYARSKESEDQWRAVNLSEFGGLDIPGKHSEVESIQIIGENHCYLTVAYHSKNKAGENKTTLNEIYELSWN

SEQ ID NO: 145 - DNA, 1002 bp, Lactobacillus helveticus
atgaagcatttaaatgaaacaactaatgttagaattttaagtcaatttgatatggatactggctatcaagcagtagttcaaaaaggcaatgtaggttcaaaatatgtatatggattacaacttcgcaaaggtgctactactatcttgcgtggttaccgtggaagtaaaattaataaccctattcttgaattatctggtcaagcaggtggtcacacacagacatgggaatttgctggtgatcgtaaagacattaatggtgaagaaagagcaggtcaatggtttataggtgttaaaccatcgaaaattgaaggaagcaaaattatttgggcaaagcaaattgcaagagttgatcttagaaatcaaatgggacctcattattcaaatactgactttcctcgattatcctacttgaatcgcgccggttctaatccatttgctggtaataagatgacgcatgccgaagccgcagtatcacctgattatactaagtttttaattgctactgttgaaaataactgtattggtcattttactatatacaatttagatacaattaatgaaaaacttgatgaaaagggaaatagtgaagatgttaatctcgaaactgttaaatacgaagatagttttatcattgataatttatatggtgatgataataattctattgtaaattcaattcaagggtatgatttggataatgatggaaatatttatatttccagtcaaaaagcgccagattttgatggctcttattatgcacatcataagcagattgttaagattccatattatgctcggtctaaagaaagcgaagaccaatggagagctgtaaatttaagcgaattcggtggcttggatattccaggtaaacatagtgaagttgaaagcatccaaattattggtgagaatcattgttacttaactgttgcatatcattctaaaaataaagcgggtgaaaataaaactactttgaatgagatttatgaattatcttggaattag

SEQ ID NO: 146 - protein, 74 aa, Enterococcus hirae; identical to SEQ ID NO: 20

SEQ ID NO: 147 - DNA, 225 bp, Enterococcus hirae; identical to SEQ ID NO: 21

SEQ ID NO: 148 - protein, 75 aa, Lactobacillus johnsonii
MKQFNYLSHKDLAVVVGGRNNWQTNVGGAVGSAMIGATVGGTICGPACAVAGAHYLPILWTAVTAATGGFGKIRK

SEQ ID NO: 149 - DNA, 228 bp, Lactobacillus johnsonii
atgaaacaatttaattatttatcacataaagatttagcagtcgttgttggtggaagaaataattggcaaacaaatgtgggaggagcagtgggatcagctatgattggggctacagttggtggtacaatttgtggacctgcatgtgctgtagctggtgcccattatcttcctattttatggacagcggttacagctgcaacaggtggttttggcaagataagaaagtag

SEQ ID NO: 150 - protein, 62 aa, Lactobacillus johnsonii
MKLNDKELSKIVGGNRWGDTVLSAASGAGTGIKACKSFGPWGMAICGVGGAAIGGYFGYTHN

SEQ ID NO: 151 - DNA, 189 bp, Lactobacillus johnsonii
atgaaattaaatgacaaagaattatcaaagattgttggtggaaatcgatggggagatactgttttatcagctgctagtggcgcaggaactggtattaaagcatgtaaaagttttggcccatggggaatggcaatttgtggtgtaggaggtgcagcaataggaggttattttggctatactcataattaa

SEQ ID NO: 152 - protein, 59 aa, Lactococcus lactis subsp. lactis
MNKNEIETQPVTWLEEVSDQNFDEDVFGACSTNTFSLSDYWGNNGAWCTLTHECMAWCK

SEQ ID NO: 153 - DNA, 180 bp, Lactococcus lactis subsp. lactis
atgaacaaaaatgaaattgaaacacaaccagttacatggttggaagaagtatctgatcaaaattttgatgaagatgtatttggtgcgtgtagtactaacacattctcgctcagtgattactggggaaataacggggcttggtgtacactcactcatgaatgtatggcttggtgtaaataa

SEQ ID NO: 154 - protein, 65 aa, Lactococcus lactis subsp. lactis
MKEKNMKKNDTIELQLGKYLEDDMIELAEGDESHGGTTPATPAISILSAYISTNTCPTTKCTRAC

SEQ ID NO: 155 - DNA, 198 bp, Lactococcus lactis subsp. lactis
atgaaagaaaaaaatatgaaaaagaatgacactattgaattacaattgggaaaataccttgaagatgatatgattgaattagctgaaggggatgagtctcatggaggaacaacaccagcaactcctgcaatctctattctcagtgcatatattagtaccaatacttgtccaacaacaaaatgtacacgtgcttgttaa

SEQ ID NO: 156 - protein, 51 aa, Lactococcus lactis subsp. lactis
MKEQNSFNLLQEVTESELDLILGAKGGSGVIHTISHECNMNSWQFVFTCCS

SEQ ID NO: 157 - DNA, 156 bp, Lactococcus lactis subsp. lactis
atgaaagaacaaaactcttttaatcttcttcaagaagtgacagaaagtgaattggaccttattttaggtgcaaaaggcggcagtggagttattcatacaatttctcatgaatgtaatatgaatagctggcaatttgtatttacttgctgctcttaa

SEQ ID NO: 158 - protein, 53 aa, Lactococcus lactis
MAGFLKVVQLLAKYGSKAVQWAWANKGKILDWLNAGQAIDWVVSKIKQILGIK

SEQ ID NO: 159 - DNA, 162 bp, Lactococcus lactis
atggcagggtttttaaaagtagttcaattactagctaaatatggttctaaagctgtacaatgggcttgggcaaacaagggtaagattttagattggcttaatgcaggtcaggctattgattgggtagtttcgaaaattaagcaaattttaggtattaagtaa

SEQ ID NO: 160 - protein, 53 aa, Lactococcus lactis
MAGFLKVVQILAKYGSKAVQWAWANKGKILDWINAGQAIDWVVEKIKQILGIK

SEQ ID NO: 161 - DNA, 162 bp, Lactococcus lactis
atggcagggtttttaaaagtagtccaaattttggctaagtatggttctaaagccgtacaatgggcatgggcaaataaaggaaaaatcttagattggattaatgcaggtcaagctattgactgggtagttgaaaagattaagcaaattttgggtattaaataa

SEQ ID NO: 162 - protein, 65 aa, Lactobacillus amylovorus
MKQLNSEQLQNIIGGNRWTNAYSAALGCAVPGVKYGKKLGGVWGAVIGGVGGAAVCGLAGYVRKG

SEQ ID NO: 163 - DNA, 198 bp, Lactobacillus amylovorus
atgaaacaattgaattcagaacaattacaaaatattatcggtggaaatagatggactaatgcatacagcgcagctttgggatgcgctgtccctggagttaaatatggaaaaaaacttggtggcgtatggggtgctgtaattggtggcgtaggcggtgcagcagtctgtggcttggcgggttatgttcgtaaaggctaa

SEQ ID NO: 164 - protein, 68 aa, Lactobacillus sakei L45
MKTEKKVLDELSLHASAKMGARDVESSMNADSTPVLASVAVSMELLPTASVLYSDVAGCFKYSAKHHC

SEQ ID NO: 165 - DNA, 207 bp, Lactobacillus sakei L45
atgaaaacagaaaaaaaggttttagatgaactgagcttacacgcttctgcaaaaatgggagcacgtgatgttgaatccagcatgaatgcagactcaacaccagttttagcatcagtcgctgtatccatggaattattgccaactgcgtctgttctttattcggatgttgcaggttgcttcaaatattctgcaaaacatcattgttag

SEQ ID NO: 166 - protein, 91 aa, Lactococcus lactis subsp. lactis
MKTKSLVLALSAVTLFSAGGIVAQAEGTWQHGYGVSSAYSNYHHGSKTHSATVVNNNTGRQGKDTQRAGVWAKATVGRNLTEKASFYYNFW

SEQ ID NO: 167 - DNA, 276 bp, Lactococcus lactis subsp. lactis
atgaaaaccaagtctctcgtattggcattatctgcggttacgttattctctgccggaggaattgtagctcaagctgaaggaacatggcaacatggatatggtgttagttcggcatattcaaattatcatcatggtagcaaaactcattcagccacagttgtaaataataatactggccgacaaggtaaggatacacaacgtgccggtgtttgggcaaaagctactgttggacgtaacttaactgaaaaagcttcattttattataacttttggtaa

SEQ ID NO: 168 - protein, 75 aa, Lactococcus lactis subsp. cremoris
MKNQLNFNIVSDEELSEANGGKLTFIQSTAAGDLYYNTNTHKYVYQQTQNAFGAAANTIVNGWMGGAAGGFGLHH

SEQ ID NO: 169 - DNA, 228 bp, Lactococcus lactis subsp. cremoris
atgaaaaatcaattaaattttaatattgtttcagatgaagaactttcagaagctaacggaggaaaattaacatttattcaatcgacagcggctggagatttatattacaatactaatacacacaaatatgtttaccaacaaactcaaaacgcttttggggctgctgctaataccattgttaatggatggatgggtggcgctgctggaggtttcgggttgcaccattga

SEQ ID NO: 170 - protein, 68 aa, Lactococcus lactis subsp. cremoris
MKNQLNFNIVSDEELAEVNGGSLQYVMSAGPYTWYKDTRTGKTICKQTIDTASYTFGVMAEGWGKTFH

SEQ ID NO: 171 - DNA, 207 bp, Lactococcus lactis subsp. cremoris
atgaaaaatcaattaaattttaatattgtttctgatgaagaacttgcagaagttaatggaggaagcttgcagtatgttatgagtgctggaccatatacttggtataaagatactagaacaggaaaaacaatatgtaaacagacaattgacacagcaagttatacatttggtgtaatggcagaaggatggggaaaaacattccactaa

SEQ ID NO: 172 - protein, 63 aa, Lactococcus sp. QU 12
MKLIDHLGAPRWAVDTILGAIAVGNLASWVLALVPGPGWAVKAGLATAAAIVKHQGKAAAAAW

SEQ ID NO: 173 - DNA, 192 bp, Lactococcus sp. QU 12
atgaaattaattgatcatttaggtgctccaagatgggccgttgatactattttaggtgcaatcgcagttgggaacttagcaagttgggttctagcgcttgtccctggtccagggtgggcagtaaaagctggtttagcaactgctgctgccatcgttaaacatcaaggtaaagctgccgctgctgcttggtaa

SEQ ID NO: 174 - protein, 50 aa, Brevibacillus sp. GI-9
MACQCPDAISGWTHTDYQCHGLENKMYRHVYAICMNGTQVYCRTEWGSSC

SEQ ID NO: 175 - DNA, 153 bp, Brevibacillus sp. GI-9
atggcttgccaatgtccagatgcgatctcaggttggacgcatacagattaccagtgtcacggtttggagaataaaatgtatagacatgtttatgcaatttgcatgaacggtactcaagtatattgcagaacagagtggggtagcagctgctag

SEQ ID NO: 176 - protein, 57 aa, Leuconostoc pseudomesenteroides
MNKEYNSISNFKKITNKDLQNINGGFIGRAIGDFVYFGAKGLRESGKLLNYYYKHKH

SEQ ID NO: 177 - DNA, 174 bp, Leuconostoc pseudomesenteroides
atgaataaagaatataatagcattagcaattttaaaaaaattactaataaagacttgcaaaacataaatggtggatttattggtagggcaataggtgactttgtgtactttggagcgaagggactaagagaatctggtaaactacttaattattactataagcataagcattga

SEQ ID NO: 178 - protein, 53 aa, Leuconostoc pseudomesenteroides
MKNQLMSFEVISEKELSTVQGGKGLGKLIGIDWLLGQAKDAVKQYKKDYKRWH

SEQ ID NO: 179 - DNA, 162 bp, Leuconostoc pseudomesenteroides
atgaaaaatcagttaatgtctttcgaagtgatatcagaaaaagaattgtccacggtacaaggtggcaaaggcttaggtaaactcataggaattgattggcttttgggtcaagctaaggacgctgttaaacagtacaagaaggattacaaacgttggcactaa

SEQ ID NO: 180 - protein, 61 aa, Leuconostoc gelidum
MMNMKPTESYEQLDNSALEQVVGGKYYGNGVHCTKSGCSVNWGEAFSAGVHRLANGGNGFW

SEQ ID NO: 181 - DNA, 186 bp, Leuconostoc gelidum
atgatgaacatgaaacctacggaaagctatgagcaattggataatagtgctctcgaacaagtcgtaggaggtaagtattatggtaacggagttcattgcacaaaaagtggttgttctgtaaactggggagaagccttttcagctggagtacatcgtttagcaaatggtggaaatggtttctggtaa

SEQ ID NO: 182 - protein, 61 aa, Leuconostoc carnosum
MNNMKSADNYQQLDNNALEQVVGGKYYGNGVHCTKSGCSVNWGEAFSAGVHRLANGGNGFW

SEQ ID NO: 183 - DNA, 186 bp, Leuconostoc carnosum
atgaataacatgaaatctgcggataattatcagcaattggataataatgctctcgaacaagtcgtaggaggtaagtattatggtaacggagttcattgcacaaaaagtggttgttctgtaaactggggagaagccttttcagctggagtacatcgtttagcaaatggtggaaatggtttctggtaa

SEQ ID NO: 184 - protein, 63 aa, Leuconostoc mesenteroides
MFLVNQLGISKSLANTILGAIAVGNLASWLLALVPGPGWATKAALATAETIVKHEGKAAAIAW

SEQ ID NO: 185 - DNA, 192 bp, Leuconostoc mesenteroides
atgttcttggtaaatcagttagggatttcaaaatcgttagctaatactattcttggtgcaattgctgttggtaatttggccagttggttattagctttggttcctggtccgggttgggcaacaaaagcagcacttgcgacagctgaaacaattgtgaagcatgaaggaaaagcagctgctattgcgtggtaa

SEQ ID NO: 186 - protein, 74 aa, Bacillus licheniformis
MSKKEMILSWKNPMYRTESSYHPAGNILKELQEEEQHSIAGGTITLSTCAILSKPLGNNGYLCTVTKECMPSCN

SEQ ID NO: 187 - DNA, 225 bp, Bacillus licheniformis
atgtcaaaaaaggaaatgattctttcatggaaaaatcctatgtatcgcactgaatcttcttatcatccagcagggaacatccttaaagaactccaggaagaggaacagcacagcatcgccggaggcacaatcacgctcagcacttgtgccatcttgagcaagccgttaggaaataacggatacctgtgtacagtgacaaaagaatgcatgccaagctgtaactaa

SEQ ID NO: 188 - protein, 266 aa, Brevibacterium linens
MNNLYRELAPIPGPAWAEIEEEARRTFKRNIAGRRIVDVAGPTGFETSAVTTGHIRDVQSETSGLQVKQRIVQEYIELRTPFTVTRQAIDDVARGSGDSDWQPVKDAATTIAMAEDRAILHGLDAAGIGGIVPGSSNAAVAIPDAVEDFADAVAQALSVLRTVGVDGPYSLLLSSAEYTKVSESTDHGYPIREHLSRQLGAGEIIWAPALEGALLVSTRGGDYELHLGQDLSIGYYSHDSETVELYLQETFGFLALTDESSVPLSL

SEQ ID NO: 189 - DNA, 801 bp, Brevibacterium linens
gtgaataacctctatcgcgagcttgcccccatccccggcccggcctgggcggagatcgaggaggaggctcgacggacattcaaacgcaatatcgccggccgccggatcgtcgatgtcgcagggcccacgggcttcgagacctccgcggtgaccactggccacatccgagacgtccagtcggagacgagcggactgcaggttaagcagcgcatcgtgcaggaatacatcgagctgcggaccccattcaccgtgactcggcaggccatcgatgacgtggcccgcgggtccggtgactcggactggcagcccgtcaaggatgcggccacgacgatcgcgatggctgaagatcgggccattctccacgggctcgatgcggccgggatcggcggaatcgttcccggcagctcgaatgccgcagtggccatccccgacgccgtcgaggacttcgcggacgccgtcgcccaggcgctgagtgtgctgcgcacggtgggagtcgacgggccctacagcctgttgctctcctccgcggagtacaccaaggtctccgagtccaccgaccacggctacccgatccgcgagcacctctcccggcagctcggcgccggagagatcatctgggcgcccgcgctcgaaggggcgctgctcgtctccacgcgcgggggtgactacgagctccacctcggccaggacctgtcgatcggttactacagccacgacagcgagaccgtcgaactctatctgcaggagaccttcggattcctcgcgctgaccgacgaatccagtgtgcctttgagcctctga

SEQ ID NO: 190 - protein, 71 aa, Listeria innocua
MKKAALKFIIVIAILGFSFSFFSIQSEAKSYGNGVQCNKKKCWVDWGSAISTIGNNSAANWATGGAAGWKS

SEQ ID NO: 191 - DNA, 216 bp, Listeria innocua
ttgaagaaggcagcgttaaaatttattattgttattgctattctaggtttcagtttttctttctttagcatacaatctgaagctaaatcttatggaaatggagttcagtgtaataagaaaaaatgttgggtagattggggtagtgctataagtactattggaaataattctgcagcgaattgggctacaggtggagcagctggttggaaaagctga

SEQ ID NO: 192 - protein, 68 aa, Bacillus sp.
MSQEAIIRSWKDPFSRENSTQNPAGNPFSELKEAQMDKLVGAGDMEAACTFTLPGGGGVCTLTSECIC

SEQ ID NO: 193 - DNA, 207 bp, Bacillus sp.
atgagtcaagaagctatcattcgttcatggaaagatcctttttcccgtgaaaattctacacaaaatccagctggtaacccattcagtgagctgaaagaagcacaaatggataagttagtaggtgcgggagacatggaagcagcatgtacttttacattgcctggtggcggcggtgtttgtactctaacttctgaatgtatttgttaa

SEQ ID NO: 194 - protein, 61 aa, Leuconostoc mesenteroides
MTNMKSVEAYQQLDNQNLKKVVGGKYYGNGVHCTKSGCSVNWGEAASAGIHRLANGGNGFW

SEQ ID NO: 195 - DNA, 186 bp, Leuconostoc mesenteroides
atgacgaatatgaagtctgtggaagcatatcagcaattagataaccagaatctcaagaaagttgttggtggaaagtattatgggaatggtgttcactgtacaaaaagtggatgctctgttaactggggagaagctgcctcagctggcatacatcgtttggccaatggtggaaatggattttggtaa

SEQ ID NO: 196 - protein, 68 aa, Clavibacter michiganensis subsp. michiganensis
MNDILETETPVMVSPRWDMLLDAGEDTSPSVQTQIDAEFRRVVSPYMSSSGWLCTLTIECGTIICACR

SEQ ID NO: 197 - DNA, 207 bp, Clavibacter michiganensis subsp. michiganensis
atgaacgacatcctcgagacggagacccccgtcatggtcagcccccggtgggacatgctgctcgacgcgggcgaggacaccagcccgtccgtccagacccagatcgacgcggagttccgtcgcgtcgtgagcccgtacatgtccagcagcggctggctctgcacgctcaccatcgaatgtggcaccatcatctgcgcgtgtcgctga

SEQ ID NO: 198 - protein, 69 aa, Escherichia coli
MELKASEFGVVLSVDALKLSRQSPLGVGIGGGGGGGGGGSCGGQGGGCGGCSNGCSGGNGGSGGSGSHI

SEQ ID NO: 199 - DNA, 207 bp, Escherichia coli
atggaattaaaagcgagtgaatttggtgtagttttgtccgttgatgctcttaaattatcacgccagtctccattaggtgttggcattggtggtggtggcggcggcggcggcggcggtagctgcggtggtcaaggtggcggttgtggtggttgcagcaacggttgtagtggtggaaacggtggcagcggcggaagtggttcacatatc

SEQ ID NO: 200 - protein, 7 aa, Escherichia coli
MRTGNAN

SEQ ID NO: 201 - DNA, 24 bp, Escherichia coli
atgcgtactggtaatgcaaactaa

SEQ ID NO: 202 - protein, 99 aa, Klebsiella pneumoniae
MREISQKDLNLAFGAGETDPNTQLLNDLGNNMAWGAALGAPGGLGSAALGAAGGALQTVGQGLIDHGPVNVPIPVLIGPSWNGSGSGYNSATSSSGSGS

SEQ ID NO: 203 - DNA, 300 bp, Klebsiella pneumoniae
atgagagaaattagtcaaaaggacttaaatcttgcttttggtgcaggagagaccgatccaaatactcaacttctaaacgaccttggaaataatatggcatggggtgctgctcttggcgctcctggcggattaggatcagcagctttgggggccgcgggaggtgcattacaaactgtagggcaaggattaattgaccatggtcctgtaaatgtccccatccctgtactcatcgggccaagctggaatggtagcggtagtggttataacagcgcaacatccagttccggtagtggtagttaa

SEQ ID NO: 204 - protein, 75 aa, Escherichia coli
MREITESQLRYISGAGGAPATSANAAGAAAIVGALAGIPGGPLGVVVGAVSAGLTTAIGSTVGSGSASSSAGGGS

SEQ ID NO: 205 - DNA, 228 bp, Escherichia coli
atgcgagaaataacagaatcacagttaagatatatttccggggcgggaggtgcgccagcgacttcagctaatgccgcaggtgctgcagctattgttggagctctcgccggaatacctggtggtccacttggggttgtagttggagccgtatctgccggtttgacaacagcaattggctcgaccgtgggaagtggtagtgccagttcttctgctggtggcggtagctaa

SEQ ID NO: 206 - protein, 58 aa, Escherichia coli
MIKHFHFNKLSSGKKNNVPSPAKGVIQIKKSASQLTKGGAGHVPEYFVGIGTPISFYG

SEQ ID NO: 207 - DNA, 177 bp, Escherichia coli
atgattaagcattttcattttaataaactgtcttctggtaaaaaaaataatgttccatctcctgcaaagggggttatacaaataaaaaaatcagcatcgcaactcacaaaaggtggtgcaggacatgtgcctgagtattttgtggggattggtacacctatatctttctatggctga

SEQ ID NO: 208 - protein, 90 aa, Escherichia coli
MYMRELDREELNCVGGAGDPLADPNSQIVRQIMSNAAWGPPLVPERFRGMAVGAAGGVTQTVLQGAAAHMPVNVPIPKVPMGPSWNGSKG

SEQ ID NO: 209 - DNA, 273 bp, Escherichia coli
atgtatatgagagagttagatagagaggaattaaattgcgttggtggggctggagatccgcttgcagatcctaattcccaaattgtaagacagataatgtctaatgcggcatggggcccgcctttggtgccagagcggtttaggggaatggctgttggagccgcaggtggggttacgcagacagttcttcaaggagcagcagctcatatgccggttaatgtccctatacctaaagttccgatgggaccctcatggaacggaagtaaaggataa

SEQ ID NO: 210 - protein, 50 aa, Enterococcus mundtii
MSQVVGGKYYGNGVSCNKKGCSVDWGKAIGIIGNNSAANLATGGAAGWKS

SEQ ID NO: 211 - DNA, 153 bp, Enterococcus mundtii
atgtcacaggtagtaggtggaaaatactacggtaatggagtctcatgtaataaaaaagggtgcagtgttgattggggaaaagcgattggcattattggaaataattctgctgcgaatttagctactggtggagcagctggttggaaaagttaa

SEQ ID NO: 212 - protein, 58 aa, Enterococcus mundtii
MKKLTSKEMAQVVGGKYYGNGLSCNKKGCSVDWGKAIGIIGNNSAANLATGGAAGWKS

SEQ ID NO: 213 - DNA, 177 bp, Enterococcus mundtii
ttgaagaaattaacatcaaaagaaatggcacaagtagtaggtgggaaatactacggtaatggattatcatgtaataaaaaagggtgcagtgttgattggggaaaagctattggcattattggaaataattctgctgcgaatttagctactggtggagcagctggttggaaaagttaa

SEQ ID NO: 214 - protein, 63 aa, Streptococcus mutans
MSNTQLLEVLGTETFDVQEDLFAFDTTDTTIVASNDDPDTRFKSWSLCTPGCARTGSFNSYCC

SEQ ID NO: 215 - DNA, 192 bp, Streptococcus mutans
atgtcaaacacacaattattagaagtccttggtactgaaacttttgatgttcaagaagatctctttgcttttgatacaacagatactactattgtggcaagcaacgacgatccagatactcgtttcaaaagttggagcctttgtacgcctggttgtgcaaggacaggtagtttcaatagttactgttgctga

SEQ ID NO: 216 - protein, 53 aa, Streptococcus mutans
MNKLNSNAVVSLNEVSDSELDTILGGNRWWQGVVPTVSYECRMNSWQHVFTCC

SEQ ID NO: 217 - DNA, 162 bp, Streptococcus mutans
atgaacaagttaaacagtaacgcagtagtttctttgaatgaagtttcagattctgaattggatactattttgggtggtaatcgttggtggcaaggtgttgtgccaacggtctcatatgagtgtcgcatgaattcatggcaacatgttttcacttgctgttaa

SEQ ID NO: 218 - protein, 57 aa, Lactococcus lactis subsp. lactis
MSTKDFNLDLVSVSKKDSGASPRITSISLCTPGCKTGALMGCNMKTATCHCSIHVSK

SEQ ID NO: 219 - DNA, 174 bp, Lactococcus lactis subsp. lactis
atgagtacaaaagattttaacttggatttggtatctgtttcgaagaaagattcaggtgcatcaccacgcattacaagtatttcgctatgtacacccggttgtaaaacaggagctctgatgggttgtaacatgaaaacagcaacttgtcattgtagtattcacgtaagcaaataa

SEQ ID NO: 220 - protein, 57 aa, Lactococcus lactis
MSTKDFNLDLVSVSKKDSGASPRITSISLCTPGCKTGALMGCNMKTATCNCSVHVSK

SEQ ID NO: 221 - DNA, 171 bp, Lactococcus lactis
atgagtacaaaagatttcaacttggatttggtatctgtttcgaagaaagattcaggtgcatcaccacgcattacaagtatttcgctatgtacacccggttgtaaaacaggagctctgatgggttgtaacatgaaaacagcaacttgtaattgtagcgttcacgtaagcaaa

SEQ ID NO: 222 - protein, 57 aa, Lactococcus lactis
MSTKDFNLDLVSVSKTDSGASTRITSISLCTPGCKTGVLMGCNLKTATCNCSVHVSK

SEQ ID NO: 223 - DNA, 174 bp, Lactococcus lactis
atgagtacaaaagatttcaacttagatttggtatctgtttcaaaaacagattctggcgcttcaacacgtattaccagcatttcgctttgtacaccaggttgtaaaacaggtgttctgatgggatgtaacctgaaaacagcaacttgtaattgtagcgttcacgtaagcaaataa

SEQ ID NO: 224 - protein, 55 aa, Streptococcus uberis
MNNEDFNLDLIKISKENNSGASPRITSKSLCTPGCKTGILMTCPLKTATCGCHFG

SEQ ID NO: 225 - DNA, 168 bp, Streptococcus uberis
atgaacaatgaagattttaatttggatctcatcaaaatctcaaaggaaaacaactcaggagcttcacctcgaataactagtaaatcattatgtactcctggatgtaagacgggtattttgatgacttgtccactaaaaactgcaacctgtggttgtcattttggataa

SEQ ID NO: 226 - protein, 57 aa, Lactococcus lactis subsp. lactis
MSTKDFNLDLVSVSKKDSGASPRITSISLCTPGCKTGALMGCNMKTATCNCSIHVSK

SEQ ID NO: 227 - DNA, 174 bp, Lactococcus lactis subsp. lactis
atgagtacaaaagattttaacttggatttggtatctgtttcgaagaaagattcaggtgcatcaccacgcattacaagtatttcgctatgtacacccggttgtaaaacaggagctctgatgggttgtaacatgaaaacagcaacttgtaattgtagtattcacgtaagcaaataa

SEQ ID NO: 228 - protein, 57 aa, Staphylococcus warneri
MENSKVMKDIEVANLLEEVQEDELNEVLGAKKKSGVIPTVSHDCHMNSFQFVFTCCS

SEQ ID NO: 229 - DNA, 174 bp, Staphylococcus warneri
atggaaaattctaaagttatgaaggacattgaagtagcaaatttattagaagaggttcaagaagatgaattgaatgaagtcttaggagctaagaaaaagtcaggagtaatcccaactgtgtcacacgattgccatatgaattctttccaatttgtatttacttgttgttcataa

SEQ ID NO: 230 - protein, 58 aa, Paenibacillus polymyxa
MAENLFDLDIQVNKSQGSVEPQVLSIVACSSGCGSGKTAASCVETCGNRCFTNVGSLC

SEQ ID NO: 231 - DNA, 177 bp, Paenibacillus polymyxa
atggctgaaaacttatttgatctggacattcaagtaaacaaatctcaaggttctgtagagcctcaggttctgagcattgttgcatgttctagcggatgtggtagcggtaaaacagctgccagttgtgttgaaacttgtggcaaccggtgctttactaacgttggttcactctgctaa

SEQ ID NO: 232 - protein, 62 aa, Pediococcus acidilactici
MKKIEKLTEKEMANIIGGKYYGNGVTCGKHSCSVDWGKATTCIINNGAMAWATGGHQGNHKC

SEQ ID NO: 233 - DNA, 189 bp, Pediococcus acidilactici
atgaaaaaaattgaaaaattaactgaaaaagaaatggccaatatcattggtggtaaatactacggtaatggggttacttgtggcaaacattcctgctctgttgactggggtaaggctaccacttgcataatcaataatggagctatggcatgggctactggtggacatcaaggtaatcataaatgctag

SEQ ID NO: 234 - protein, 60 aa, Pediococcus pentosaceus
MTEIKVLNDKELKNVVGGKYYGNGVHCGKKTCYVDWGQATASIGKIIVNGWTQHGPWAHR

SEQ ID NO: 235 - DNA, 183 bp, Pediococcus pentosaceus
atgactgaaattaaagtactaaacgataaggaactaaaaaatgtcgtaggaggaaagtattacggtaacggagtgcattgtggtaaaaagacttgctatgtggactggggacaagctacagctagcattggaaaaattatagtgaacggatggacacaacacgggccttgggcacatagataa

SEQ ID NO: 236 - protein, 60 aa, Staphylococcus epidermidis
MKNNKNLFDLEIKKETSQNTDELEPQTAGPAIRASVKQCQKTLKATRLFTVSCKGKNGCK

SEQ ID NO: 237 - DNA, 183 bp, Staphylococcus epidermidis
atgaaaaataacaaaaatttatttgatttagaaattaaaaaagaaacaagtcaaaacactgatgaacttgaacctcaaactgctggaccagcgattagagcttctgtgaaacaatgtcagaaaactttgaaagctacgcgtttatttacagtgtcttgcaaaggaaaaaacggatgtaaatag

SEQ ID NO: 238 - protein, 62 aa, Carnobacterium maltaromaticum
MKTVKELSVKEMQLTTGGKYYGNGVSCNKNGCTVDWSKAIGIIGNNAAANLTTGGAAGWNKG

SEQ ID NO: 239 - DNA, 189 bp, Carnobacterium maltaromaticum
atgaaaactgttaaagaacttagcgttaaagaaatgcaactaactacaggaggtaagtattacggaaatggcgtttcctgtaataaaaatggttgtactgtagattggagcaaagctattgggattataggaaacaatgcagcagcaaatttgactacaggtggagccgctggttggaacaaaggataa

SEQ ID NO: 240 - protein, 69 aa, Lactobacillus plantarum
  VARIANT 40: Xaa = any amino acid
MYKELTVDELALIDGGKKKKKKVACTWGNAATAAASGAVXGILGGPTGALAGAIWGVSQCASNNLHGMH

SEQ ID NO: 241 - DNA, 210 bp, Lactobacillus plantarum
  misc_feature 119: n = a, c, t or g
atgtataaagaattaacagttgatgaattagcattgattgatggaggaaaaaagaagaagaaaaaagtagcttgtacttggggaaatgcagcaacagccgctgcttctggtgcagttangggtattcttggtgggcctactggtgcactggctggagctatctggggcgtttcacaatgcgcgtctaacaacttacacggcatgcactaa

SEQ ID NO: 242 - protein, 56 aa, Lactobacillus plantarum
MMKKIEKLTEKEMANIIGGKYYGNGVTCGKHSCSVNWGQAFSCSVSHLANFGHGKC

SEQ ID NO: 243 - DNA, 171 bp, Lactobacillus plantarum
atgatgaaaaaaattgaaaaattaactgaaaaagaaatggccaatatcattggtggtaaatactatggtaatggggttacttgtggtaaacattcctgctctgttaactggggccaagcattttcttgtagtgtgtcacatttagctaacttcggtcatggaaagtgctaa

SEQ ID NO: 244 - protein, 64 aa, Lactobacillus plantarum
MSKLVKTLTVDEISKIQTNGGKPAWCWYTLAMCGAGYDSGTCDYMYSHCFGVKHSSGGGGSYHC

SEQ ID NO: 245 - DNA, 195 bp, Lactobacillus plantarum
atgagtaaactagttaaaacattaactgtcgatgaaatctctaagattcaaaccaatggtggaaaacctgcatggtgttggtacacattggcaatgtgcggtgctggttatgattcaggcacttgtgattatatgtattcacactgctttggtgtaaaacactctagcggtggtggcggtagctaccattgttag

SEQ ID NO: 246 - protein, 56 aa, Lactobacillus plantarum
MLQFEKLQYSRLPQKKLAKISGGFNRGGYNFGKSVRHVVDAIGSVAGIRGILKSIR

SEQ ID NO: 247 - DNA, 171 bp, Lactobacillus plantarum
atgctacagtttgagaaattacaatattccaggttgccgcaaaaaaagcttgccaaaatatctggtggttttaatcggggcggttataactttggtaaaagtgttcgacatgttgttgatgcaattggttcagttgcaggcattcgtggtattttgaaaagtattcgttaa

SEQ ID NO: 248 - protein, 52 aa, Lactobacillus plantarum
MKKFLVLRDRELNAISGGVFHAYSARGVRNNYKSAVGPADWVISAVRGFIHG

SEQ ID NO: 249 - DNA, 159 bp, Lactobacillus plantarum
atgaaaaaatttctagttttgcgtgaccgtgaattaaatgctatttcaggtggcgttttccatgcctatagcgcgcgtggcgttcggaataattataaaagtgctgttgggcctgccgattgggtcattagcgctgtccgaggattcatccacggatag

SEQ ID NO: 250 - protein, 55 aa, Lactobacillus plantarum
MTVNKMIKDLDVVDAFAPISNNKLNGVVGGGAWKNFWSSLRKGFYDGEAGRAIRR

SEQ ID NO: 251 - DNA, 168 bp, Lactobacillus plantarum
atgactgtgaacaaaatgattaaggatttggatgtagtagatgcatttgcacctatttctaataataagttgaacggggttgttgggggaggcgcttggaaaaatttctggtctagtttaagaaaaggattttatgatggcgaagctggcagagcaatccgtcgttaa

SEQ ID NO: 252 - protein, 57 aa, Lactobacillus plantarum
MKIKLTVLNEFEELTADAEKNISGGRRSRKNGIGYAIGYAFGAVERAVLGGSRDYNK

SEQ ID NO: 253 - DNA, 174 bp, Lactobacillus plantarum
atgaaaattaaattaactgttttaaatgaatttgaagaattaactgctgacgctgaaaagaatatttctggtggccgtcggagtcgtaaaaatggaattggatacgctattggttatgcgtttggcgcggttgaacgggccgtgcttggtggttcaagggattataataagtga

SEQ ID NO: 254 - protein, 47 aa, Lactobacillus plantarum
MDKFEKISTSNLEKISGGDLTTKLWSSWGYYLGKKARWNLKHPYVQF

SEQ ID NO: 255 - DNA, 141 bp, Lactobacillus plantarum
atggataaatttgaaaaaattagtacatctaacctagaaaagatctctggcggtgatttaacaaccaagttatggagctcttggggatattatcttggcaagaaagcacgttggaatttaaagcacccatatgttcaattt

SEQ ID NO: 256 - protein, 55 aa, Lactobacillus plantarum
MNNLNKFSTLGKSSLSQIEGGSVPTSVYTLGIKILWSAYKHRKTIEKSFNKGFYH

SEQ ID NO: 257 - DNA, 168 bp, Lactobacillus plantarum
atgaataacttgaataaattttctactctaggcaagagtagcttgtctcaaattgagggcggatcagtcccaacttcagtatatacgcttggaattaaaattctatggtctgcgtataagcatcgcaaaacgattgaaaaaagttttaataaaggcttttatcattaa

SEQ ID NO: 258 - protein, 55 aa, Lactobacillus plantarum
MNNALSFEQQFTDFSTLSDSELESVEGGRNKLAYNMGHYAGKATIFGLAAWALLA

SEQ ID NO: 259 - DNA, 168 bp, Lactobacillus plantarum
atgaataacgcattaagttttgaacaacaatttacagacttcagcaccttatcggactctgaattagaatccgttgagggtggccgaaataagcttgcatataatatggggcattacgctggtaaggcaaccatttttggacttgcagcatgggcactccttgcatga

SEQ ID NO: 260 - protein, 47 aa, Lactobacillus plantarum
MDKIIKFQGISDDQLNAVIGGKKKKQSWYAAAGDAIVSFGEGFLNAW

SEQ ID NO: 261 - DNA, 144 bp, Lactobacillus plantarum
atggataagattattaagtttcaagggatttctgatgatcaattaaatgctgttatcggtgggaaaaagaaaaaacaatcttggtacgcagcagctggtgatgcaatcgttagttttggtgaaggatttttaaatgcttggtaa

SEQ ID NO: 262 - protein, 59 aa, Lactobacillus plantarum
MKISKIEAQARKDFFKKIDTNSNLLNVNGAKCKWWNISCDLGNNGHVCTLSHECQVSCN

SEQ ID NO: 263 - DNA, 180 bp, Lactobacillus plantarum
atgaaaatttctaagattgaagctcaggctcgtaaagatttttttaaaaaaatcgatactaactcgaacttattaaatgtaaatggtgccaaatgcaagtggtggaatatttcgtgtgatttaggaaataatggccatgtttgtaccttgtcacatgaatgccaagtatcttgtaactaa

SEQ ID NO: 264 - protein, 67 aa, Lactobacillus plantarum
MTKTSRRKNAIANYLEPVDEKSINESFGAGDPEARSGIPCTIGAAVAASIAVCPTTKCSKRCGKRKK

SEQ ID NO: 265 - DNA, 204 bp, Lactobacillus plantarum
atgactaaaactagtcgtcgtaagaatgctattgctaattatttagaaccagtcgacgaaaaaagtattaatgaatcttttggggctggggatccggaagcaagatccggaattccatgtacaatcggcgcagctgtcgcagcatcaattgcagtttgtccaactactaagtgtagtaaacgttgtggcaagcgtaagaaataa

SEQ ID NO: 266 - protein, 48 aa, Lactobacillus plantarum
MKIQIKGMKQLSNKEMQKIVGGKSSAYSLQMGATAIKQVKKLFKKWGW

SEQ ID NO: 267 - DNA, 147 bp, Lactobacillus plantarum
atgaaaattcaaattaaaggtatgaagcaacttagtaataaggaaatgcaaaaaatagtaggtggaaagagtagtgcgtattctttgcagatgggggcaactgcaattaaacaggtaaagaaactgtttaaaaaatggggatggtaa

SEQ ID NO: 268 - protein, 207 aa, Propionibacterium jensenii
MNKTHKMATLVIAAILAAGMTAPTAYADSPGNTRITASEQSVLTQILGHKPTQTEYNRYVETYGSVPTEADINAYIEASESEGSSSQTAAHDDSTSPGTSTEIYTQAAPARFSMFFLSGTWITRSGVVSLSLKPRKGGIGNEGDERTWKTVYDKFHNAGQWTRYKNNGVDASMKKQYMCHFKYGMVKTPWNLEPHKKAADVSPVKCN

SEQ ID NO: 269 - DNA, 624 bp, Propionibacterium jensenii
atgaacaaaacacacaaaatggcgacgctggtaattgccgcgatcttggccgccggaatgaccgcaccaactgcctatgcagattctcctggaaacaccagaattacagccagcgagcaaagcgtccttacccagatactcggccacaaacctacacaaactgaatataaccgatacgttgagacttacggaagcgtaccgaccgaagcagacatcaacgcatatatagaagcgtctgaatctgagggatcatcaagtcaaacggctgctcacgatgactcgacatcacccggcacgagtaccgaaatctacacgcaggcagcccctgccaggttctcaatgtttttcctgtccggaacttggatcactaggagtggtgtagtatcgctctccttgaagccaaggaagggtggtattggcaacgagggggacgagcgtacctggaagactgtatacgacaaattccataacgctgggcaatggacacgatacaagaacaacggcgtagacgccagcatgaaaaagcagtacatgtgccacttcaagtacgggatggtgaagacgccatggaatctggagccccacaagaaggctgcagacgtcagtccagtcaagtgcaactag

SEQ ID NO: 270 - protein, 96 aa, Propionibacterium thoenii
MKKTLLRSGTIALATAAAFGASLAAAPSAMAVPGGCTYTRSNRDVIGTCKTGSGQFRIRLDCNNAPDKTSVWAKPKVMVSVHCLVGQPRSISFETK

SEQ ID NO: 271 - DNA, 291 bp, Propionibacterium thoenii
atgaagaagaccctcctgcgaagtggaacgatcgcactggcgaccgcggctgcatttggcgcatcattggcagccgccccatctgccatggccgttcctggtggttgcacgtacacaagaagcaatcgcgacgtcatcggtacctgcaagactggaagcggccagttccgaatccgacttgactgcaacaacgctccagacaaaacttcagtctgggccaagcccaaggtaatggtgtcggttcactgtcttgttggtcaaccgaggtccatctcgttcgagaccaagtga

SEQ ID NO: 272 - protein, 255 aa, Propionibacterium freudenreichii subsp freudenreii
MNTKAVNLKSENTTKLVSYLTENQLDEFIRRIRIDGALVEEVSQNAKQALDNTGLNGWINTDCDEGLLSDFISKIASARWIPLAESIRPAVTDRDKYRVSCWFYQGMNIAIYANIGGVANIIGYTEAAVATLLGAVVAVAPVVPGTPTPPKDKSSQYKEVPLAVRLSETYHEEGVRGLFDELNYSESRMISTLRRASTDGVLINSWNDGQDTILLKKYNFQDLQLTVRSRIVGNQTIIEECKITDGRKTLSDETV

SEQ ID NO: 273 - DNA, 768 bp, Propionibacterium freudenreichii subsp freudenreii
atgaataccaaagctgtaaatctgaagtcagaaaacacgactaagttggtgagctaccttacggaaaatcaattggatgagtttattagaaggattcgcattgatggcgctcttgtggaagaggtcagtcaaaatgctaagcaggccttagataatactgggctcaatggctggataaatactgattgcgatgaaggccttctctctgatttcatttcaaagatagcaagtgctagatggattccattagctgagtcaattcgacctgcggtgactgacagggataagtatcgagtaagttgctggttctaccaggggatgaatatagcaatttacgcaaatatcggtggcgtggccaatattatcggctatacggaggccgcagtcgcaacactccttggtgcagttgtggcggtagctcctgtggtccctggaactccaacccctccaaaggacaagagttcgcaatataaggaggttccccttgccgttcgtctttccgaaacataccacgaagagggagtacgaggtctattcgacgagctgaactactccgagagccgtatgatctctactctaaggcgagcatcaaccgatggagtcctaattaattcttggaacgatgggcaggatacaattctgcttaagaagtacaatttccaagacttgcaactgactgtcaggagccgcattgttgggaatcaaacaataattgaagaatgcaaaatcactgatggtagaaaaactctttcagacgagactgtgtag

SEQ ID NO: 274 - protein, 618 aa, Pseudomonas aeruginosa
MARPIADLIHFNSTTVTASGDVYYGPGGGTGIGPIARPIEHGLDSSTENGWQEFESYADVGVDPRRYVPLQVKEKRREIELQFRDAEKKLEASVQAELDKADAALGPAKNLAPLDVINRSLTIVGNALQQKNQKLLLNQKKITSLGAKNFLTRTAEEIGEQAVREGNINGPEAYMRFLDREMEGLTAAYNVKLFTEAISSLQIRMNTLTAAKASIEAAAANKAREQAAAEAKRKAEEQARQQAAIRAANTYAMPANGSVVATAAGRGLIQVAQGAASLAQAISDAIAVLGRVLASAPSVMAVGFASLTYSSRTAEQWQDQTPDSVRYALGMDAAKLGLPPSVNLNAVAKASGTVDLPMRLTNEARGNTTTLSVVSTDGVSVPKAVPVRMAAYNATTGLYEVTVPSTTAEAPPLILTWTPASPPGNQNPSSTTPVVPKPVPVYEGATLTPVKATPETYPGVITLPEDLIIGFPADSGIKPIYVMFRDPRDVPGAATGKGQPVSGNWLGAASQGEGAPIPSQIADKLRGKTFKNWRDFREQFWIAVANDPELSKQFNPGSLAVMRDGGAPYVRESEQAGGRIKIEIHHKVRVADGGGVYNMGNLVAVTPKRHIEIHKGGK

SEQ ID NO: 275 - DNA, 1857 bp, Pseudomonas aeruginosa
atggcacgacccattgctgaccttatccacttcaactctacaactgtcacggcaagcggagacgtttattacggccctgggggaggtaccggcattggccccattgccagacctatagagcacggcttggattcgtccactgaaaatggctggcaagagtttgaaagttatgctgatgtgggcgttgaccccagacgctatgttcctcttcaggttaaagaaaaacgcagggagatcgagcttcagttccgagatgccgagaaaaaacttgaggcgtcggtacaagccgagctggataaggctgatgccgctcttggtccggcaaagaatcttgcaccattggacgtcatcaaccgcagtctgaccatcgttggaaacgccctccagcaaaagaatcaaaaactactgctgaatcagaagaagattaccagcctgggtgcaaagaatttccttacccgtacggcggaagagatcggtgaacaagcggtgcgagaaggcaatattaacgggcctgaagcctatatgcgcttcctcgacagggaaatggaaggtctcacggcagcttataacgtaaaactcttcaccgaagcgatcagtagtctccagatccgcatgaatacgttgaccgccgccaaagcaagtattgaggcggccgcagcaaacaaggcgcgtgaacaagcagcggctgaggccaaacgcaaagccgaagagcaggcccgccagcaagcggcgataagagctgccaatacctatgccatgccggccaatggcagcgttgtcgccaccgccgcaggccggggtctgatccaggtcgcacaaggcgccgcatcccttgctcaagcgatctccgatgcgattgccgtcctgggccgggtcctggcttcagcaccctcggtgatggccgtgggctttgccagtctgacctactcctcccggactgccgagcaatggcaggaccaaacgcccgatagcgttcgttacgccctgggcatggatgccgctaaattggggcttcccccaagcgtaaacctgaacgcggttgcaaaagccagcggtaccgtcgatctgccgatgcgcctgaccaacgaggcacgaggcaacacgacgaccctttcggtggtcagcaccgatggtgtgagcgttccgaaagccgttccggtccggatggcggcctacaatgccacgacaggcctgtacgaggttacggttccctctacgaccgcagaagcgccgccactgatcctgacctggacgccggcgagtcctccaggaaaccagaacccttcgagtaccactccggtcgtaccgaagccggtgccggtatatgagggagcgacccttacaccggtgaaggctaccccggaaacctatcctggggtgattacactaccggaagacctgatcatcggcttcccggccgactcggggatcaagccgatctatgtgatgttcagggatccgcgggatgtacctggtgctgcgactggcaagggacagcccgtcagcggtaattggctcggcgccgcctctcaaggtgagggggctccaattccaagccagattgcggataaactacgtggtaagacattcaaaaactggcgggactttcgggaacaattctggatagctgtggctaatgatcctgagttaagtaaacagtttaatcctggtagtttagctgtaatgagagatggaggggctccttatgtcagagagtcagaacaggctggcgggagaataaagatcgaaatccaccacaaggttcgagtagcagatggaggcggcgtttacaatatggggaaccttgttgcagtaacgccaaaacgtcatatagaaatccacaagggagggaagtga

SEQ ID NO: 276 - protein, 689 aa, Pseudomonas aeruginosa
MAVNDYEPGSMVITHVQGGGRDIIQYIPARSSYGTPPFVPPGPSPYVGTGMQEYRKLRSTLDKSHSELKKNLKNETLKEVDELKSEAGLPGKAVSANDIRDEKSIVDALMDAKAKSLKAIEDRPANLYTASDFPQKSESMYQSQLLASRKFYGEFLDRHMSELAKAYSADIYKAQIAILKQTSQELENKARSLEAEAQRAAAEVEADYKARKANVEKKVQSELDQAGNALPQLTNPTPEQWLERATQLVTQAIANKKKLQTANNALIAKAPNALEKQKATYNADLLVDEIASLQARLDKLNAETARRKEIARQAAIRAANTYAMPANGSVVATAAGRGLIQVAQGAASLAQAISDAIAVLGRVLASAPSVMAVGFASLTYSSRTAEQWQDQTPDSVRYALGMDAAKLGLPPSVNLNAVAKASGTVDLPMRLTNEARGNTTTLSVVSTDGVSVPKAVPVRMAAYNATTGLYEVTVPSTTAEAPPLILTWTPASPPGNQNPSSTTPVVPKPVPVYEGATLTPVKATPETYPGVITLPEDLIIGFPADSGIKPIYVMFRDPRDVPGAATGKGQPVSGNWLGAASQGEGAPIPSQIADKLRGKTFKNWRDFREQFWIAVANDPELSKQFNPGSLAVMRDGGAPYVRESEQAGGRIKIEIHHKVRIADGGGVYNMGNLVAVTPKRHIEIHKGGK

SEQ ID NO: 277 - DNA, 2070 bp, Pseudomonas aeruginosa
atggctgtcaatgattacgaacctggttcgatggttattacacatgtgcagggtggtgggcgtgacataatccagtatattcctgctcgatcaagctacggtactccaccatttgtcccaccaggaccaagtccgtatgtcggtactggaatgcaggagtacaggaagctaagaagtacgcttgataagtcccattcagaactcaagaaaaacctgaaaaatgaaaccctgaaggaggttgatgaactcaagagtgaagcggggttgccaggtaaagcggtcagtgccaatgacatccgcgatgaaaagagtatcgttgatgcactcatggatgccaaagcaaaatcgctaaaggccattgaggatcgcccggccaatctttatacggcttcagactttcctcagaagtcagagtcgatgtaccagagtcagttgctggccagccgaaaattctatggagagttcctggatcgccatatgagtgagctggccaaagcgtacagcgccgatatctataaggcgcaaatcgctatcttgaaacaaacgtctcaagagctggagaataaagcccggtcattggaagcagaagcccagcgagccgctgctgaggtggaggcggactacaaggccaggaaggcaaatgtcgagaaaaaagtgcagtccgagcttgaccaggctgggaatgctttgcctcaactgaccaatccaacgccagagcagtggcttgaacgcgctactcaactggttacgcaggcgatcgccaataagaagaaattgcagactgcaaacaatgccttgattgccaaggcacccaatgcactggagaaacaaaaggcaacctacaacgccgatctcctagtggatgaaatcgccagcctgcaagcacggctggacaagctgaacgccgaaacggcaaggcgcaaggaaatcgctcgtcaagcggcgatcagggctgccaatacttatgccatgccagccaatggcagcgttgtcgccaccgccgcaggccggggtctgatccaggtcgcacaaggcgccgcatcccttgctcaagcgatctccgatgcgattgccgtcctgggccgggtcctggcttcagcaccctcggtgatggccgtgggctttgccagtctgacctactcctcccggactgccgagcaatggcaggaccaaacgcccgatagcgttcgttacgccctgggcatggatgccgctaaattggggcttcccccaagcgtaaacctgaacgcggttgcaaaagccagcggtaccgtcgatctgccgatgcgcctgaccaacgaggcacgaggcaacacgacgaccctttcggtggtcagcaccgatggtgtgagcgttccgaaagccgttccggtccggatggcggcctacaatgccacgacaggcctgtacgaggttacggttccctctacgaccgcagaagcgccgccactgatcctgacctggacgccggcgagtcctccaggaaaccagaacccttcgagtaccactccggtcgtaccgaagccggtgccggtatatgagggagcgacccttacaccggtgaaggctaccccggaaacctatcctggggtgattacactaccggaagacctgatcatcggcttcccggccgactcggggatcaagccgatctatgtgatgttcagggatccgcgggatgtacctggtgctgcgactggcaagggacagcccgtcagcggtaattggctcggcgccgcctctcaaggtgagggggctccaattccaagccagattgcggataaactacgtggtaagacattcaaaaactggcgggactttcgggaacaattctggatagctgtggctaatgatcctgagttaagtaaacagtttaatcctggtagtttagctgtaatgagagatggaggggctccttatgtcagagagtcagaacaggctggcgggagaataaagatcgaaatccaccacaaggttcgaatagcagatggaggcggcgtttacaatatggggaaccttgttgcagtaacgccaaaacgtcatatagaaatccacaagggagggaagtga

SEQ ID NO: 278 - protein, 47 aa, Ruminococcus gnavus
MRNDVLTLTNPMEEKELEQILGGGNGVLKTISHECNMNTWQFLFTCC

SEQ ID NO: 279 - DNA, 144 bp, Ruminococcus gnavus
atgagaaatgacgtattaacattaacaaacccaatggaagagaacgaactggagcagatcttaggtggtggcaatggtgtgttaaaaacgattagccacgaatgcaatatgaacacatggcagttcctgtttacttgttgctaa

SEQ ID NO: 280 - protein, 55 aa, Lactobacillus sakei
MKNAKSLTIQEMKSITGGKYYGNGVSCNSHGCSVNWGQAWTCGVNHLANGGHGVC

SEQ ID NO: 281 - DNA, 168 bp, Lactobacillus sakei
atgaaaaacgcaaaaagcctaacaattcaagaaatgaaatctattacaggtggtaaatactatggtaatggcgttagctgtaactctcacggctgttcagtaaattgggggcaagcatggacttgtggagtaaaccatctagctaatggcggtcatggagtttgttaa

SEQ ID NO: 282 - protein, 59 aa, Lactobacillus sakei; identical to SEQ ID NO: 68

SEQ ID NO: 283 - DNA, 180 bp, Lactobacillus sakei; identical to SEQ ID NO: 69

SEQ ID NO: 284 - protein, 61 aa, Lactobacillus sakei
MEKFIELSLKEVTAITGGKYYGNGVHCGKHSCTVDWGTAIGNIGNNAAANWATGGNAGWNK

SEQ ID NO: 285 - DNA, 186 bp, Lactobacillus sakei
atggaaaagtttattgaattatctttaaaagaagtaacagcaattacaggtggaaaatattatggtaacggtgtacactgtggaaaacattcatgtaccgtagactggggaacagctattggaaatatcggaaataatgcagctgcaaactgggccacaggcggaaacgctggctggaataaataa

SEQ ID NO: 286 - protein, 56 aa, Streptococcus salivarius
MKSTNNQSIAEIAAVNSLQEVSMEELDQIIGAGNGVVLTLTHECNLATWTKKLKCC

SEQ ID NO: 287 - DNA, 171 bp, Streptococcus salivarius
atgaaatcaacaaataatcaaagtatcgcagaaattgcagcagtaaactcactacaagaagtaagtatggaggaactagaccaaattattggtgccggaaacggagtggttcttactcttactcatgaatgtaacctagcaacttggacaaaaaaactaaaatgttgctaa

SEQ ID NO: 288 - protein, 51 aa, Streptococcus pyogenes serotype M28
MSFMKNSKDILTNAIEEVSEKELMEVAGGKKGSGWFATITDDCPNSVFVCC

SEQ ID NO: 289 - DNA, 156 bp, Streptococcus pyogenes serotype M28
atgagttttatgaaaaattcaaaggatattttgactaatgctatcgaagaagtttctgaaaaagaacttatggaagtagctggtggtaaaaaaggttccggttggtttgcaactattactgatgactgtccgaactcagtattcgtttgttgttaa

SEQ ID NO: 290 - protein, 48 aa, Streptococcus salivarius
MKNSKDVLNNAIEEVSEKELMEVAGGKKGPGWIATITDDCPNSIFVCC

SEQ ID NO: 291 - DNA, 147 bp, Streptococcus salivarius
atgaaaaactcaaaagatgttttgaacaatgctatcgaagaggtttctgaaaaagaacttatggaagtagctggtggtaaaaaaggtccaggttggattgcaactattactgatgactgtccaaactcaatattcgtttgttgttaa

SEQ ID NO: 292 - protein, 48 aa, Streptococcus salivarius
MKNSKDILNNAIEEVSEKELMEVAGGKRGSGWIATITDDCPNSVFVCC

SEQ ID NO: 293 - DNA, 147 bp, Streptococcus salivarius
atgaaaaactcaaaagatattttgaacaatgctatcgaagaagtttctgaaaaagaacttatggaagtagctggtggtaaaagaggttcaggttggattgcaactattactgatgactgtccaaactcagtattcgtttgttgttaa

SEQ ID NO: 294 - protein, 62 aa, Staphylococcus aureus
MKSSFLEKDIEEQVTWFEEVSEQEFDDDIFGACSTNTFSLSDYWGNKGNWCTATHECMSWCK

SEQ ID NO: 295 - DNA, 189 bp, Staphylococcus aureus
atgaaaagttcttttttagaaaaagatatagaagaacaagtgacatggttcgaggaagtttcagaacaagaatttgacgatgatatttttggagcttgtagtacaaacactttttctttgagtgactattggggtaataaaggaaattggtgtactgctactcacgaatgtatgtcttggtgtaaataa

SEQ ID NO: 296 - protein, 67 aa, Staphylococcus aureus
MKNELGKFLEENELELGKFSESDMLEITDDEVYAAGTPLALLGGAATGVIGYISNQTCPTTACTRAC

SEQ ID NO: 297 - DNA, 204 bp, Staphylococcus aureus
atgaaaaatgaattaggtaagtttttagaagaaaacgaattagagttaggtaaattttcagaatcagacatgctagaaattactgatgatgaagtatatgcagctggaacacctttagccttattgggtggagctgccaccggggtgataggttatatttctaaccaaacatgtccaacaactgcttgtacacgcgcttgctag

SEQ ID NO: 298 - protein, 46 aa, Streptococcus pyogenes
MNNTIKDFDLDLKTNKKDTATPYVGSRYLCTPGSCWKLVCFTTTVK

SEQ ID NO: 299 - DNA, 141 bp, Streptococcus pyogenes
atgaataacacaattaaagactttgatctcgatttgaaaacaaataaaaaagacactgctacaccttatgttggtagccgttacctatgtacccctggttcttgttggaaattagtttgctttacaacaactgttaaataa

SEQ ID NO: 300 - protein, 51 aa, Streptococcus pyogenes
MEKNNEVINSIQEVSLEELDQIIGAGKNGVFKTISHECHLNTWAFLATCCS

SEQ ID NO: 301 - DNA, 156 bp, Streptococcus pyogenes
atggaaaaaaataatgaagtaatcaactctattcaagaagttagtcttgaagaactcgatcaaattatcggtgctggaaaaaatggtgtgtttaaaacaatttctcatgagtgtcatttgaatacatgggcattccttgctacttgttgttcataa

SEQ ID NO: 302 - protein, 51 aa, Streptococcus pyogenes serotype M49
MTKEHEIINSIQEVSLEELDQIIGAGKNGVFKTISHECHLNTWAFLATCCS

SEQ ID NO: 303 - DNA, 156 bp, Streptococcus pyogenes serotype M49
atggaaaaaaataatgaagtaatcaactctattcaagaagttagtcttgaagaactcgatcaaattatcggtgctggaaaaaatggtgtgtttaaaacaatttctcatgagtgtcatttgaatacatgggcattccttgctacttgttgctcataa

SEQ ID NO: 304 - protein, 56 aa, Bacillus subtilis
MEKLFKEVKLEELENQKGSGLGKAQCAALWLQCASGGTIGCGGGAVACQNYRQFCR

SEQ ID NO: 305 - DNA, 171 bp, Bacillus subtilis
atggaaaagctatttaaagaagttaaactagaggaactcgaaaaccaaaaaggtagtggattaggaaaagctcagtgtgctgcgttgtggctacaatgtgctagtggcggtacaattggttgtggtggcggagctgttgcttgtcaaaactatcgtcaattctgcagataa

SEQ ID NO: 306 - protein, 56 aa, Bacillus subtilis
MSKFDDFDLDVVKVSKQDSKITPQWKSESLCTPGCVTGALQTCFLQTLTCNCKISK

SEQ ID NO: 307 - DNA, 171 bp, Bacillus subtilis
atgtcaaagttcgatgatttcgatttggatgttgtgaaagtctctaaacaagactcaaaaatcactccgcaatggaaaagtgaatcactttgtacaccaggatgtgtaactggtgcattgcaaacttgcttccttcaaacactaacttgtaactgcaaaatctctaaataa

SEQ ID NO: 308 - protein, 50 aa, Bacillus subtilis
MKLPVQQVYSVYGGKDLPKGHSHSTMPFLSKLQFLTKIYLLDIHTQPFFI

SEQ ID NO: 309 - DNA, 153 bp, Bacillus subtilis
ttgaaattgccggtgcaacaggtctattcggtctatgggggtaaggatctcccaaaagggcatagtcattctactatgccctttttaagtaaattacaatttttaactaaaatctacctcttggatatacatacacaaccgtttttcatttga

SEQ ID NO: 310 - protein, 43 aa, Bacillus subtilis
MKKAVIVENKGCATCSIGAACLVDGPIPDFEIAGATGLFGLWG

SEQ ID NO: 311 - DNA, 132 bp, Bacillus subtilis
atgaaaaaagctgtcattgtagaaaacaaaggttgtgcaacatgctcgatcggagccgcttgtctagtggacggtcctatccctgattttgaaattgccggtgcaacaggtctattcggtctatgggggtaa

SEQ ID NO: 312 - protein, 58 aa, Streptococcus thermophilus; identical to SEQ ID NO: 24

SEQ ID NO: 313 - DNA, 177 bp, Streptococcus thermophilus
atgatgaatgctactgaaaaccaaatttttgttgagactgtgagtgaccaagaattagaaatgttaattggtggtgcagatcgtggatggattaagactttaacaaaagattgtccaaatgtaatttcttcaatttgtgcaggtacaattattacagcctgtaaaaattgtgcttaa

SEQ ID NO: 314 - protein, 64 aa, Streptococcus thermophilus
MKQYNGFEVLHELDLANVTGGQINWGSVVGHCIGGAIIGGAFSGGAAAGVGCLVGSGKAIINGL

SEQ ID NO: 315 - DNA, 195 bp, Streptococcus thermophilus
atgaagcagtataatggttttgaggttctacatgaacttgacttagcaaatgtaactggcggtcaaattaattggggatcagttgtaggacactgtataggtggagctattatcggaggtgcattttcaggaggtgcagcggctggagtaggatgccttgttgggagcggaaaggcaatcataaatggattataa

SEQ ID NO: 316 - protein, 85 aa, Streptococcus thermophilus
MNTITICKFDVLDAELLSTVEGGYSGKDCLKDMGGYALAGAGSGALWGAPAGGVGALPGAFVGAHVGAIAGGFACMGGMIGNKFN

SEQ ID NO: 317 - DNA, 258 bp, Streptococcus thermophilus
atgaatacaataactatttgtaaatttgatgttttagatgctgaacttctttcgacagttgagggtggatactctggtaaggattgtttaaaagacatgggaggatatgcattggcaggagctggaagtggagctctgtggggagctccagcaggaggtgttggagcacttccaggtgcatttgtcggagctcatgttggggcaattgcaggaggctttgcatgtatgggtggaatgattggtaataagtttaactaa

SEQ ID NO: 318 - protein, 52 aa, Bacillus cereus
MSEIKKALNTLEIEDFDAIEMVDVDAMPENEALEIMGASCTTCVCTCSCCTT

SEQ ID NO: 319 - DNA, 159 bp, Bacillus cereus
atgagtgaaattaaaaaagcattaaatacgcttgaaattgaagattttgatgcaattgaaatggttgatgttgatgctatgccagaaaacgaagcgcttgaaattatgggagcgtcatgtacgacatgcgtatgtacatgcagttgttgtacaacttga

SEQ ID NO: 320 - protein, 47 aa, Bacillus cereus
MEVMNNALITKVDEEIGGNAACVIGCIGSCVISEGIGSLVGTAFTLG

SEQ ID NO: 321 - DNA, 144 bp, Bacillus cereus
atggaagttatgaacaatgctttaattacaaaagtagatgaggagattggaggaaacgctgcttgtgtaattggttgtattggcagttgcgtaattagtgaaggaattggttcacttgtaggaacagcatttactttaggttaa

SEQ ID NO: 322 - protein, 49 aa, Bacillus cereus
MEVLNKQNVNIIPESEEVGGWVACVGACGTVCLASGGVGTEFAAASYFL

SEQ ID NO: 323 - DNA, 150 bp, Bacillus cereus
atggaagttttaaacaaacaaaatgtaaatattattccagaatctgaagaagtaggtggatgggtagcatgtgttggagcatgtggtacagtatgtcttgctagtggtggtgttggaacagagtttgcagctgcatcttatttcctataa

SEQ ID NO: 324 - protein, 40 aa, Bacillus thuringiensis
METPVVQPRDWTCWSCLVCAACSVELLNLVTAATGASTAS

SEQ ID NO: 325 - DNA, 123 bp, Bacillus thuringiensis
atggaaacaccagtagtacaaccaagggattggacttgttggagttgcttagtatgtgcagcatgttctgtggaattattaaatttagttactgcggcaacaggggctagtactgcaagctaa

SEQ ID NO: 326 - protein, 42 aa, Rhizobium leguminosarum bv. trifolii
MDNKVAKNVEVKKGSIKATFKAAVLKSKTKVDIGGSRQGCVA

SEQ ID NO: 327 - DNA, 129 bp, Rhizobium leguminosarum bv. trifolii
atggataacaaggttgcgaagaatgtcgaagtgaagaagggctccatcaaggcgaccttcaaggctgctgttctgaagtcgaagacgaaggtcgacatcggaggtagccgtcagggctgcgtcgcttaa

SEQ ID NO: 328 - protein, 70 aa, Streptococcus uberis
MNTIEKFENIKLFSLKKIIGGKTVNYGNGLYCNQKKCWVNWSETATTIVNNSIMNGLTGGNAGWHSGGRA

SEQ ID NO: 329 - DNA, 213 bp, Streptococcus uberis
atgaatacaattgaaaaatttgaaaatattaaacttttttcactaaagaaaattatcggtggcaaaactgtaaattatggtaatggcctttattgtaaccaaaaaaaatgctgggtaaactggtcagaaactgctacaacaatagtaaataattccatcatgaacgggctcacaggtggtaatgcgggttggcactcaggcgggagagcataa

SEQ ID NO: 330 - protein, 76 aa, Streptococcus uberis
MDILLELAGYTGIASGTAKKVVDAIDKGAAAFVIISIISTVISAGALGAVSASADFIILTVKNYISRNLKAQAVIW

SEQ ID NO: 331 - DNA, 231 bp, Streptococcus uberis
atggacattttattagaactcgcaggatatactgggatagcctcaggtactgcaaaaaaagttgttgatgccattgataaaggagctgcagcctttgttattatttcaattatctcaacagtaattagtgcgggagcattgggagcagtttcagcctcagctgattttattattttaactgtaaaaaattacattagtagaaatttaaaagcacaagctgtcatttggtaa

SEQ ID NO: 332 - protein, 64 aa, Clostridium perfringens
MDSELFKLMATQGAFAILFSYLLFYVLKENSKREDKYQNIIEELTELLPKIKEDVEDIKEKLNK

SEQ ID NO: 333 - DNA, 195 bp, Clostridium perfringens
atggatagtgaattatttaagttaatggcaacacaaggagcctttgcaatattattttcgtatttattgttttatgttttaaaagagaatagtaaaagagaagataagtatcaaaatataatagaggagcttacagaattattgccaaaaataaaagaagatgtagaagatataaaagaaaaacttaataaatag

SEQ ID NO: 334 - protein, 47 aa, Micrococcus varians
MTNAFQALDEVTDAELDAILGGGSGVIPTISHECHMNSFQFVFTCCS

SEQ ID NO: 335 - DNA, 144 bp, Micrococcus varians
atgacgaacgcatttcaggcactggacgaagtcacggacgccgagctcgacgccatccttggcgggggcagtggtgttattcccacgatcagccacgagtgccacatgaactccttccagttcgtgttcacctgctgctcctga

SEQ ID NO: 336 - protein, 285 aa, Streptococcus equi subsp. zooepidemicus
MKRIFFAFLSLCLFIFGTQTVSAATYTRPLDTGNITTGFNGYPGHVGVDYAVPVGTPVRAVANGTVKFAGNGANHPWMLWMAGNCVLIQHADGMHTGYAHLSKISVSTDSTVKQGQIIGYTGATGQVTGPHLHFEMLPANPNWQNGFSGRIDPTGYIANAPVFNGTTPTEPTTPTTNLKIYKVDDLQKINGIWQVRNNILVPTDFTWVDNGIAADDVIEVTSNGTRTSDQVLQKGGYFVINPNNVKSVGTPMKGSGGLSWAQVNFTTGGNVWLNTTSKDNLLYGK

SEQ ID NO: 337 - DNA, 858 bp, Streptococcus equi subsp. zooepidemicus
atgaaacgtatattttttgctttcttaagtttatgcttatttatattcggaacacaaacggtatctgcagctacttatactcggccattagatacgggaaatatcactacagggtttaacggataccctggtcatgttggagtcgattatgcagtacccgttggaactccggttagagcagttgcaaatggtacagtcaaatttgcaggtaatggggctaatcacccatggatgctttggatggctggaaactgtgttctaattcaacatgctgacgggatgcatactggatatgcacacttatcaaaaatttcagttagcacagatagtacagttaaacaaggacaaatcataggttatactggtgccaccggccaagttaccggtccacatttgcattttgaaatgttgccagcaaatcctaactggcaaaatggtttttctggaagaatagatccaaccggatacatcgctaatgcccctgtatttaatggaacaacacctacagaacctactactcctacaacaaatttaaaaatctataaagttgatgatttacaaaaaattaatggtatttggcaagtaagaaataacatacttgtaccaactgatttcacatgggttgataatggaattgcagcagatgatgtaattgaagtaactagcaatggaacaagaacctctgaccaagttcttcaaaaaggtggttattttgtcatcaatcctaataatgttaaaagtgttggaactccgatgaaaggtagtggtggtctatcttgggctcaagtaaactttacaacaggtggaaatgtctggttaaatactactagcaaagacaacttactttacggaaaataa

SEQ ID NO: 338 - protein, 45 aa, Myxococcus fulvus
ANCSCSTASDYCPILTFCTTGTACSYTPTGCGTGWVYCACNGNFY

SEQ ID NO: 339 - DNA, 135 bp, Artificial Sequence
  Polynucleotide encoding the polypeptide of SEQ ID NO: 338
gcgaactgcagctgcagcaccgcgagcgattattgcccgattctgaccttttgcaccaccggcaccgcgtgcagctataccccgaccggctgcggcaccggctgggtgtattgcgcgtgcaacggcaacttttat

SEQ ID NO: 340 - protein, 19 aa, Streptomyces griseoluteus
CANSCSYGPLTWSCDGNTK

SEQ ID NO: 341 - DNA, 57 bp, Artificial Sequence
  Polynucleotide encoding the polypeptide of SEQ ID NO: 340
tgcgcgaacagctgcagctatggcccgctgacctggagctgcgatggcaacaccaaa

SEQ ID NO: 342 - protein, 19 aa, Streptoverticillium griseoverticillatum
CKQSCSFGPFTFVCDGNTK

SEQ ID NO: 343 - DNA, 57 bp, Artificial Sequence
  Polynucleotide encoding the polypeptide of SEQ ID NO: 342
tgcaaacagagctgcagctttggcccgtttacctttgtgtgcgatggcaacaccaaa

SEQ ID NO: 344 - protein, 7 aa, Carnobacterium sp.
GSEIQPR

SEQ ID NO: 345 - DNA, 21 bp, Artificial Sequence
  Polynucleotide encoding the polypeptide of SEQ ID NO: 344
ggcagcgaaattcagccgcgc

SEQ ID NO: 346 - protein, 39 aa, Lactococcus lactis subsp. lactis
GTWDDIGQGIGRVAYWVGKAMGNMSDVNQASRINRKKKH

SEQ ID NO: 347 - DNA, 117 bp, Artificial Sequence
  Polynucleotide encoding the polypeptide of SEQ ID NO: 346
ggcacctgggatgatattggccagggcattggccgcgtggcgtattgggtgggcaaagcgatgggcaacatgagcgatgtgaaccaggcgagccgcattaaccgcaaaaaaaaacat

SEQ ID NO: 348 - protein, 35 aa, Lactococcus lactis subsp. lactis
KKWGWLAWVDPAYEFIKGFGKGAIKEGNKDKWKNI

SEQ ID NO: 349 - DNA, 105 bp, Artificial Sequence
  Polynucleotide encoding the polypeptide of SEQ ID NO: 348
aaaaaatggggctggctggcgtgggtggatccggcgtatgaatttattaaaggctttggcaaaggcgcgattaaagaaggcaacaaagataaatggaaaaacatt

SEQ ID NO: 350 - protein, 19 aa, Streptomyces sp.
CVQSCSFGPLTWSCDGNTK

SEQ ID NO: 351 - DNA, 57 bp, Artificial Sequence
  Polynucleotide encoding the polypeptide of SEQ ID NO: 350
tgcgtgcagagctgcagctttggcccgctgacctggagctgcgatggcaacaccaaa

SEQ ID NO: 352 - protein, 19 aa, Actinoplanes liguriae
SSGWVCTLTIECGTVICAC

SEQ ID NO: 353 - DNA, 57 bp, Artificial Sequence
  Polynucleotide encoding the polypeptide of SEQ ID NO: 352
agcagcggctgggtgtgcaccctgaccattgaatgcggcaccgtgatttgcgcgtgc

SEQ ID NO: 354 - protein, 38 aa, Lactobacillus curvatus
  VARIANT 34: Xaa = any amino acid
  VARIANT 37: Xaa = any amino acid
YTAKQCLQAIGSCGIAGTGAGAAGGPAGAFVGAXVVXI

SEQ ID NO: 355 - DNA, 114 bp, Artificial Sequence
  Polynucleotide encoding the polypeptide of SEQ ID NO: 354
  misc_feature 100, 101, 102, 109, 110, 111: n = A,T,C or G
  misc_feature (100)...(102): nnn = a codon other than a stop codon
  misc_feature (109)...(111): nnn = a codon other than a stop codon
tataccgcgaaacagtgcctgcaggcgattggcagctgcggcattgcgggcaccggcgcgggcgcggcgggcggcccggcgggcgcgtttgtgggcgcgnnngtggtgnnnatt

SEQ ID NO: 356 - protein, 42 aa, Lactobacillus sakei
  VARIANT 32: Xaa = any amino acid
TKYYGNGVYCNSKKCWVDWGQAAGGIGQTVVXGWLGGAIPGK

SEQ ID NO: 357 - DNA, 126 bp, Artificial Sequence
  Polynucleotide encoding the polypeptide of SEQ ID NO: 356
  misc_feature (94)...(96): nnn = any amino acid-coding triplet
accaaatattatggcaacggcgtgtattgcaacagcaaaaaatgctgggtggattggggccaggcggcgggcggcattggccagaccgtggtgnnnggctggctgggcggcgcgattccgggcaaa

SEQ ID NO: 358 - protein, 22 aa, Streptococcus mutans
FKSWSFCTPGCAKTGSFNSYCC

SEQ ID NO: 359 - DNA, 132 bp, Artificial Sequence
  Polynucleotide encoding the polypeptide of SEQ ID NO: 358
tttaaaagctggagcttttgcaccccgggctgcgcgaaaaccggcagctttaacagctattgctgctttaaaagctggagcttttgcaccccgggctgcgcgaaaaccggcagctttaacagctattgctgc

SEQ ID NO: 360 - protein, 43 aa, Enterococcus mundtii
KYYGNGVSCNKKGCSVDWGKAIGIIGNNSAANLATGGAAGWSK

SEQ ID NO: 361 - DNA, 129 bp, Artificial Sequence
  Polynucleotide encoding the polypeptide of SEQ ID NO: 360
aaatattatggcaacggcgtgagctgcaacaaaaaaggctgcagcgtggattggggcaaagcgattggcattattggcaacaacagcgcggcgaacctggcgaccggcggcgcggcgggctggagcaaa

SEQ ID NO: 362 - protein, 41 aa, Lactobacillus sakei
  VARIANT 9, 14, 33, 37: Xaa = any amino acid
KYYGNGVHXGKHSXTVDWGTAIGNIGNNAAANXATGXNAGG

SEQ ID NO: 363 - DNA, 123 bp, Artificial Sequence
  Polynucleotide encoding the polypeptide of SEQ ID NO: 362
  misc_feature (25)...(27): nnn = any amino acid-coding triplet
  misc_feature (40)...(42): nnn = any amino acid-coding triplet
  misc_feature (97)...(99): nnn = any amino acid-coding triplet
  misc_feature (109)...(111): nnn = any amino acid-coding triplet
aaatattatggcaacggcgtgcatnnnggcaaacatagcnnnaccgtggattggggcaccgcgattggcaacattggcaacaacgcggcggcgaacnnngcgaccggcnnnaacgcgggcggc

SEQ ID NO: 364 - protein, 31 aa, Lactobacillus paracasei
GMSGYIQGIPDFLKGYLHGISAANKHKKGRL

SEQ ID NO: 365 - DNA, 93 bp, Artificial Sequence
  Polynucleotide encoding the polypeptide of SEQ ID NO: 364
ggcatgagcggctatattcagggcattccggattttctgaaaggctatctgcatggcattagcgcggcgaacaaacataaaaaaggccgcctg

SEQ ID NO: 366 - protein, 31 aa, Leuconostoc mesenteroides
KGKGFWSWASKATSWLTGPQQPGSPLLKKHR

SEQ ID NO: 367 - DNA, 93 bp, Artificial Sequence
  Polynucleotide encoding the polypeptide of SEQ ID NO: 366
aaaggcaaaggcttttggagctgggcgagcaaagcgaccagctggctgaccggcccgcagcagccgggcagcccgctgctgaaaaaacatcgc

SEQ ID NO: 368 - protein, 43 aa, Leuconostoc mesenteroides
KNYGNGVHCTKKGCSVDWGYAWTNIANNSVMNGLTGGNAGWHN

SEQ ID NO: 369 - DNA, 129 bp, Artificial Sequence
  Polynucleotide encoding the polypeptide of SEQ ID NO: 368
aaaaactatggcaacggcgtgcattgcaccaaaaaaggctgcagcgtggattggggctatgcgtggaccaacattgcgaacaacagcgtgatgaacggcctgaccggcggcaacgcgggctggcataac

SEQ ID NO: 370 - protein, 47 aa, Bacillus subtilis
AIKLVQSPNGNFAASFVLDGTKWIFKSKYYDSSKGYWVGIYEVWDRK

SEQ ID NO: 371 - DNA, 141 bp, Artificial Sequence
  Polynucleotide encoding the polypeptide of SEQ ID NO: 370
gcgattaaactggtgcagagcccgaacggcaactttgcggcgagctttgtgctggatggcaccaaatggatttttaaaagcaaatattatgatagcagcaaaggctattgggtgggcatttatgaagtgtgggatcgcaaa

SEQ ID NO: 372 - protein, 12 aa, Bacillus licheniformis
  VARIANT 7: Xaa = any amino acid
ISLEICXIFHDN

SEQ ID NO: 373 - DNA, 36 bp, Artificial Sequence
  Polynucleotide encoding the polypeptide of SEQ ID NO: 372
  misc_feature (19)...(21): nnn = any amino acid-coding triplet
attagcctggaaatttgcnnnatttttcatgataac

SEQ ID NO: 374 - protein, 37 aa, Lactococcus lactis subsp. lactis
TSYGNGVHCNKSKCWIDVSELETYKAGTVSNPKDILW

SEQ ID NO: 375 - DNA, 111 bp, Artificial Sequence
  Polynucleotide encoding the polypeptide of SEQ ID NO: 374
accagctatggcaacggcgtgcattgcaacaaaagcaaatgctggattgatgtgagcgaactggaaacctataaagcgggcaccgtgagcaacccgaaagatattctgtgg

SEQ ID NO: 376 - protein, 9 aa, Serratia plymuthica
DYHHGVRVL

SEQ ID NO: 377 - DNA, 27 bp, Artificial Sequence
  Polynucleotide encoding the polypeptide of SEQ ID NO: 376
gattatcatcatggcgtgcgcgtgctg

SEQ ID NO: 378 - protein, 15 aa, Halobacterium sp.
DIDITGCSACKYAAG

SEQ ID NO: 379 - DNA, 45 bp, Artificial Sequence
  Polynucleotide encoding the polypeptide of SEQ ID NO: 378
gatattgatattaccggctgcagcgcgtgcaaatatgcggcgggc

SEQ ID NO: 380 - protein, 12 aa, Bacillus subtilis
  VARIANT 1, 2, 6: Xaa = any amino acid
XXKEIXHIFHDN

SEQ ID NO: 381 - DNA, 36 bp, Artificial Sequence
  Polynucleotide encoding the polypeptide of SEQ ID NO: 380
  misc_feature (1)...(3): nnn = any amino acid-coding triplet
  misc_feature (4)...(6): nnn = any amino acid-coding triplet
  misc_feature (16)...(18): nnn = any amino acid-coding triplet
nnnnnnaaagaaattnnncatatttttcatgataac

SEQ ID NO: 382 - protein, 12 aa, Lactobacillus curvatus
TPVVNPPFLQQT

SEQ ID NO: 383 - DNA, 36 bp, Artificial Sequence
  Polynucleotide encoding the polypeptide of SEQ ID NO: 382
accccggtggtgaacccgccgtttctgcagcagacc

SEQ ID NO: 384 - protein, 10 aa, Lactobacillus curvatus
  VARIANT 10: Xaa = any amino acid
VAPFPEQFLX

SEQ ID NO: 385 - DNA, 30 bp, Artificial Sequence
  Polynucleotide encoding the polypeptide of SEQ ID NO: 384
  misc_feature (28)...(30): nnn = any amino acid-coding triplet
gtggcgccgtttccggaacagtttctgnnn

SEQ ID NO: 386 - protein, 9 aa, Lactobacillus curvatus
NIPQLTPTP

SEQ ID NO: 387 - DNA, 27 bp, Artificial Sequence
  Polynucleotide encoding the polypeptide of SEQ ID NO: 386
aacattccgcagctgaccccgaccccg

SEQ ID NO: 388 - protein, 18 aa, Bacillus thuringiensis subsp. entomocidus
  VARIANT 4, 7, 10: Xaa = any amino acid
DWTXWSXLVXAACSVELL

SEQ ID NO: 389 - DNA, 54 bp, Artificial Sequence
  Polynucleotide encoding the polypeptide of SEQ ID NO: 388
  misc_feature (10)...(12): nnn = any amino acid-coding triplet
  misc_feature (19)...(21): nnn = any amino acid-coding triplet
  misc_feature (28)...(30): nnn = any amino acid-coding triplet
gattggaccnnntggagcnnnctggtgnnngcggcgtgcagcgtggaactgctg

SEQ ID NO: 390 - protein, 30 aa, Lactobacillus curvatus
AYPGNGVHCGKYSCTVDKQTAIGNIGNNAA

SEQ ID NO: 391 - DNA, 90 bp, Artificial Sequence
  Polynucleotide encoding the polypeptide of SEQ ID NO: 390
gcgtatccgggcaacggcgtgcattgcggcaaatatagctgcaccgtggataaacagaccgcgattggcaacattggcaacaacgcggcg

SEQ ID NO: 392 - protein, 43 aa, Carnobacterium divergens
TKYYGNGVYCNSKKCWVDWGTAQGCIDVVIGQLGGGIPGKGKC

SEQ ID NO: 393 - DNA, 129 bp, Artificial Sequence
  Polynucleotide encoding the polypeptide of SEQ ID NO: 392
accaaatattatggcaacggcgtgtattgcaacagcaaaaaatgctgggtggattggggcaccgcgcagggctgcattgatgtggtgattggccagctgggcggcggcattccgggcaaaggcaaatgc

SEQ ID NO: 394 - protein, 62 aa, Enterococcus sp.
NRWYCNSAAGGVGGAAVCGLAGYVGEAKENIAGEVRKGWGMAGGFTHNKACKSFPGSGWASG

SEQ ID NO: 395 - DNA, 186 bp, Artificial Sequence
  Polynucleotide encoding the polypeptide of SEQ ID NO: 394
aaccgctggtattgcaacagcgcggcgggcggcgtgggcggcgcggcggtgtgcggcctggcgggctatgtgggcgaagcgaaagaaaacattgcgggcgaagtgcgcaaaggctggggcatggcgggcggctttacccataacaaagcgtgcaaaagctttccgggcagcggctgggcgagcggc

SEQ ID NO: 396 - protein, 39 aa, Enterococcus faecium
TTKNYGNGVCNSVNWCQCGNVWASCNLATGCAAWLCKLA

SEQ ID NO: 397 - DNA, 117 bp, Artificial Sequence
  Polynucleotide encoding the polypeptide of SEQ ID NO: 396
accaccaaaaactatggcaacggcgtgtgcaacagcgtgaactggtgccagtgcggcaacgtgtgggcgagctgcaacctggcgaccggctgcgcggcgtggctgtgcaaactggcg

SEQ ID NO: 398 - protein, 30 aa, Paenibacillus polymyxa
ASIIKTTIKVSKAVCKTLTCICTGSCSNCK

SEQ ID NO: 399 - DNA, 90 bp, Artificial Sequence
  Polynucleotide encoding the polypeptide of SEQ ID NO: 398
gcgagcattattaaaaccaccattaaagtgagcaaagcggtgtgcaaaaccctgacctgcatttgcaccggcagctgcagcaactgcaaa

SEQ ID NO: 400 - protein, 31 aa, Staphylococcus epidermidis
SASIVKTTIKASKKLCRGFTLTCGCHFTGKK

SEQ ID NO: 401 - DNA, 93 bp, Artificial Sequence
  Polynucleotide encoding the polypeptide of SEQ ID NO: 400
agcgcgagcattgtgaaaaccaccattaaagcgagcaaaaaactgtgccgcggctttaccctgacctgcggctgccattttaccggcaaaaaa

SEQ ID NO: 402 - protein, 43 aa, Enterococcus faecium
KYYGNGVSCNKKGCSVDWGKAIGIIGNNAAANLTTGGKAAWAC

SEQ ID NO: 403 - DNA, 129 bp, Artificial Sequence
  Polynucleotide encoding the polypeptide of SEQ ID NO: 402
aaatattatggcaacggcgtgagctgcaacaaaaaaggctgcagcgtggattggggcaaagcgattggcattattggcaacaacgcggcggcgaacctgaccaccggcggcaaagcggcgtgggcgtgc

SEQ ID NO: 404 - protein, 39 aa, Paenibacillus polymyxa
ATYYGNGLYCNKQKHYTWVDWNKASREIGKITVNGWVQH

SEQ ID NO: 405 - DNA, 117 bp, Artificial Sequence
  Polynucleotide encoding the polypeptide of SEQ ID NO: 404
gcgacctattatggcaacggcctgtattgcaacaaacagaaacattatacctgggtggattggaacaaagcgagccgcgaaattggcaaaattaccgtgaacggctgggtgcagcat

SEQ ID NO: 406 - protein, 35 aa, Bacillus circulans
VNYGNGVSCSKTKCSVNWGIITHQAFRVTSGVASG

SEQ ID NO: 407 - DNA, 105 bp, Artificial Sequence
  Polynucleotide encoding the polypeptide of SEQ ID NO: 406
gtgaactatggcaacggcgtgagctgcagcaaaaccaaatgcagcgtgaactggggcattattacccatcaggcgtttcgcgtgaccagcggcgtggcgagcggc

SEQ ID NO: 408 - protein, 30 aa, Paenibacillus polymyxa
FVYGNGVTSILVQAQFLVNGQRRFFYTPDK

SEQ ID NO: 409 - DNA, 90 bp, Artificial Sequence
  Polynucleotide encoding the polypeptide of SEQ ID NO: 408
tttgtgtatggcaacggcgtgaccagcattctggtgcaggcgcagtttctggtgaacggccagcgccgctttttttataccccggataaa

SEQ ID NO: 410 - protein, 13 aa, Lactobacillus rhamnosus
AVPAVRKTNETLD

SEQ ID NO: 411 - DNA, 39 bp, Artificial Sequence
  Polynucleotide encoding the polypeptide of SEQ ID NO: 410
gcggtgccggcggtgcgcaaaaccaacgaaaccctggat

SEQ ID NO: 412 - protein, 69 aa, Bacillus licheniformis
MKNSAAREAFKGANHPAGMVSEEELKALVGGNDVNPETTPATTSSWTCITAGVTVSASLCPTTKCTSRC

SEQ ID NO: 413 - DNA, 207 bp, Artificial Sequence
  Polynucleotide encoding the polypeptide of SEQ ID NO: 412
atgaaaaacagcgcggcgcgcgaagcgtttaaaggcgcgaaccatccggcgggcatggtgagcgaagaagaactgaaagcgctggtgggcggcaacgatgtgaacccggaaaccaccccggcgaccaccagcagctggacctgcattaccgcgggcgtgaccgtgagcgcgagcctgtgcccgaccaccaaatgcaccagccgctgc

SEQ ID NO: 414 - protein, 36 aa, Lactobacillus plantarum
KYYGNGLSCSKKGCTVNWGQAFSCGVNRVATAGHGK

SEQ ID NO: 415 - DNA, 108 bp, Artificial Sequence
  Polynucleotide encoding the polypeptide of SEQ ID NO: 414
aaatattatggcaacggcctgagctgcagcaaaaaaggctgcaccgtgaactggggccaggcgtttagctgcggcgtgaaccgcgtggcgaccgcgggccatggcaaa

SEQ ID NO: 416 - protein, 24 aa, Lactobacillus acidophilus
GNPKVAHCASQIGRSTAWGAVSGA

SEQ ID NO: 417 - DNA, 72 bp, Artificial Sequence
  Polynucleotide encoding the polypeptide of SEQ ID NO: 416
ggcaacccgaaagtggcgcattgcgcgagccagattggccgcagcaccgcgtggggcgcggtgagcggcgcg

SEQ ID NO: 418 - protein, 40 aa, Enterococcus faecalis; identical to SEQ ID NO: 1

SEQ ID NO: 419 - DNA, 120 bp, Artificial Sequence
  Polynucleotide encoding the polypeptide of SEQ ID NO: 418
tggctgccgccggcgggcctgctgggccgctgcggccgctggtttcgcccgtggctgctgtggctgcagagcggcgcgcagtataaatggctgggcaacctgtttggcctgggcccgaaa

SEQ ID NO: 420 - protein, 40 aa, Anabaena variabilis
NLDQWLTEQVHEFQDMYLEPQAISNQDITFKLSDLDFIHN

SEQ ID NO: 421 - DNA, 124 bp, Anabaena variabilis
taatttagatcagtggttaacagaacaagttcatgagtttcaagatatgtacttggaaccacaagcaatatccaatcaagacattaccttcaaactatctgacctagattttattcataattga

SEQ ID NO: 422 - protein, 40 aa, Nostoc sp; identical to SEQ ID NO: 420

SEQ ID NO: 423 - DNA, 123 bp, Nostoc sp
aatttagatcaatggttaacagaacaagttcatgagtttcaagatatgtacttggaaccacaagcaatatccaatcaagacattaccttcaaactgtcagacctagattttattcataattga

SEQ ID NO: 424 - protein, 7 aa, Nostoc azollae
HREKKSA

SEQ ID NO: 425 - DNA, 24 bp, Nostoc azollae
cacagagagaaaaaatcagcatag

SEQ ID NO: 426 - protein, 23 aa, Acaryochloris marina
TSNNWLAKNYLSMWNKKSSNPNL

SEQ ID NO: 427 - DNA, 72 bp, Acaryochloris marina
acaagcaataactggctagccaaaaactatctttctatgtggaataaaaagagcagtaatccaaacctttag

SEQ ID NO: 428 - protein, 6 aa, Cyanothece
FRYFWW

SEQ ID NO: 429 - DNA, 21 bp, Cyanothece
tttagatatttttggtggtaa

SEQ ID NO: 430 - protein, 6 aa, Cyanothece
FRYFWW

SEQ ID NO: 431 - DNA, 21 bp, Cyanothece
tttagatatttttggtggtaa

SEQ ID NO: 432 - protein, 9 aa, Cyanothece
CGEKWRIFS

SEQ ID NO: 433 - DNA, 27 bp, Cyanothece
tgtggagaaaaatggagaatttttagc

SEQ ID NO: 434 - protein, 8 aa, Cyanothece
FRLQLWQF

SEQ ID NO: 435 - DNA, 24 bp, Cyanothece
tttcgcttacaactgtggcaattt

SEQ ID NO: 436 - protein, 16 aa, Cyanothece
LGCNQSSIWSIFFWNH

SEQ ID NO: 437 - DNA, 51 bp, Cyanothece
ctaggatgtaaccagagcagtatctggtcaatttttttctggaatcattaa

SEQ ID NO: 438 - protein, 40 aa, Microcoleus chthonoplastes
YNLQGLPAIESEDCIPDSVAPSDDWFSGVSSLFNRLTGLG

SEQ ID NO: 439 - DNA, 123 bp, Microcoleus chthonoplastes
tataacctacaggggttgccagcaattgagtcagaagactgtatcccagattctgtagcgccttcggatgattggttttcaggcgtatcgtctctgtttaaccgcttgactgggttgggttag

SEQ ID NO: 440 - protein, 37 aa, Nostoc sp
WMAIRRILRCHPFHPGGYDPVPELGEHCCHHDSGNKG

SEQ ID NO: 441 - DNA, 114 bp, Nostoc sp
tggatggcgattcgccgcattttgcgttgtcatccattccacccagggggttatgatcctgtaccagagttgggtgagcattgttgtcatcatgatagcgggaataaggggtga

SEQ ID NO: 442 - protein, 35 aa, Anabaena variabilis
WMGIRRILRCHPFHPGGYDPVPEVGEHCCHHDSGK

SEQ ID NO: 443 - DNA, 108 bp, Anabaena variabilis
tggatggggattcgccgcattttgcgttgtcatccattccacccaggcggttatgatcctgtaccagaggtgggtgagcattgttgtcatcatgatagcgggaagtag

SEQ ID NO: 444 - protein, 48 aa, Nodularia spumigena
WMATRRILRCHPFHPGGYDPVPEVKHNCCDQHLSDSGKQTTEDHHKGS

SEQ ID NO: 445 - DNA, 147 bp, Nodularia spumigena
tggatggcgactcggcggattttgcgttgtcatcccttccatcctggtggatatgatccagttccagaggtaaaacacaattgctgcgatcagcatctgtccgattctgggaaacagaccacagaagaccatcacaaaggctcgtag

SEQ ID NO: 446 - protein, 34 aa, Nostoc azollae
WMATLRILRCHPFHPGGYDPVPGLAEKSCCDHHD

SEQ ID NO: 447 - DNA, 105 bp, Nostoc azollae
tggatggcaactttgcggattttacgctgtcatcctttccatcctggtggttatgatcctgtaccaggactagcggaaaaatcctgttgtgaccatcatgattga

SEQ ID NO: 448 - protein, 28 aa, Synechococcus
WLTAKRFCRCHPLHPGGYDPVPEKKSVL

SEQ ID NO: 449 - DNA, 87 bp, Synechococcus
tggctaacagccaagcgcttttgtcgctgtcatccgcttcatcctggcgggtatgatccggtaccggagaagaaatcggtactctaa

SEQ ID NO: 450 - protein, 23 aa, Prochlorococcus marinus
WLTLRRLSRCHPFTPCGCDPVPD

SEQ ID NO: 451 - DNA, 72 bp, Prochlorococcus marinus
tggctcaccctgcggcgcctgtctcgttgccatccttttaccccctgtggttgcgacccggtgcctgattaa

SEQ ID NO: 452 - protein, 69 aa, Escherichia coli
MSYKKLYQLTAIFSLPLTILLVSLSSLRIVGEGNSYVDVFLSFIIFLGFIELIHGIRKILVWSGWKNGS

SEQ ID NO: 453 - DNA, 210 bp, Escherichia coli
atgagttataaaaaactgtaccaattgacggctatatttagtttacctcttactatcttattggtttcactttcatcccttcggattgttggcgaagggaattcttatgttgacgtttttctaagctttataatatttcttggttttattgagctgattcatgggattcgaaagattttggtctggtcaggctggaaaaacggaagttaa

SEQ ID NO: 454 - protein, 85 aa, Escherichia coli
MGLKLDLTWFDKSTEDFKGEEYSKDFGDDGSVMESLGVPFKDNVNNGCFDVIAEWVPLLQPYFNHQIDISDNEYFVSFDYRDGDW

SEQ ID NO: 455 - DNA, 258 bp, Escherichia coli
atgggacttaaattggatttaacttggtttgataaaagtacagaagattttaagggtgaggagtattcaaaagattttggagatgacggttcagttatggaaagtctaggtgtgccttttaaggataatgttaataacggttgctttgatgttatagctgaatgggtacctttgctacaaccatactttaatcatcaaattgatatttccgataatgagtattttgtttcgtttgattatcgtgatggtgattggtga

SEQ ID NO: 456 - protein, 113 aa, Escherichia coli
MSLRYYIKNILFGLYCTLIYIYLITKNSEGYYFLVSDKMLYAIVISTILCPYSKYAIEYIAFNFIKKDFFERRKNLNNAPVAKLNLFMLYNLLCLVLAIPFGLLGLFISIKNN

SEQ ID NO: 457 - DNA, 342 bp, Escherichia coli
atgagcttaagatactacataaaaaatattttatttggcctgtactgcacacttatatatatataccttataacaaaaaacagcgaagggtattatttccttgtgtcagataagatgctatatgcaatagtgataagcactattctatgtccatattcaaaatatgctattgaatacatagcttttaacttcataaagaaagattttttcgaaagaagaaaaaacctaaataacgcccccgtagcaaaattaaacctatttatgctatataatctactttgtttggtcctagcaatcccatttggattgctaggactttttatatcaataaagaataattaa

SEQ ID NO: 458 - protein, 85 aa, Escherichia coli
MGLKLHIHWFDKKTEEFKGGEYSKDFGDDGSVIESLGMPLKDNINNGWFDVEKPWVSILQPHFKNVIDISKFDYFVSFVYRDGNW

SEQ ID NO: 459 - DNA, 258 bp, Escherichia coli
atggggcttaaattacatattcattggtttgataagaaaaccgaagagtttaaaggcggtgaatactcaaaagacttcggtgatgatggttctgtcattgaaagtctggggatgcctttaaaggataatattaataatggttggtttgatgttgaaaaaccatgggtttcgatattacagccacactttaaaaatgtaatcgatattagtaaatttgattactttgtatcctttgtttaccgggatggtaactggtaa

SEQ ID NO: 460 - protein, 86 aa, Escherichia coli
MELKHSISDYTEAEFLEFVKKICRAEGATEEDDNKLVREFERLTEHPDGSDLIYYPRDDREDSPEGIVKEIKEWRAANGKSGFKQG

SEQ ID NO: 461 - DNA, 261 bp, Escherichia coli
atggaactgaaacatagtattagtgattataccgaggctgaatttctggagtttgtaaaaaaaatatgtagagctgaaggtgctactgaagaggatgacaataaattagtgagagagtttgagcgattaactgagcacccagatggttcagatctgatttattatcctcgcgatgacagggaagatagtcctgaagggattgtcaaggaaattaaagaatggcgagctgctaacggtaagtcaggatttaaacagggctga

SEQ ID NO: 462 - protein, 178 aa, Citrobacter freundii
MMNEHSIDTDNRKANNALYLFIIIGLIPLLCIFVVYYKTPDALLLRKIATSTENLPSITSSYNPLMTKVMDIYCKTAPFLALILYILTFKIRKLINNTDRNTVLRSCLLSPLVYAAIVYLFCFRNFELTTAGRPVRLMATNDATLLLFYIGLYSIIFFTTYITLFTPVTAFKLLKKRQ

SEQ ID NO: 463 - DNA, 537 bp, Citrobacter freundii
atgatgaatgaacactcaatagatacggacaacagaaaggccaataacgcattgtatttatttataataatcggattaataccattattgtgcatttttgttgtttactacaaaacgccagacgctttacttttacgtaaaattgctacaagcactgagaatctcccgtcaataacatcctcctacaacccattaatgacaaaggttatggatatttattgtaaaacagcgcctttccttgccttaatactatacatcctaacctttaaaatcagaaaattaatcaacaacaccgacaggaacactgtacttagatcttgtttattaagtccattggtctatgcagcaattgtttatctattctgcttccgaaattttgagttaacaacagccggaaggcctgtcagattaatggccaccaatgacgcaacactattgttattttatattggtctgtactcaataattttctttacaacctatatcacgctattcacaccagtcactgcatttaaattattaaaaaaaaggcagtaa

SEQ ID NO: 464 - protein, 111 aa, Escherichia coli
MNRKYYFNNMWWGWVTGGYMLYMSWDYEFKYRLLFWCISLCGMVLYPVAKWYIEDTALKFTRPDFWNSGFFADTPGKMGLLAVYTGTVFILSLPLSMIYILSVIIKRLSVR

SEQ ID NO: 465 - DNA, 336 bp, Escherichia coli
atgaacagaaaatattattttaataatatgtggtggggatgggtgacggggggatatatgctgtatatgtcatgggattatgagtttaaatacagattactgttctggtgtatttctctctgcggaatggttttgtatccggttgcaaaatggtatattgaagatacagctctaaaatttacccggcctgatttctggaacagcggtttttttgctgatacacctggaaaaatggggttgcttgcggtttatacgggtactgttttcatattatctcttccgttaagtatgatatatattctttctgttattataaaaaggctgtctgtaagatag

SEQ ID NO: 466 - protein, 115 aa, Escherichia coli
MKLDISVKYLLKSLIPILIILTVFYLGWKDNQENARMFYAFIGCIISAITFPFSMRIIQKMVIRFTGKEFWQKDFFTNPVGGSLTAIFELFCFVISVPVVAIYLIFILCKALSGK

SEQ ID NO: 467 - DNA, 348 bp, Escherichia coli
atgaaactggatatatctgtaaagtatttactgaaaagcctgataccaatcctcattattcttacagttttttatctgggatggaaagataaccaggaaaatgcaagaatgttttatgcgttcatcggatgcattatcagtgccattacttttcctttttcaatgaggataatacagaaaatggtaataaggtttacagggaaagaattctggcaaaaagacttctttacaaatccagttggcggaagcttaactgcaatatttgaattattctgtttcgttatatcagttcctgtggttgccatttacttaatttttatactctgcaaagccctttcaggaaaatga

SEQ ID NO: 468 - protein, 131 aa, Escherichia coli
MHNTLLEKIIAYLSLPGFHSLNNPPLSEAFNLYVHTAPLAATSLFIFTHKELELKPKSSPLRALKILTPFTILYISMIYCFLLTDTELTLSSKTFVLIVKKRSVFVFFLYNTIYWDIYIHIFVLLVPYRNI

SEQ ID NO: 469 - DNA, 396 bp, Escherichia coli
atgcacaatacactcctcgaaaaaatcatcgcatacctatccctaccaggatttcattcattaaacaacccgcccctaagcgaagcattcaatctctatgttcatacagcccctttagctgcaaccagcttattcatattcacacacaaagaattagagttaaaaccaaagtcgtcacctctgcgggcactaaagatattaactcctttcactattctttatatatccatgatatactgtttcttgctaactgacacagaactaaccttgtcatcaaaaacatttgtattaatagtcaaaaaacgatctgtttttgtcttttttctatataacactatatattgggatatatatattcacatatttgtacttttggttccttataggaacatataa

SEQ ID NO: 470 - protein, 85 aa, Escherichia coli
MELKNSISDYTETEFKKIIEDIINCEGDEKKQDDNLEHFISVTEHPSGSDLIYYPEGNNDGSPEAVIKEIKEWRAANGKSGFKQG

SEQ ID NO: 471 - DNA, 258 bp, Escherichia coli
atggaactgaaaaacagcattagtgattacactgaaactgaattcaaaaaaattattgaagacatcatcaattgtgaaggtgatgaaaaaaaacaggatgataacctcgagcattttataagtgttactgagcatcctagtggttctgatctgatttattacccagaaggtaataatgatggtagccctgaagctgttattaaagagattaaagaatggcgagctgctaacggtaagtcaggatttaaacagggctga

SEQ ID NO: 472 - protein, 98 aa, Lactococcus lactis subsp. lactis
MKKKQIEFENELRSMLATALEKDISQEERNALNIAEKALDNSEYLPKIILNLRKALTPLAINRTLNHDLSELYKFITSSKASNKNLGGGLIMSWGRLF

SEQ ID NO: 473 - DNA, 297 bp, Lactococcus lactis subsp. lactis
atgaaaaaaaaacaaatagaatttgaaaacgagctaagaagtatgttggctaccgcccttgaaaaagacattagtcaagaggaaagaaatgctctgaatattgcagaaaaggcgcttgacaattctgaatatttaccaaaaattattttaaacctcagaaaagccctaactccattagctataaatcgaacacttaaccatgatttatctgaactgtataaattcattacaagttccaaagcatcaaacaaaaatttaggtggtggtttaattatgtcgtggggacgactattctaa

SEQ ID NO: 474 - protein, 98 aa, Lactococcus lactis subsp. cremoris; identical to SEQ ID NO: 472

SEQ ID NO: 475 - DNA, 297 bp, Lactococcus lactis subsp. cremoris; identical to SEQ ID NO: 473

SEQ ID NO: 476 - protein, 87 aa, Escherichia coli
MNKMAMIDLAKLFLASKITAIEFSERICVERRRLYGVKDLSPNILNCGEELFMAAERFEPDADRANYEIDDNGLKVEVRSILEKFKL

SEQ ID NO: 477 - DNA, 249 bp, Escherichia coli
atgatcgatttggcgaaattatttttagcttcgaaaattacagtgattgagttttcagagcgaatttgtgttgaacggagaagattgtatggtgttaaggatttgtctccgaatatattaaattgtggggaagagttgtctatggctgctgagcgatttgagcctgatgcagatagggctaattatgaaattgatgataatggacttaaggtcgaggtccgatctatcttggaaaaacttaaatcataa

SEQ ID NO: 478 - protein, 83 aa, Escherichia coli
MKLSPKAAIEVCNEAAKKGLWILGIDGGHWLNPGFRIDSSASWTYDMPEEYKSKIPENNRLAIENIKDDIENGYTAFIITLKM

SEQ ID NO: 479 - DNA, 243 bp, Escherichia coli
atgaagttatcaccaaaagctgcaatagaagtttgtaatgaagcagcgaaaaaaggcttatggattttgggcattgatggtgggcattggctgaatcctggattcaggatagatagttcagcatcatggacatatgatatgccggagaatacaaatcaaaaatccctgaaaataatagattggctattgaaaatattaaagatgatattgagaatggatacactgctttcattatcacgttaa

SEQ ID NO: 480 - protein, 85 aa, Escherichia coli
MGLKLHINWFDKRTEEFKGGEYSKDFGDDGSVIERLGMPFKDNINNGWFDVIAEWVPLLQPYFNHQIDISDNEYFVSFDYRDGDW

SEQ ID NO: 481 - DNA, 258 bp, Escherichia coli
atggggcttaaattacatattaattggtttgataagacgaccgaggaatttaaaggtggtgagtattcaaaagattttggagatgatggctcggtcattgaacgtcttggaatgcctttaaaagataatatcaataatggttggtttgatgttatagctgaatgggtacctttgctacaaccatactttaatcatcaaattgatatttccgataatgagtattttgtttcgtttgattatcgtgatggtgattggtga

SEQ ID NO: 482 - protein, 85 aa, Escherichia coli
MELKKSIGDYTETEFKKIIENIINCEGDEKKQDDNLEHFISVTEHPSGSDLIYYPEGNNDGSPEAVIKEIKEWRAANGKSGFKQG

SEQ ID NO: 483 - DNA, 258 bp, Escherichia coli
gtggagctaaagaaaagtattggtgattacactgaaaccgaattcaaaaaaattattgaaaacatcatcaattgtgaaggtgatgaaaaaaaacaggatgataacctcgagcattttataagtgttactgagcatcctagtggttctgatctgatttattacccagaaggtaataatgatggtagccctgaagctgttattaaagagattaaagaatggcgagctgctaacggtaagtcaggatttaaacagggctga

SEQ ID NO: 484 - protein, 86 aa, Escherichia coli [sequence omitted]

SEQ ID NO: 485 - DNA, 261 bp, Escherichia coli
atggaactgaagcatagcattagtgattatacagaagctgaatttttacaacttgtaacaacaatttgtaatgcgaacacttccagtgaagaagaactggttaaattggttacacactttgaggaaatgactgagcaccctagtggtagtgatttaatatattacccaaaagaaggtgatgatgactcaccttcaggtattgtaaacacagtaaaacaatggcgagccgctaacggtaagtcaggatttaaacagggctaa

SEQ ID NO: 486 - protein, 141 aa, Escherichia coli
MLTLYGYIRNVFLYRMNDRSCGDFMKVISMKFIFILTIIALAAVFFWSEDKGPACYQVSDEQARTFVKNDYLQRMKRWDNDVQLLGTEIPKITWEKIERSLTDVEDEKTLLVPFKAEGPDGKRMYYGMYHCEEGYVEYAND

SEQ ID NO: 487 - DNA, 354 bp, Escherichia coli
atgaaagtaattagcatgaaatttatttttattttaacgattattgctcttgctgctgtttttttctggtctgaagataaaggtccggcatgctatcaggtcagcgatgaacaggccagaacgtttgtaaaaaatgattacctgcaaagaatgaaacgctgggacaacgatgtacaacttcttggtacagaaatcccgaaaattacatgggaaaagattgagagaagtttaacagatgttgaagatgaaaaaacacttcttgtcccatttaaagctgaaggcccggacggtaagagaatgtattatggcatgtaccattgtgaggagggatatgttgaatatgcgaatgactaa

SEQ ID NO: 488 - protein, 175 aa, Escherichia coli
MTSNKDKNKKANEILYAFSIIGIIPLMAILILRINDPYSQVLYYLYNKVAFLPSITSLHDPVMTTLMSNYNKTAPVMGILVFLCTYKTREIIKPVTRKLVVQSCFWGPVFYAILIYITLFYNLELTTAGGFFKLLSHNVITLFILYCSIYFTVLTMTYAILLMPLLVIKYFKGRQ

SEQ ID NO: 489 - DNA, 528 bp, Escherichia coli
atgaccagcaataaagataagaacaagaaagcaaacgaaatattatatgcattttccataatcgggattattccattaatggctatattaatacttcgaataaatgatccatattctcaagtgctgtactacttatataataaggtggcatttctcccttctattacatcattgcatgatcccgtcatgacaacacttatgtcaaactacaacaagacagcgccagttatgggtattctcgtttttctttgcacatataagacaagagaaatcataaagccagtaacaagaaaacttgttgtgcaatcctgtttctgggggcccgttttttatgccattctgatttatatcacactgttctataatctggaactaacaacagcaggtggtttttttaaattattatctcataatgtcatcactctgtttattttatattgctccatttactttactgttttaaccatgacatatgcgattttactgatgccattacttgtcattaaatattttaaagggaggcagtaa

SEQ ID NO: 490 - protein, 78 aa, Escherichia coli
MDRKRTKLELLFAFIINATAIYIALAIYDCVFRGKDFLSMHTFCFSALMSAICYFVGDNYYSISDKIKRRSYENSDSK

SEQ ID NO: 491 - DNA, 237 bp, Escherichia coli
atggatagaaaaagaacaaaattagagttgttatttgcatttataataaatgccaccgcaatatatattgcattagctatatatgattgtgtttttagaggaaaggactttttatccatgcatacattttgcttctctgcattaatgtctgcaatatgttactttgttggtgataattattattcaatatccgataagataaaaaggagatcatatgagaactctgactctaaatga

SEQ ID NO: 492 - protein, 113 aa, Shigella sonnei
MSLRYYIKNILFGLYCALIYIYLITKNNEGYYFLASDKMLYAIVISTILCPYSKYAIEHIFFKFIKKDFFRKRKNLNKCPRGKIKPYLCVYNLLCLVLAIPFGLLGLVYINKE

SEQ ID NO: 493 - DNA, 342 bp, Shigella sonnei
atgagtttaagatactacataaaaaatattttgtttggcctatactgcgcacttatatatatataccttataacaaaaaacaacgaagggtattatttcctagcgtcagataagatgctatacgcaatagtgataagcactattctatgcccatattcaaaatatgctattgaacacatattttttaagttcataaagaaagattttttcagaaaaagaaaaaacctaaataaatgcccccgtggcaaaattaaaccgtatttatgcgtatacaatctactttgtttggtcctagcaatcccatttggattgctaggacttgtttatatcaataaagaataa

SEQ ID NO: 494 - protein, 113 aa, Escherichia coli
MSLRYYIKNILFGLYCTLIYIYLITKNSEEYYFLVTDKMLYAIVISTILCPYSKYAIEHIAFNFIKKHFFERRKNLNNAPVAKLNLFMLYNLLCLVLAIPFGLLGLFISIKNN

SEQ ID NO: 495 - DNA, 342 bp, Escherichia coli
atgagcttaagatactacataaaaaatattttatttggcctgtactgcacacttatatatatataccttataacaaaaaacagcgaagagtattatttccttgtgacagataagatgctatatgcaatagtgataagcactattctatgtccatattcaaaatatgctattgaacacatagcttttaacttcataaagaaacattttttcgaaagaagaaaaaacctaaataacgcccccgtagcaaaattaaacctatttatgctatataatctactttgtttggtcctagcaatcccatttggattgctaggactttttatatcaataaagaataattaa

SEQ ID NO: 496 - protein, 113 aa, Leuconostoc gelidum
MRKNNILLDDAKIYTNKLYLLLIDRKDDAGYGDICDVLFQVSKKLDSTKNVEALINRLVNYIRITASTNRIKFSKDEEAVIIELGVIGQKAGLNGQYMADFSDKSQFYSIFER

SEQ ID NO: 497 - DNA, 342 bp, Leuconostoc gelidum
ttgagaaaaaataacattttattggacgatgctaaaatatacacgaacaaactctatttgctattaatcgatagaaaagatgacgctgggtatggagatatttgtgatgttttgtttcaggtatccaaaaaattagatagcacaaaaaatgtagaagcattgattaaccgattggtcaattatatacgaattaccgcttcaacaaacagaattaagttttcaaaagatgaagaggctgtaattatagaacttggtgtaattggtcagaaggctggattaaacggccaatacatggctgatttttctgacaaatctcagttttatagtatctttgaaagataa

SEQ ID NO: 498 - protein, 91 aa, Lactococcus lactis subsp. cremoris
MKKKVDTEKQITSWASDLASKNETKVQEKLILSSYIQDIENHVYFPKAMISLEKKLRDQNNICALSKEVNQFYFKVVEVNQRKSWMVGLIV

SEQ ID NO: 499 - DNA, 276 bp, Lactococcus lactis subsp. cremoris
atgaaaaaaaaagttgatacagaaaaacaaattacttcttgggcatctgacttagcttccaaaaatgaaacaaaggttcaagaaaaattaatactgtcttcttatattcaggacatcgaaaaccatgtttactttccaaaagcaatgatttctttagaaaaaaaattacgagaccaaaataatatttgcgctttatcaaaagaagtcaatcagttttattttaaagttgttgaagtaaatcaaagaaaatcctggatggtaggtttgatagtttaa

SEQ ID NO: 500 - protein, 112 aa, Pediococcus acidilactici
MNKTKSEHIKQQALDLFTRLQFLLQKHDTIEPYQYVLDILETGISKTKHNQQTPERQARVVYNKIASQALVDKLHFTAEENKVLAAINELAHSQKGWGEFNMLDTTNTWPSQ

SEQ ID NO: 501 - DNA, 339 bp, Pediococcus acidilactici
atgaataagactaagtcggaacatattaaacaacaagctttggacttatttactaggctacagtttttactacagaagcacgatactatcgaaccttaccagtacgttttagatattctggagactggtatcagtaaaactaaacataaccagcaaacgcctgaacgacaagctcgtgtagtctacaacaagattgccagccaagcgttagtagataagttacattttactgccgaagaaaacaaagttctagcagccatcaatgaattggcgcattctcaaaaagggtggggcgagtttaacatgctagatactaccaatacgtggcctagccaatag

SEQ ID NO: 502 - protein, 88 aa, Carnobacterium maltaromaticum
MIKDEKINKIYALVKSALDNTDVKNDKKLSLLLMRIQETSINGELFYDYKKELQPAISMYSIQHNFRVPDDLVKLLALVQTPKAWSGF

SEQ ID NO: 503 - DNA, 267 bp, Carnobacterium maltaromaticum
atgataaaagatgaaaaaataaataaaatctatgctttagttaagagcgcacttgataatacggatgttaagaatgataaaaaactttctttacttcttatgagaatacaagaaacatcaattaatggagaactattttacgattataaaaaagaattacagccagctattagtatgtactctattcaacataactttcgggttcctgacgatctagtaaaactgttagcattagttcaaacacctaaagcttggtcagggttttaa

SEQ ID NO: 504 - protein, 111 aa, Carnobacterium maltaromaticum
MDIKSQTLYLNLSEAYKDPEVKANEFLSKLVVQCAGKLTASNSENSYIEVISLLSRGISSYYLSHKRIIPSSMLTIYTQIQKDIKNGNIDTEKLRKYEIAKGLMSVPYIYF

SEQ ID NO: 505 - DNA, 336 bp, Carnobacterium maltaromaticum
atggatataaagtctcaaacattatatttgaatctaagcgaggcatataaagaccctgaagtaaaagctaatgaattcttatcaaaattagttgtacaatgtgctgggaaattaacagcttcaaacagtgagaacagttatattgaagtaatatcattgctatctaggggtatttctagttattatttatcccataaacgtataattccttcaagtatgttaactatatatactcaaatacaaaaggatataaaaaacgggaatattgacaccgaaaaattaaggaaatatgagatagcaaaaggattaatgtccgttccttatatatatttctaa

SEQ ID NO: 506 - protein, 245 aa, Lactococcus lactis subsp. lactis
MRRYLILIVALIGITGLSGCYQTSHKKVRFDEGSYTNFIYDNKSYFVTDKEIPQENVNNSKVKFYKLLIVDMKSEKLLSSSNKNSVTLVLNNIYEASDKSLCMGINDRYYKILPESDKGAVKALRLQNFDVTSDISDDNFVIDKNDSRKIDYMGNIYSISDTTVSDEELGEYQDVLAEVRVFDSVSGKSIPRSEWGRIDKDGSNSKQSRTEWDYGEIHSIRGKSLTEAFAVEINDDFKLATKVGN

SEQ ID NO: 507 - DNA, 738 bp, Lactococcus lactis subsp. lactis
atgagaagatatttaatacttattgtggccttaatagggataacaggtttatcagggtgttatcaaacaagtcataaaaaggtgaggtttgacgaaggaagttatactaattttatttatgataataaatcgtatttcgtaactgataaggagattcctcaggagaacgttaacaattccaaagtaaaattttataagctgttgattgttgacatgaaaagtgagaaacttttatcaagtagcaacaaaaatagtgtgactttggtcttaaataatatttatgaggcttctgacaagtcgctatgtatgggtattaacgacagatactataagatacttccagaaagtgataagggggcggtcaaagctttgagattacaaaactttgatgtgacaagcgatatttctgatgataattttgttattgataaaaatgattcacgaaaaattgactatatgggaaatatttacagtatatcggacaccaccgtatctgatgaagaattgggagaatatcaggatgttttagctgaagtacgtgtgtttgattcagttagtggcaaaagtatcccgaggtctgaatgggggagaattgataaggatggttcaaattccaaacagagtaggacggaatgggattatggcgaaatccattctattagaggaaaatctcttactgaagcatttgccgttgagataaatgatgattttaagcttgcaacgaaggtaggaaactag

SEQ ID NO: 508 - protein, 261 aa, Rhizobium leguminosarum bv. trifolii
MNDEICLTGGGRTTVTRRGGVVYREGGPWSSTVISLLRHLEASGFAEAPSVVGTGFDERGRETLSFIEGEFVHPGPWSEEAFPQFGMMLRRLHDATASFKPPENSMWRDWFGRNLGEGQHVIGHCDTGPWNIVCRSGLPVGLIDWEVAGPVRADIELAQACWLNAQLYDDDIAERVGLGSVTMRAHQVRLLLDGYGLSRKQRGGFVDKLITFAVHDAAEQAKEAAVTPESNDAEPLWAIAWRTRSASWMLHHRQTLEAALA

SEQ ID NO: 509 - DNA, 786 bp, Rhizobium leguminosarum bv. trifolii
atgaatgatgagatttgcctgacaggtggcggacgaacgactgtcacgcggcgcggcggagtcgtgtatcgcgaaggcggcccgtggtcatcaaccgtcatttcgctcctgcggcatctggaagcctctggcttcgctgaagctccttccgttgtcggcaccggtttcgatgagcgcggccgggagacattatcgtttatcgagggtgagtttgttcacccaggcccttggtcggaggaggcttttccgcaatttggaatgatgttgcggcgactgcacgatgccaccgcctcgttcaaacctcccgaaaactcgatgtggcgcgattggttcgggcgtaacctcggtgagggtcaacacgtaataggacactgcgacacaggcccatggaacattgtttgccggtcaggattgcctgtcgggttgatagattgggaggtggctgggcctgtcagggcggatatcgaattggcccaggcttgttggctgaatgcccagctctacgatgacgacattgcggagagggtcggattaggctctgtgaccatgagagcgcatcaagttcgcctgctgcttgacggctatggtctgtctcggaagcaacgcggcggcttcgtcgacaagctaatcacgttcgcagttcacgatgcggccgagcaggcgaaagaggcggctgtcacgccagagtcgaacgatgcggaaccgctatgggcaattgcctggcgcactagaagtgcctcctggatgctccatcatcggcaaacactggaagcagcgctggcatag

SEQ ID NO: 510 - protein, 436 aa, Bacillus subtilis
MNNIIPIMSLLFKQLYSRQGKKDAIRIAAGLVILAVFEIGLIRQAGIDESVLRKTYIILALLLMNTYMVFLSVTSQWKESYMKLSCLLPISSRSFWLAQSVVLFVDTCLRRTLFFFILPLFLFGNGTLSGAQTLFWLGRFSFFTVYSIIFGVVLSNHFVKKKNLMFLLHAAIFACVCISAALMPAATIPLCAVHILWAVVIDFPVFLQAPPQQGKMHSFMRRSEFSFYKREWNRFISSKAMLLNYAVMAVFSGFFSFQMMNTGIFNQQVIYIVISALLLICSPIALLYSIEKNDRMLLITLPIKRKTMFWAKYRFYSGLLAGGFLLVVMIVGFISGRSISVLTFLQCIELLLAGAYIRLTADEKRPSFSWQTEQQLWSGFSKYRSYLFCLPLFLAILAGTAVSLAVIPIAGLVIVYYLQKQDGGFFDTSKRERLGS

SEQ ID NO: 511 - DNA, 1000 bp, Bacillus subtilis
atgaataacataatccctatcatgtctttgctgttcaaacagctttacagccggcaagggaaaaaggacgccatccgcattgccgcaggccttgtcattctggccgtgtttgaaatcgggctgatccgccaggccggcattgatgaatcggtgttgcgcaaaacgtatatcatactcgcgcttcttttgatgaacacatatatggtgtttctttccgtgacatcacaatggaaggaatcttatatgaagctgagctgcctgctgccgatttcttcacggagcttttggctcgcccagagtgtcgttttgtttgtcgatacctgtttgagaagaactttattcttttttattttaccgctgttcttatttggaaacggaacgctgtcaggggcgcaaacattgttttggctcggcaggttttcgttttttaccgtttactccattattttcggagttgtgctaagcaaccacttcgtcaaaaagaagaacttgatgtttctgctgcatgcggcgatattcgcctgtgtatgtatcagcgccgctttgatgccggccgccacgattccgctttgcgcggttcatatcctgtgggcggtggtcattgactttcctgtctttctgcaggcgcctccgcagcagggcaagatgcattcatttatgcggcgatctgaattttcgttttacaaaagagaatggaaccgatttatctcttctaaagcgatgctgttaaattacgcggtaatggcggtattcagcggcttcttttcgttccagatgatgaacaccggcatcttcaatcagcaagtgatttatatcgtgatttccgcgcttttgctcatctgctcgccgatcgcccttttgtattcgattgaaaaaaatgaccggatgctgctcatcacgcttccgatcaagcgaaaaacgatgttttgggcgaaatatcgcttttattcaggcctattggcaggcggatttctccttgtcgtgatgattgtgggtttca

SEQ ID NO: 512 - protein, 239 aa, Bacillus subtilis
MSILDIHDVSVWYERDNVILEQVDLHLEKGAVYGLLGVNGAGKTTLINTLTGVNRNFSGRFTLCGIEAEAGMPQKTSDQLKTHRYFAADYPLLFTEITAKDYVSFVHSLYQKDFSEQQFASLAEAFHFSKYINRRISELSLGNRQKVVLMTGLLLRAPLFILDEPLVGLDVESIEVFYQKMREYCEAGGTILFSSHLLDVVQRFCDYAAILHNKQIQKVIPIGEETDLRREFFEVIGHE

SEQ ID NO: 513 - DNA, 716 bp, Bacillus subtilis
gcattttggatatacacgatgtatccgtttggtatgaacgggacaacgtcatcttagagcacgtggacttacacttagaaaaaggcgccgtttacggattgcttggggtaaacggtgccggcaaaacaacactgatcaatacgctgacaggagtgaaccgcaattacagcgggggctttacgctgtgcggcattgaagctgaggccggcatgccgcagaaaacatcagatcaactgaagattcaccgttacttcgccgctgattatccgctgctgtttacagaaattacggcgaaggactatgtgtctttcgtccattcgctttatcaaaaggatttttcagagcgacagtttgccagtttggctgaggcctttcatttttcaaaatacatcaacaggagaatctcggagctgtccttggggaacaggcaaaaggttgtgttgatgacaggattattgctgcgggctcccctgtttattttggatgagccgctcgtcggtttggatgtggaatcaatagaggtcttttatcagaaaatgcgggagtactgtgaggaaggcggaaccattttgttttcttcccatctgctcgatgtcgtgcagagattttgtgattttgcggccattctgcacaacaaacagatccaaaaggtcattccgattggggaggagaccgatctgcggcgggaattttttgaggttatcggccatgaataa

SEQ ID NO: 514 - protein, 53 aa, Bacillus subtilis
MSPAQRRILLYILSFIFVIGAVVYFVKSDYLFTLIFIAIAILFGMRARKADSR

SEQ ID NO: 515 - DNA, 162 bp, Bacillus subtilis
ttgtcaccagcacaaagaagaattttactgtatatcctttcatttatctttgtcatcggcgcagtcgtctattttgtcaaaagcgattatctgtttacgctgattttcattgccattgccattctgttcgggatgcgcgcgcggaaggctgactcgcgatga

SEQ ID NO: 516 - protein, 87 aa, Escherichia coli
MELKNSISDYTEAEFVQLLKEIEKENVAATDDVLDVLLEHFVKITEHPDGTDLIYYPSDNRDDSPEGIVKEIKEWRAANGKPGFKQG

SEQ ID NO: 517 - DNA, 264 bp, Escherichia coli
atggaactgaaaaatagtattagtgattacacagaggctgagtttgttcaacttcttaaggaaattgaaaaagagaatgttgctgcaactgatgatgtgttagatgtgttactcgaacactttgtaaaaattactgagcatccagatggaacggatctgatttattatcctagtgataatagagacgatagccccgaagggattgtcaaggaaattaaagaatggcgagctgctaacggtaagccaggatttaaacagggctga

SEQ ID NO: 518 - protein, 87 aa, Pseudomonas aeruginosa
MKSKISEYTEKEFLEFVEDIYTNNKKKFPTEESHIQAVLEFKKLTEHPSGSDLLYYPNENREDSPAGVVKEVKEWRASKGLPGFKAG

SEQ ID NO: 519 - DNA, 264 bp, Pseudomonas aeruginosa
atgaagtccaagatttccgaatatacggaaaaagagtttcttgagtttgttgaagacatatacacaaacaataagaaaaagttccctaccgaggagtctcatattcaagccgtgcttgaatttaaaaaactaacggaacacccaagcggctcagaccttctttactaccccaacgaaaatagagaagatagcccagctggagttgtaaaggaagttaaagaatggcgtgcttccaaggggcttcctggctttaaggccggttag

SEQ ID NO: 520 - protein, 87 aa, Pseudomonas aeruginosa
MKSKISEYTEKEFLEFVKDIYTNNKKKFPTEESHIQAVLEFKKLTEHPSGSDLLYYPNENREDSPAGVVKEVKEWRASKGLPGFKAG

SEQ ID NO: 521 - DNA, 264 bp, Pseudomonas aeruginosa
atgaagtccaagatttccgaatatacggaaaaagagtttcttgagtttgttaaagacatatacacaaacaataagaaaaagttccctaccgaggagtctcatattcaagccgtgcttgaatttaaaaaactaacggaacacccaagcggctcagaccttctttactaccccaacgaaaatagagaagatagcccagctggagttgtaaaggaagttaaagaatggcgtgcttccaaggggcttcctggctttaaggccggttag

SEQ ID NO: 522 - protein, 95 aa, Enterococcus hirae
MDFTKEEKLLNAISKVYNEATIDDYPDLKEKLFLYSKEISEGKSVGEVSMKLSSFLGRYILKHKFGLPKSLIELQEIVSKESQVYRGWASIGIWS

SEQ ID NO: 523 - DNA, 288 bp, Enterococcus hirae
atggattttactaaagaagaaaaacttttaaatgcaattagtaaagtatacaatgaagcaactatagatgactatcctgacttaaaagaaaagctctttctttattctaaagaaatcagtgagggaaaaagtgttggtgaagttagtatgaaattaagtagttttcttggaagatatattttaaaacataaatttggattacctaaatctttaatagaattacaagaaattgttagtaaggaatctcaagtatatagaggatgggcttctattggtatttggagttaa

SEQ ID NO: 524 - protein, 113 aa, Leuconostoc mesenteroides
MKKKYRYLEDSKNYTSTLYSLLVDNVDKPGYSDICDVLLQVSKKLDNTQSVEALINRLVNYIRITASTYKIIFSKKEEELIIKLGVIGQKAGLNGQYMADFSDKSQFYSVFDQ

SEQ ID NO: 525 - DNA, 342 bp, Leuconostoc mesenteroides
ttgaaaaaaaagtatcggtatttagaagatagcaaaaattacactagtacactctattctctgttagttgataatgttgacaaacctggatactcagatatttgcgatgttttgcttcaagtttctaagaagttggataatactcaaagtgttgaagcgctaattaatcgattggttaattatattcgtattactgcttcaacatacaaaattattttttcaaaaaaagaagaggaattgattataaaacttggtgttattggacaaaaagctggacttaatggtcagtatatggctgatttttcagacaagtctcagttttacagcgttttcgatcagtaa

SEQ ID NO: 526 - protein, 93 aa, Escherichia coli
MSFLNFAFSPVFFSIMACYFIVWRNKRNEFVCNRLLSIIIISFLICFIYPWLNYKIEVKYYIFEQFYLFCFLSSLVAVVINLIVYFILYRRCI

SEQ ID NO: 527 - DNA, 282 bp, Escherichia coli
atgagttttcttaattttgcattttctcctgtattcttctccattatggcgtgttatttcattgtatggagaaataaacgaaacgaatttgtctgcaatagattgctatcaattataataatatcttttttgatatgcttcatatatccatggctaaattacaaaatcgaagttaaatattatatatttgaacagttttatcttttttgttttttatcgtcactcgtggctgttgtaataaacctaattgtatactttatattatacaggagatgtatatga

SEQ ID NO: 528 - protein, 96 aa, Escherichia coli
MHLKYYLHNLPESLIPWILILIFNDNDNTPLLFIFISSIHVLLYPYSKLTISRYIKENTKLKKEPWYLCKLSALFYLLMAIPVGLPSFIYYTLKRN

SEQ ID NO: 529 - DNA, 291 bp, Escherichia coli
atgcatttaaaatactacctacataatttacctgaatcacttataccatggattcttattttaatatttaacgacaatgataacactcctttgttatttatatttatatcatcaatacatgtattgctatatccatactctaaattaaccatatctagatatatcaaagaaaatacaaagttaaaaaaagaaccctggtacttatgcaagttatctgcattgttttatttattaatggcaatcccagtaggattgccaagtttcatatattacactctaaagagaaattaa

SEQ ID NO: 530 - protein, 344 aa, Escherichia coli
MMIQSHPLLAAPLAVGDTIGFFSSSAPATVTAKNRFFRGVEFLQRKGFKLVSGKLTGKTDFYRSGTIKERAQEFNELVYNPDITCIMSTIGGDNSNSLLPFLDYDAIIANPKIIIGYSDTTALLAGIYAKTGLITFYGPALIPSFGEHPPLVDITYESFIKILTRKQSGIYTYTLPEKWSDESINWNENKILRPKKLYKNNCAFYGSGKVEGRVIGGNLNTLTGIWGSEWMPEILNGDILFIEDSRKSIATIERLFSMLKLNRVFDKVSAIILGKHELFDCAGSKRRPYEVLTEVLDGKQIPVLDGFDCSHTHPMLTLPLGVKLAIDFDNKNISITEQYLSTEK

SEQ ID NO: 531 - DNA, 1000 bp, Escherichia coli
atgatgatacaatctcatccactactggccgctcccctggcagtaggagatacaattggtttcttttcatcatctgctccggcaacagttactgcaaaaaatcgtttttttcggggagttgagtttcttcagagaaagggatttaagctggtatcagggaagcttaccggtaaaacagatttttatcgttcaggtactattaaagaaagagctcaagaatttaatgagttagtctacaatcctgatattacctgtataatgtcaacgatcggtggagataacagtaattcactactaccgtttctggactatgatgctatcattgcaaaccccaaaattatcataggttactcagatacaactgctttattagcaggaatatatgcaaaaacagggttaataacattctatggaccagctcttattccttcgtttggtgaacatccacctcttgtggatataacatatgaatcatttattaaaatactaacaagaaaacaatcaggaatatatacctacacattacctgaaaagtggagtgatgagagcataaactggaatgaaaacaagatattaaggcctaagaagctatataaaaacaactgtgccttttatggttccggaaaagttgaggggcgtgtaattggaggaaatctaaatactttgacaggtatatgggggagtgaatggatgcctgaaattcttaatggagatatattgtttattgaggacagtcggaaaagcattgcaacaattgaacgattattctctatgctaaagcttaatcgcgtgtttgataaagttagtgcaataatactcgggaaacatgagctttttgattgtgcaggaagtaaacgcagaccatatgaagtattaacagaggtattagatgggaaacagattcctgtactggatggatttgattgttcacatacacatccaatgctaactcttccacttggtgtaaaattagctattgactttgacaacaaaaatatat

SEQ ID NO: 532 - protein, 90 aa, Lactobacillus sakei
MKADYKKINSILTYTSTALKNPKIIKDKDLVVLLTIIQEEAKQNRIFYDYKRKFRPAVTRFTIDNNFEIPDCLVKLLSAVETPKAWSGFS

SEQ ID NO: 533 - DNA, 268 bp, Lactobacillus sakei
ggcagattataaaaaaataaattcaatactaacttacacatctactgctttaaaaaaccctaaaattataaaagataaagatttagtagtccttctaactattattcaagaagaagccaaacaaaatagaatcttttatgattataaaagaaaatttcgtccagcggttactcgctttacaattgataataattttgagattcctgattgtttggttaaactactgtcagctgttgaaacacctaaggcgtggtctggatttagttag

SEQ ID NO: 534 - protein, 83 aa, Escherichia coli
MKLSPKAAIEVCNEAAKKGLWILGIDGGHWLNPGFRIDSSASWTYDMPEEYKSKTPENNRLAIENIKDDIENGYTAFIITLKM

SEQ ID NO: 535 - DNA, 251 bp, Escherichia coli
tgaagttatcaccaaaagctgcaatagaagtttgtaatgaagcagcgaaaaaaggcttatggattttgggcattgatggtgggcattggctgaatcctggattcaggatagatagttcagcatcatggacatatgatatgccggaggaatacaaatcaaaaacccctgaaaataatagattggctattgaaaatattaaagatgatattgagaatggatacactgctttcattatcacgttaaagatgtaa

SEQ ID NO: 536 - protein, 436 aa, Bacillus subtilis
MNNIFPIMSLLFKQLYSRQGKKDAIRIAAGLVILAVFEIGLIRQAGIDESVLGKTYIILALLLMNTYMVFLSVTSQWKESYMKLSCLLPISSRSFWLAQSVVLFVDTCLRRTLFFFILPLFLFGNGTLSGAQTLFWLGRFSFFTVYSILFGVMLSNHFVKKKNSMFLLHAAVFAFVCLSAAFMPAVTIPLCAVHMLWAVIIDFPVFLQAPPHQSKMHFFMRRSEFSFYKREWNRFISSKAMLLNYVVMAAFSGFFSFQMMNTGIFNQQVIYIVISALLLICSPIALLYSIEKNDRMLLITLPIKRRTMFWAKYRFYSGLLAGGFLLVAIIVGFISGRPISALTFVQCMELLLAGAFIRLTADEKRPSFGWQTEQQLWSGFSKYRSYLFCLPLFLATLAGTAVSLAVIPIAALIIVYYLQKQDGGFFDTSKRERIGS

SEQ ID NO: 537 - DNA, 1000 bp, Bacillus subtilis
ttggggaggagaccgatctgcggcgggaattttttgaggttatcggccatgaataacatattccccatcatgtcgttgctgttcaaacagctgtacagccggcaagggaaaaaggacgctatccgcattgctgcagggcttgtgattctcgccgtgtttgaaatcgggctgatccgacaagccggcattgacgaatcggtgttgggaaaaacgtatatcatattggcgcttctcttaatgaacacgtatatggtgtttctttccgtgacatcacaatggaaggaatcttatatgaagctgagctgtctgctgccgatttcatcacggagcttttggctcgcccagagtgtcgttctgtttgtcgatacctgtttgagaagaacgttattcttttttattttaccgctgttcttatttggaaacggaacgctgtcaggggcgcaaacattgttttggcttggcagattttcgttttttaccgtttactcgattctattcggagttatgctaagcaaccatttcgtcaaaaagaagaactcgatgtttctgctgcatgcggcggtattcgcctttgtatgcctcagtgccgcttttatgccggccgtcacgatcccgctatgcgcggttcacatgctatgggcggtgatcattgactttccggtctttctgcaggcgcctccgcatcagagcaagatgcatttttttatgcggcgatctgaattttcgttttacaaaagagaatggaaccgatttatttcttctaaagcgatgctgttaaattacgtggtgatggcggcgttcagcggattcttttcgttccagatgatgaacactggcatcttcaatcagcaagtgatttatattgtgatttccgctctattgctgatttgctcgccgatcgcccttttgtactctattgaaaaaaacgatcgcatgctgctcatcacgcttccaattaaaagaagaacgatgttttgggcgaaatatcgcttttattcag

SEQ ID NO: 538 - protein, 580 aa, Escherichia coli
MERKQKNSLFNYIYSLMDVRGKFLFFSMLFITSLSSIIISISPLILAKITDLLSGSLSNFSYEYLVLLACLYMFCVISNKASVFLFMILQSSLRINMQKKMSLKYLRELYNENITNLSKNNAGYTTQSLNQASNDIYILVRNVSQNILSPVIQLISTIVVVLSTKDWFSAGVFFLYILVFVIFNTRLTGSLASLRKHSMDITLNSYSLLSDTVDNMIAAKKNNALRLISERYEDALTQENNAQKKYWLLSSKVLLLNSLLAVILFGSVFIYNILGVLNGVVSIGHFIMITSYIILLSTPVENIGALLSEIRQSMSSLAGFIQRHAENKATSPSIPFLNMERKLNLSIRELSFSYSDDKKILNSVSLDLFTGKMYSLTGPSGSGKSTLVKIISGYYKNYFGDIYLNDISLRNISDEDLNDAIYYLTQDDYIFMDTLRFNLRLANYDASENEIFKVLKLANLSVVNNEPVSLDTHLINRGNNYSGGQKQRISLARLFLRKPAIIIIDEATSALDYINESEILSSIRTHFPDALIINISHRINLLECSDCVYVLNEGNIVASGHFRDLMVSNEYISGLASVTE

SEQ ID NO: 539 - DNA, 1000 bp, Escherichia coli
atggaaagaaaacagaaaaactcattatttaattatatttattcattaatggatgtaagaggtaaatttttattcttttccatgttattcattacatcattatcatcgataatcatatctatttcaccattgattcttgcaaagattacagatttactgtctggctcattgtcaaattttagttatgaatatctggttttacttgcctgtttatacatgttttgcgttatatctaataaagcaagtgtttttttatttatgatactgcaaagtagtctacgtattaacatgcagaaaaaaatgtcgctaaagtatttgagagaattgtataacgaaaatataactaacttgagtaaaaataatgctggatatacaacgcaaagtcttaaccaggcttcaaatgacatttatattcttgtgagaaatgtttcccagaatatcctgtcacctgttatacaacttatttccactattgttgttgttttatctacgaaggactggttttctgccggtgtgttttttctctatattctggtatttgtaatttttaataccagactgactggcagtttagcgtctctcagaaaacacagcatggatatcactcttaactcttatagtctgttatctgatactgttgataacatgatagcagctaaaaagaataatgcattaagacttatttctgaacgttatgaagatgctctcactcaggaaaacaatgctcagaaaaaatactggttactcagttctaaagttcttttattgaactctttacttgctgtaatattatttggttctgtattcatatataatattttaggtgtgctgaatggtgtagttagtatcggccacttcattatgattacatcatatatcattcttctttcaacgccagtggaaaatataggggcattgctaagtgagatcaggcagtcaatgtctagcctggcaggttttattcaacgtcatgccgagaataaagccacatctccttcaa

SEQ ID NO: 540 - protein, 95 aa, Klebsiella pneumoniae
MTLLSFGFSPVFFSVMAFCIISRSKFYPQRTRNKVIVLILLTFFICFLYPLTKVYLVGSYGIFDKFYLFCFISTLIAIAINVVILTINGAKNERN

SEQ ID NO: 541 - DNA, 288 bp, Klebsiella pneumoniae
atgacattactttcatttggattttctcctgttttcttttcagtcatggcgttctgtatcatttcacgtagtaaattctatccgcagagaacgcgaaacaaagttattgttctgattttactaactttttttatttgttttttatatccattaacaaaagtgtatctggtgggaagttacggtatatttgacaaattctacctcttttgctttatttctacgttaattgcaatagcaattaacgtagtgatacttacaataaatggagctaagaatgagagaaattag

SEQ ID NO: 542 - RNA, 13 nt, Artificial Sequence
  Kozak sequence
gccgccrccaugg

SEQ ID NO: 543 - RNA, 6 nt, Artificial Sequence
  Shine-Delgarno sequence
ggaggu

SEQ ID NO: 544 - DNA, 30 bp, Artificial Sequence
  Lead promoter
gaaaaccttgtcaatgaagagcgatctatg

SEQ ID NO: 545 - DNA, 30 bp, Artificial Sequence
  FecA promoter
ttctcgttcgactcatagctgaacacaaca

SEQ ID NO: 546 - DNA, 16 bp, Artificial Sequence
  Cu-sensitive promoter
atgacaaaattgtcat

SEQ ID NO: 547 - DNA, 30 bp, Artificial Sequence
  Fe promoter
accaatgctgggaacggccagggcacctaa

SEQ ID NO: 548 - DNA, 30 bp, Artificial Sequence
  Fe and UV promoters
ctgaaagcgcataccgctatggagggggtt

SEQ ID NO: 549 - DNA, 30 bp, Artificial Sequence
  PrFe (PI + PII rus operon)
tagatatgcctgaaagcgcataccgctatg

SEQ ID NO: 550 - DNA, 30 bp, Artificial Sequence
  Lux cassette right promoter
tgttatagtcgaatacctctggcggtgata

SEQ ID NO: 551 - DNA, 30 bp, Artificial Sequence
  P(Las) TetO
ttttggtacactccctatcagtgatagaga

SEQ ID NO: 552 - DNA, 30 bp, Artificial Sequence
  P(Las) CIO
ctttttggtacactacctctggcggtgata

SEQ ID NO: 553 - DNA, 30 bp, Artificial Sequence
  P(Rhl)
tacgcaagaaaatggtttgttatagtcgaa

SEQ ID NO: 554 - DNA, 30 bp, Artificial Sequence
  Double Promoter (LuxR/HSL, positive / cI, negative)
cgtgcgtgttgataacaccgtgcgtgttga

SEQ ID NO: 555 - DNA, 30 bp, Artificial Sequence
  P2 promoter in agr operon from S. aureus
agattgtactaaatcgtataatgacagtga

SEQ ID NO: 556 - DNA, 30 bp, Artificial Sequence
  plux-cI hybrid promoter
gtgttgatgcttttatcaccgccagtggta

SEQ ID NO: 557 - DNA, 30 bp, Artificial Sequence
  plux-lac hybrid promoter
agtgtgtggaattgtgagcggataacaatt

SEQ ID NO: 558 - DNA, 30 bp, Artificial Sequence
  CinR, CinL and glucose controlled promotor
acatcttaaaagttttagtatcatattcgt

SEQ ID NO: 559 - DNA, 30 bp, Artificial Sequence; identical to SEQ ID NO: 553
  RhIR promoter repressible by CI

SEQ ID NO: 560 - DNA, 30 bp, Artificial Sequence
  Reverse Lux Promoter
tcttgcgtaaacctgtacgatcctacaggt

SEQ ID NO: 561 - DNA, 30 bp, Artificial Sequence
  rhlI promoter
atcctcctttagtcttccccctcatgtgtg

SEQ ID NO: 562 - DNA, 30 bp, Artificial Sequence
  lasI promoter
taaaattatgaaatttgcataaattcttca

SEQ ID NO: 563 - DNA, 30 bp, Artificial Sequence
  LuxR+3OC6HSL independent R0065
gtgttgactattttacctctggcggtgata

SEQ ID NO: 564 - DNA, 30 bp, Artificial Sequence
  LasR/LasI Inducible & RHLR/RHLI repressible Promoter
gaaatctggcagtttttggtacacgaaagc

SEQ ID NO: 565 - DNA, 30 bp, Artificial Sequence
  pLux/cI Hybrid Promoter
acaccgtgcgtgttgatatagtcgaataaa

SEQ ID NO: 566 - DNA, 30 bp, Artificial Sequence
  pLas promoter
aaaattatgaaatttgtataaattcttcag

SEQ ID NO: 567 - DNA, 30 bp, Artificial Sequence
  pLas/cI Hybrid Promoter
ggttctttttggtacctctggcggtgataa

SEQ ID NO: 568 - DNA, 30 bp, Artificial Sequence
  pLas/Lux Hybrid Promoter
tgtaggatcgtacaggtataaattcttcag

SEQ ID NO: 569 - DNA, 30 bp, Artificial Sequence
  pLux
caagaaaatggtttgttatagtcgaataaa

SEQ ID NO: 570 - DNA, 30 bp, Artificial Sequence
  pLux/Las Hybrid Promoter
ctatctcatttgctagtatagtcgaataaa

SEQ ID NO: 571 - DNA, 30 bp, Artificial Sequence
  Hybrid promoter: HSL-LuxR activated, P22 C2 repressed
tagtttataatttaagtgttctttaatttc

SEQ ID NO: 572 - DNA, 30 bp, Artificial Sequence
  PAI+LasR -> LuxI (AI)
caccttcgggtgggcctttctgcgtttata

SEQ ID NO: 573 - DNA, 30 bp, Artificial Sequence
  PAI+LasR -> LasI & AI+LuxR --| LasI
aataactctgatagtgctagtgtagatctc

SEQ ID NO: 574 - DNA, 30 bp, Artificial Sequence; identical to SEQ ID NO: 572
  PAI+LasR -> LasI+GFP & AI+LuxR --| LasI+GFP

SEQ ID NO: 575 - DNA, 30 bp, Artificial Sequence; identical to SEQ ID NO: 572
  Complex QS -> LuxI & LasI circuit

SEQ ID NO: 576 - DNA, 30 bp, Artificial Sequence; identical to SEQ ID NO: 569
  position 3 mutated promoter lux pR-3 (luxR & HSL regulated)

SEQ ID NO: 577 - DNA, 30 bp, Artificial Sequence; identical to SEQ ID NO: 569
  position 5 mutated promoter lux pR-5 (luxR & HSL regulated)

SEQ ID NO: 578 - DNA, 30 bp, Artificial Sequence; identical to SEQ ID NO: 569
  position 3&5 mutated promoter lux pR-3/5 (luxR & HSL regulated)

SEQ ID NO: 579 - DNA, 30 bp, Artificial Sequence
  Promoter (HSL-mediated luxR repressor)
ttgacacctgtaggatcgtacaggtataat

SEQ ID NO: 580 - DNA, 30 bp, Artificial Sequence; identical to SEQ ID NO: 569
  Promoter (luxR & HSL regulated -- lux pR)

SEQ ID NO: 581 - DNA, 30 bp, Artificial Sequence
  Promoter (luxR & HSL regulated -- lux pL)
cacgcaaaacttgcgacaaacaataggtaa

SEQ ID NO: 582 - DNA, 30 bp, Artificial Sequence
  Promoter (RhlR & C4-HSL regulated)
gttagctttcgaattggctaaaaagtgttc

SEQ ID NO: 583 - DNA, 30 bp, Artificial Sequence
  Promoter (cinR and HSL regulated)
ccattctgctttccacgaacttgaaaacgc

SEQ ID NO: 584 - DNA, 30 bp, Artificial Sequence
  Promoter (LasR & PAI regulated)
ggccgcgggttctttttggtacacgaaagc

SEQ ID NO: 585 - DNA, 30 bp, Artificial Sequence
  Promoter, Standard (luxR and HSL regulated -- lux pR)
aagaaaatggtttgttgatactcgaataaa

SEQ ID NO: 586 - DNA, 30 bp, Artificial Sequence
  P(Bla)
gtttatacataggcgagtactctgttatgg

SEQ ID NO: 587 - DNA, 30 bp, Artificial Sequence
  P(Cat)
agaggttccaactttcaccataatgaaaca

SEQ ID NO: 588 - DNA, 30 bp, Artificial Sequence
  P(Kat)
taaacaactaacggacaattctacctaaca

SEQ ID NO: 589 - DNA, 30 bp, Artificial Sequence
  Template for Building Primer Family Member
acatcaagccaaattaaacaggattaacac

SEQ ID NO: 590 - DNA, 30 bp, Artificial Sequence
  Reverse lambda cI-regulated promoter
gaggtaaaatagtcaacacgcacggtgtta

SEQ ID NO: 591 - DNA, 30 bp, Artificial Sequence
  Key Promoter absorbs 3
caggccggaataactccctataatgcgcca

SEQ ID NO: 592 - DNA, 30 bp, Artificial Sequence
  constitutive promoter family member
ggctagctcagtcctaggtacagtgctagc

SEQ ID NO: 593 - DNA, 30 bp, Artificial Sequence
  constitutive promoter family member
agctagctcagtcctaggtattatgctagc

SEQ ID NO: 594 - DNA, 30 bp, Artificial Sequence
  constitutive promoter family member
agctagctcagtcctaggtactgtgctagc

SEQ ID NO: 595 - DNA, 30 bp, Artificial Sequence
  constitutive promoter family member
agctagctcagtcctagggattatgctagc

SEQ ID NO: 596 - DNA, 30 bp, Artificial Sequence
  constitutive promoter family member
agctagctcagtcctaggtattgtgctagc

SEQ ID NO: 597 - DNA, 30 bp, Artificial Sequence
  constitutive promoter family member
ggctagctcagtcctaggtactatgctagc

SEQ ID NO: 598 - DNA, 30 bp, Artificial Sequence
  constitutive promoter family member
ggctagctcagtcctaggtatagtgctagc

SEQ ID NO: 599 - DNA, 30 bp, Artificial Sequence
  constitutive promoter family member
ggctagctcagccctaggtattatgctagc

SEQ ID NO: 600 - DNA, 30 bp, Artificial Sequence
  constitutive promoter family member
agctagctcagtcctaggtataatgctagc

SEQ ID NO: 601 - DNA, 30 bp, Artificial Sequence
  constitutive promoter family member
agctagctcagtcctagggactgtgctagc

SEQ ID NO: 602 - DNA, 30 bp, Artificial Sequence
  constitutive promoter family member
ggctagctcagtcctaggtacaatgctagc

SEQ ID NO: 603 - DNA, 30 bp, Artificial Sequence; identical to SEQ ID NO: 598
  constitutive promoter family member

SEQ ID NO: 604 - DNA, 30 bp, Artificial Sequence; identical to SEQ ID NO: 595
  constitutive promoter family member

SEQ ID NO: 605 - DNA, 30 bp, Artificial Sequence
  constitutive promoter family member
ggctagctcagtcctagggattatgctagc

SEQ ID NO: 606 - DNA, 30 bp, Artificial Sequence; identical to SEQ ID NO: 602
  constitutive promoter family member

SEQ ID NO: 607 - DNA, 30 bp, Artificial Sequence
  constitutive promoter family member
agctagctcagcccttggtacaatgctagc

SEQ ID NO: 608 - DNA, 30 bp, Artificial Sequence
  constitutive promoter family member
agctagctcagtcctagggactatgctagc

SEQ ID NO: 609 - DNA, 30 bp, Artificial Sequence
  constitutive promoter family member
agctagctcagtcctagggattgtgctagc

SEQ ID NO: 610 - DNA, 30 bp, Artificial Sequence
  constitutive promoter family member
ggctagctcagtcctaggtattgtgctagc

SEQ ID NO: 611 - DNA, 30 bp, Artificial Sequence; identical to SEQ ID NO: 600
  constitutive promoter family member

SEQ ID NO: 612 - DNA, 30 bp, Artificial Sequence
  1bp mutant from J23107
ggctagctcagtcctaggtattatgctagc

SEQ ID NO: 613 - DNA, 30 bp, Artificial Sequence; identical to SEQ ID NO: 602
  1bp mutant from J23114

SEQ ID NO: 614 - DNA, 30 bp, Artificial Sequence
  pBAD reverse
aaagtgtgacgccgtgcaaataatcaatgt

SEQ ID NO: 615 - DNA, 30 bp, Artificial Sequence
  NikR promoter, a protein of the ribbon helix-helix family of trancription factors that repress expre
gacgaatacttaaaatcgtcatacttattt

SEQ ID NO: 616 - DNA, 30 bp, Artificial Sequence
  lacq_Promoter
aaacctttcgcggtatggcatgatagcgcc

SEQ ID NO: 617 - DNA, 30 bp, Artificial Sequence
  lacIQ - promoter sequence
tgatagcgcccggaagagagtcaattcagg

SEQ ID NO: 618 - DNA, 30 bp, Artificial Sequence
  E. Coli CreABCD phosphate sensing operon promoter
ttatttaccgtgacgaactaattgctcgtg

SEQ ID NO: 619 - DNA, 30 bp, Artificial Sequence
  GlnRS promoter
catacgccgttatacgttgtttacgctttg

SEQ ID NO: 620 - DNA, 30 bp, Artificial Sequence
  Constitutive weak promoter of lacZ
ttatgcttccggctcgtatgttgtgtggac

SEQ ID NO: 621 - DNA, 30 bp, Artificial Sequence
  Mutated LacZ promoter
ttatgcttccggctcgtatggtgtgtggac

SEQ ID NO: 622 - DNA, 30 bp, Artificial Sequence
  constitutive promoter with (TA)10 between -10 and -35 elements
atatatatatatatataatggaagcgtttt

SEQ ID NO: 623 - DNA, 30 bp, Artificial Sequence; identical to SEQ ID NO: 622
  constitutive promoter with (TA)9 between -10 and -35 elements

SEQ ID NO: 624 - DNA, 30 bp, Artificial Sequence
  constitutive promoter with (C)10 between -10 and -35 elements
ccccgaaagcttaagaatataattgtaagc

SEQ ID NO: 625 - DNA, 30 bp, Artificial Sequence; identical to SEQ ID NO: 624
  constitutive promoter with (C)12 between -10 and -35 elements

SEQ ID NO: 626 - DNA, 30 bp, Artificial Sequence
  optimized (TA) repeat constitutive promoter with 13 bp between -10 and -35 elements
tgacaatatatatatatatataatgctagc

SEQ ID NO: 627 - DNA, 30 bp, Artificial Sequence
  optimized (TA) repeat constitutive promoter with 15 bp between -10 and -35 elements
acaatatatatatatatatataatgctagc

SEQ ID NO: 628 - DNA, 30 bp, Artificial Sequence
  optimized (TA) repeat constitutive promoter with 17 bp between -10 and -35 elements
aatatatatatatatatatataatgctagc

SEQ ID NO: 629 - DNA, 30 bp, Artificial Sequence
  optimized (TA) repeat constitutive promoter with 19 bp between -10 and -35 elements
tatatatatatatatatatataatgctagc

SEQ ID NO: 630 - DNA, 30 bp, Artificial Sequence; identical to SEQ ID NO: 629
  optimized (TA) repeat constitutive promoter with 21 bp between -10 and -35 elements

SEQ ID NO: 631 - DNA, 30 bp, Artificial Sequence
  optimized (A) repeat constitutive promoter with 17 bp between -10 and -35 elements
aaaaaaaaaaaaaaaaaatataatgctagc

SEQ ID NO: 632 - DNA, 30 bp, Artificial Sequence; identical to SEQ ID NO: 631
  optimized (A) repeat constitutive promoter with 18 bp between -10 and -35 elements

SEQ ID NO: 633 - DNA, 30 bp, Artificial Sequence; identical to SEQ ID NO: 572
  J23101:GFP

SEQ ID NO: 634 - DNA, 30 bp, Artificial Sequence; identical to SEQ ID NO: 572
  J23119:IFP

SEQ ID NO: 635 - DNA, 30 bp, Artificial Sequence; identical to SEQ ID NO: 572
  J23119:HO1

SEQ ID NO: 636 - DNA, 30 bp, Artificial Sequence; identical to SEQ ID NO: 572
  Infrared signal reporter (J23119:IFP:J23119:HO1)

SEQ ID NO: 637 - DNA, 30 bp, Artificial Sequence; identical to SEQ ID NO: 592
  Double terminator + constitutive promoter

SEQ ID NO: 638 - DNA, 30 bp, Artificial Sequence
  Double terminator + Constitutive promoter + Strong RBS
tgctagctactagagattaaagaggagaaa

SEQ ID NO: 639 - DNA, 30 bp, Artificial Sequence
  IPTG inducible Lac promoter cassette
ttgtgagcggataacaagatactgagcaca

SEQ ID NO: 640 - DNA, 30 bp, Artificial Sequence; identical to SEQ ID NO: 639
  IPTG inducible Lac promoter cassette

SEQ ID NO: 641 - DNA, 30 bp, Artificial Sequence; identical to SEQ ID NO: 639
  IPTG inducible Lac promoter cassette

SEQ ID NO: 642 - DNA, 30 bp, Artificial Sequence
  M13K07 gene I promoter
cctgtttttatgttattctctctgtaaagg

SEQ ID NO: 643 - DNA, 30 bp, Artificial Sequence
  M13K07 gene II promoter
aaatatttgcttatacaatcttcctgtttt

SEQ ID NO: 644 - DNA, 30 bp, Artificial Sequence
  M13K07 gene III promoter
gctgataaaccgatacaattaaaggctcct

SEQ ID NO: 645 - DNA, 30 bp, Artificial Sequence
  M13K07 gene IV promoter
ctcttctcagcgtcttaatctaagctatcg

SEQ ID NO: 646 - DNA, 30 bp, Artificial Sequence
  M13K07 gene V promoter
atgagccagttcttaaaatcgcataaggta

SEQ ID NO: 647 - DNA, 30 bp, Artificial Sequence
  M13K07 gene VI promoter
ctattgattgtgacaaaataaacttattcc

SEQ ID NO: 648 - DNA, 30 bp, Artificial Sequence
  M13K07 gene VIII promoter
gtttcgcgcttggtataatcgctgggggtc

SEQ ID NO: 649 - DNA, 30 bp, Artificial Sequence
  M13110
ctttgcttctgactataatagtcagggtaa

SEQ ID NO: 650 - DNA, 30 bp, Artificial Sequence
  Modified promoter sequence of g3.
aaaccgatacaattaaaggctcctgctagc

SEQ ID NO: 651 - DNA, 30 bp, Artificial Sequence
  Constitutive Promoter I
caccacactgatagtgctagtgtagatcac

SEQ ID NO: 652 - DNA, 30 bp, Artificial Sequence
  Constitutive Promoter II
gccggaataactccctataatgcgccacca

SEQ ID NO: 653 - DNA, 30 bp, Artificial Sequence
  --Specify Parts List--
ttgacaagcttttcctcagctccgtaaact

SEQ ID NO: 654 - DNA, 30 bp, Artificial Sequence
  Full-length stationary phase osmY promoter
ggtttcaaaattgtgatctatatttaacaa

SEQ ID NO: 655 - DNA, 30 bp, Artificial Sequence; identical to SEQ ID NO: 654
  Minimal stationary phase osmY promoter

SEQ ID NO: 656 - DNA, 30 bp, Artificial Sequence
  htpG Heat Shock Promoter
tctattccaataaagaaatcttcctgcgtg

SEQ ID NO: 657 - DNA, 30 bp, Artificial Sequence
  Promoter veg a constitutive promoter for B. subtilis
aaaaatgggctcgtgttgtacaataaatgt

SEQ ID NO: 658 - DNA, 30 bp, Artificial Sequence
  Promoter 43 a constitutive promoter for B. subtilis
aaaaaaagcgcgcgattatgtaaaatataa

SEQ ID NO: 659 - DNA, 30 bp, Artificial Sequence
  Strong constitutive promoter for Bacillus subtilis
aattgcagtaggcatgacaaaatggactca

SEQ ID NO: 660 - DNA, 30 bp, Artificial Sequence
  PliaG
caagcttttcctttataatagaatgaatga

SEQ ID NO: 661 - DNA, 30 bp, Artificial Sequence
  PlepA
tctaagctagtgtattttgcgtttaatagt

SEQ ID NO: 662 - DNA, 30 bp, Artificial Sequence
  Pveg
aatgggctcgtgttgtacaataaatgtagt

SEQ ID NO: 663 - DNA, 30 bp, Artificial Sequence
  Promoter ctc for B. subtilis
atccttatcgttatgggtattgtttgtaat

SEQ ID NO: 664 - DNA, 30 bp, Artificial Sequence
  Promoter gsiB for B. subtilis
taaaagaattgtgagcgggaatacaacaac

SEQ ID NO: 665 - DNA, 30 bp, Artificial Sequence; identical to SEQ ID NO: 658
  Promoter 43 a constitutive promoter for B. subtilis

SEQ ID NO: 666 - DNA, 30 bp, Artificial Sequence
  Pspv2 from Salmonella
tacaaaataattcccctgcaaacattatca

SEQ ID NO: 667 - DNA, 30 bp, Artificial Sequence
  Pspv from Salmonella
tacaaaataattcccctgcaaacattatcg

SEQ ID NO: 668 - DNA, 30 bp, Artificial Sequence
  T7 promoter (strong promoter from T7 bacteriophage)
agggaatacaagctacttgttctttttgca

SEQ ID NO: 669 - DNA, 23 bp, Artificial Sequence
  T7 Promoter
taatacgactcactatagggaga

SEQ ID NO: 670 - DNA, 28 bp, Artificial Sequence
  T7 Promoter
gaatttaatacgactcactatagggaga

SEQ ID NO: 671 - DNA, 19 bp, Artificial Sequence
  T7 consensus -10 and rest
taatacgactcactatagg

SEQ ID NO: 672 - DNA, 30 bp, Artificial Sequence
  overlapping T7 promoter
gagtcgtattaatacgactcactatagggg

SEQ ID NO: 673 - DNA, 30 bp, Artificial Sequence
  more overlapping T7 promoter
agtgagtcgtactacgactcactatagggg

SEQ ID NO: 674 - DNA, 30 bp, Artificial Sequence
  weaken overlapping T7 promoter
gagtcgtattaatacgactctctatagggg

SEQ ID NO: 675 - DNA, 23 bp, Artificial Sequence
  T7 Consensus Promoter Sequence
taatacgactcactatagggaga

SEQ ID NO: 676 - DNA, 23 bp, Artificial Sequence
  T7 RNAP promoter
ttatacgactcactatagggaga

SEQ ID NO: 677 - DNA, 23 bp, Artificial Sequence
  T7 RNAP promoter
gaatacgactcactatagggaga

SEQ ID NO: 678 - DNA, 23 bp, Artificial Sequence
  T7 RNAP promoter
taatacgtctcactatagggaga

SEQ ID NO: 679 - DNA, 23 bp, Artificial Sequence
  T7 RNAP promoter
tcatacgactcactatagggaga

SEQ ID NO: 680 - DNA, 30 bp, Artificial Sequence
  T7 strong promoter
taatacgactcactatagggagaccacaac

SEQ ID NO: 681 - DNA, 30 bp, Artificial Sequence
  T7 weak binding and processivity
taattgaactcactaaagggagaccacagc

SEQ ID NO: 682 - DNA, 30 bp, Artificial Sequence
  T7 weak binding promoter
cgaagtaatacgactcactattagggaaga

SEQ ID NO: 683 - DNA, 30 bp, Artificial Sequence
  pCyc (Medium) Promoter
acaaacacaaatacacacactaaattaata

SEQ ID NO: 684 - DNA, 30 bp, Artificial Sequence
  pAdh (Strong) Promoter
ccaagcatacaatcaactatctcatataca

SEQ ID NO: 685 - DNA, 30 bp, Artificial Sequence
  pSte5 (Weak) Promoter
gatacaggatacagcggaaacaacttttaa

SEQ ID NO: 686 - DNA, 30 bp, Artificial Sequence
  yeast ADH1 promoter
tttcaagctataccaagcatacaatcaact

SEQ ID NO: 687 - DNA, 30 bp, Artificial Sequence
  cyc100 minimal promoter
cctttgcagcataaattactatacttctat

SEQ ID NO: 688 - DNA, 30 bp, Artificial Sequence; identical to SEQ ID NO: 687
  cyc70 minimal promoter

SEQ ID NO: 689 - DNA, 30 bp, Artificial Sequence; identical to SEQ ID NO: 687
  cyc43 minimal promoter

SEQ ID NO: 690 - DNA, 30 bp, Artificial Sequence; identical to SEQ ID NO: 687
  cyc28 minimal promoter

SEQ ID NO: 691 - DNA, 30 bp, Artificial Sequence; identical to SEQ ID NO: 687
  cyc16 minimal promoter

SEQ ID NO: 692 - DNA, 30 bp, Artificial Sequence
  pPGK1
ttatctactttttacaacaaatataaaaca

SEQ ID NO: 693 - DNA, 30 bp, Artificial Sequence; identical to SEQ ID NO: 683
  pCYC Yeast Promoter

SEQ ID NO: 694 - DNA, 30 bp, Artificial Sequence
  Yeast GPD (TDH3) Promoter
gtttcgaataaacacacataaacaaacaaa

SEQ ID NO: 695 - DNA, 30 bp, Artificial Sequence; identical to SEQ ID NO: 684
  yeast mid-length ADH1 promoter

SEQ ID NO: 696 - DNA, 30 bp, Artificial Sequence
  Yeast CLB1 promoter region, G2/M cell cycle specific
accatcaaaggaagctttaatcttctcata

SEQ ID NO: 697 - DNA, 30 bp, Artificial Sequence
  CMV promoter
agaacccactgcttactggcttatcgaaat

SEQ ID NO: 698 - DNA, 30 bp, Artificial Sequence
  Ubc Promoter
ggccgtttttggcttttttgttagacgaag

SEQ ID NO: 699 - protein, 9 aa, Lactobacillus curvatus
NIPQLTPTP

SEQ ID NO: 700 - DNA, 27 bp, Lactobacillus curvatus
aacattccgcagctgaccccgaccccg

SEQ ID NO: 701 - protein, 18 aa, Bacillus thuringiensis
  VARIANT 4, 7, 10: Xaa = any amino acid
DWTXWSXLVXAACSVELL

SEQ ID NO: 702 - DNA, 54 bp, Bacillus thuringiensis; identical to SEQ ID NO: 389
  misc_feature 10, 11, 12, 19, 20, 21, 28, 29, 30: n = A,T,C or G

SEQ ID NO: 703 - protein, 30 aa, Lactobacillus curvatus L442; identical to SEQ ID NO: 390

SEQ ID NO: 704 - DNA, 90 bp, Lactobacillus curvatus L442; identical to SEQ ID NO: 391

SEQ ID NO: 705 - protein, 43 aa, Carnobacterium divergens; identical to SEQ ID NO: 392

SEQ ID NO: 706 - DNA, 129 bp, Carnobacterium divergens; identical to SEQ ID NO: 393

SEQ ID NO: 707 - protein, 24 aa, Microbispora sp. (strain 107891)
VTSWSLCTPGCTSPGGGSNCSFCC

SEQ ID NO: 708 - DNA, 72 bp, Microbispora sp. (strain 107891)
gtgaccagctggagcctgtgcaccccgggctgcaccagcccgggcggcggcagcaactgcagcttttgctgc

SEQ ID NO: 709 - protein, 62 aa, Enterococcus sp.; identical to SEQ ID NO: 394

SEQ ID NO: 710 - DNA, 186 bp, Enterococcus sp.; identical to SEQ ID NO: 395

SEQ ID NO: 711 - protein, 39 aa, Enterococcus faecium; identical to SEQ ID NO: 396

SEQ ID NO: 712 - DNA, 117 bp, Enterococcus faecium; identical to SEQ ID NO: 397

SEQ ID NO: 713 - protein, 30 aa, Paenibacillus polymyxa; identical to SEQ ID NO: 398

SEQ ID NO: 714 - DNA, 90 bp, Paenibacillus polymyxa; identical to SEQ ID NO: 399

SEQ ID NO: 715 - protein, 31 aa, Staphylococcus epidermidis; identical to SEQ ID NO: 400

SEQ ID NO: 716 - DNA, 93 bp, Staphylococcus epidermidis; identical to SEQ ID NO: 401

SEQ ID NO: 717 - protein, 58 aa, Enterococcus faecium
MEKLTVKEMSQVVGGKYYGNGVSCNKKGCSVDWGKAIGIIGNNAAANLTTGGKAGWKG

SEQ ID NO: 718 - DNA, 178 bp, Enterococcus faecium
atggaaaaattaactgtgaaagaaatgtcgcaagtagttggcggaaagtactatggtaacggagtatcatgtaataaaaagggatgtagtgttgattggggaaaagctattggtattattggaaataatgctgctgctaatttaactactggcggaaaagcagggtggaaaggttaac

SEQ ID NO: 719 - protein, 39 aa, Paenibacillus polymyxa; identical to SEQ ID NO: 404

SEQ ID NO: 720 - DNA, 93 bp, Paenibacillus polymyxa; identical to SEQ ID NO: 401

SEQ ID NO: 721 - protein, 35 aa, Bacillus circulans; identical to SEQ ID NO: 406

SEQ ID NO: 722 - DNA, 105 bp, Bacillus circulans; identical to SEQ ID NO: 407

SEQ ID NO: 723 - protein, 30 aa, Paenibacillus polymyxa; identical to SEQ ID NO: 408

SEQ ID NO: 724 - DNA, 90 bp, Paenibacillus polymyxa; identical to SEQ ID NO: 409

SEQ ID NO: 725 - protein, 13 aa, Lactobacillus rhamnosus
AVPAVRKTNETLD

SEQ ID NO: 726 - DNA, 39 bp, Lactobacillus rhamnosus; identical to SEQ ID NO: 411

SEQ ID NO: 727 - protein, 60 aa, Bacillus licheniformis
MKNSAAREAFKGANHPAGMVSEEELKALVGGNDVNPETTPATTSSWTCITAGVTVSASLC

SEQ ID NO: 728 - DNA, 180 bp, Bacillus licheniformis
atgaaaaacagcgcggcgcgcgaagcgtttaaaggcgcgaaccatccggcgggcatggtgagcgaagaagaactgaaagcgctggtgggcggcaacgatgtgaacccggaaaccaccccggcgaccaccagcagctggacctgcattaccgcgggcgtgaccgtgagcgcgagcctgtgc

SEQ ID NO: 729 - protein, 689 aa, Pseudomonas aeruginosa; identical to SEQ ID NO: 276

SEQ ID NO: 730 - DNA, 2070 bp, Pseudomonas aeruginosa; identical to SEQ ID NO: 277

SEQ ID NO: 731 - protein, 36 aa, Lactobacillus plantarum; identical to SEQ ID NO: 414

SEQ ID NO: 732 - DNA, 108 bp, Lactobacillus plantarum; identical to SEQ ID NO: 415

SEQ ID NO: 733 - protein, 30 aa, Lactococcus lactis
MKTILRFVAGYDIASHKKKTGGYPWERGKA

SEQ ID NO: 734 - DNA, 93 bp, Lactococcus lactis
atgaaaacaatcctacgttttgttgctggctacgatattgctagtcataaaaagaaaactggcggctatccatgggaacgtggaaaagcttaa

SEQ ID NO: 735 - protein, 24 aa, Lactobacillus acidophilus
GNPKVAHCASQIGRSTAWGAVSGA

SEQ ID NO: 736 - DNA, 72 bp, Lactobacillus acidophilus; identical to SEQ ID NO: 417

SEQ ID NO: 737 - protein, 53 aa, Lactobacillus salivarius cp400
MFFNFMKKVDVKKNFGYKEVSRKDLAKVNGGKRKKHRCRVYNNGMPTGMYRWC

SEQ ID NO: 738 - DNA, 162 bp, Lactobacillus salivarius cp400
atgttttttaattttatgaaaaaagtagatgtgaagaagaattttggatataaagaagtttctagaaaagatctagctaaagtaaatggtggaaagagaaagaaacatcgttgcagagtttataataatggaatgcctacaggaatgtatcgttggtgctaa

SEQ ID NO: 739 - protein, 5 aa, Artificial Sequence
  Caspase 2 consensus sequence
DVADL

SEQ ID NO: 740 - protein, 5 aa, Artificial Sequence
  Caspase 2 consensus sequence
DVADI

SEQ ID NO: 741 - protein, 12 aa, Artificial Sequence
  Synthetic RAP-binding peptide, RBP
FHWWQTSPAHFS

SEQ ID NO: 742 - protein, 12 aa, Artificial Sequence
  Synthetic RAP-binding peptide, RBP
WPFAHWPWQYPR

SEQ ID NO: 743 - protein, 9 aa, Artificial Sequence
  Synthetic AgrC ligand
  VARIANT 5, 9: Thiolacton linkage between C5 and F9
GDSVCASYF

SEQ ID NO: 744 - protein, 7 aa, Artificial Sequence
  Synthetic AgrC ligand
  VARIANT 3, 7: Thiolacton linkage between C3 and F7
SVCASYF

SEQ ID NO: 745 - protein, 5 aa, Artificial Sequence
  Synthetic Cry1Aa ligand
SKADT

SEQ ID NO: 746 - protein, 5 aa, Artificial Sequence
  Synthetic Cry1Aa ligand
SKPAD

SEQ ID NO: 747 - protein, 11 aa, Artificial Sequence
  Synthetic Fsr ligand
  VARIANT 3, 11: Lacton linkage between S3 and A11
QNSAAAFAAWA

SEQ ID NO: 748 - protein, 11 aa, Artificial Sequence
  Synthetic Fsr ligand
  VARIANT 3, 11: Lacton linkage between S3 and A11
QNSAAAFGQWA

SEQ ID NO: 749 - protein, 7 aa, Artificial Sequence
  Synthetic AgrC1, AgrC2
  VARIANT 4, 7: Thiolacton linkage between C4 and M7)
YSTCFIM

SEQ ID NO: 750 - protein, 7 aa, Artificial Sequence
  Synthetic AgrC1, AgrC2
  VARIANT 3, 7: Thiolacton linkage between C3 and M7
STCAFIM